European Patent Specification EP 3 461 896 B1, published November 29, 2023. Title: METHODS OF TRANSCRIPTION ACTIVATOR LIKE EFFECTOR ASSEMBLY. Applicant: THE GENERAL HOSPITAL CORPORATION. The sequence listing filed with the application follows.

SEQUENCE LISTING (439 sequences)

SEQ ID NO: 1 - DNA, 2710 bp, Artificial Sequence
  Description of Artificial Sequence: Synthetic polynucleotide
tcgcgcgtttcggtgatgacggtgaaaacctctgacacatgcagctcccggagacggtcacagcttgtctgtaagcggatgccgggagcagacaagcccgtcagggcgcgtcagcgggtgttggcgggtgtcggggctggcttaactatgcggcatcagagcagattgtactgagagtgcaccatatgcggtgtgaaataccgcacagatgcgtaaggagaaaataccgcatcaggcgccattcgccattcaggctgcgcaactgttgggaagggcgatcggtgcgggcctcttcgctattacgccagctggcgaaagggggatgtgctgcaaggcgattaagttgggtaacgccagggttttcccagtcacgacgttgtaaaacgacggccagtgaattcgagctcggtacctcgcgaatgcatctagatatcggatcccgggcccgtcgactgcagaggcctgcatgcaagcttggcgtaatcatggtcatagctgtttcctgtgtgaaattgttatccgctcacaattccacacaacatacgagccggaagcataaagtgtaaagcctggggtgcctaatgagtgagctaactcacattaattgcgttgcgctcactgcccgctttccagtcgggaaacctgtcgtgccagctgcattaatgaatcggccaacgcgcggggagaggcggtttgcgtattgggcgctcttccgcttcctcgctcactgactcgctgcgctcggtcgttcggctgcggcgagcggtatcagctcactcaaaggcggtaatacggttatccacagaatcaggggataacgcaggaaagaacatgtgagcaaaaggccagcaaaaggccaggaaccgtaaaaaggccgcgttgctggcgtttttccataggctccgcccccctgacgagcatcacaaaaatcgacgctcaagtcagaggtggcgaaacccgacaggactataaagataccaggcgtttccccctggaagctccctcgtgcgctctcctgttccgaccctgccgcttaccggatacctgtccgcctttctcccttcgggaagcgtggcgctttctcatagctcacgctgtaggtatctcagttcggtgtaggtcgttcgctccaagctgggctgtgtgcacgaaccccccgttcagcccgaccgctgcgccttatccggtaactatcgtcttgagtccaacccggtaagacacgacttatcgccactggcagcagccactggtaacaggattagcagagcgaggtatgtaggcggtgctacagagttcttgaagtggtggcctaactacggctacactagaagaacagtatttggtatctgcgctctgctgaagccagttaccttcggaaaaagagttggtagctcttgatccggcaaacaaaccaccgctggtagcggtggtttttttgtttgcaagcagcagattacgcgcagaaaaaaaggatctcaagaagatcctttgatcttttctacggggtctgacgctcagtggaacgaaaactcacgttaagggattttggtcatgagattatcaaaaaggatcttcacctagatccttttaaattaaaaatgaagttttaaatcaatctaaagtatatatgagtaaacttggtctgacagttaccaatgcttaatcagtgaggcacctatctcagcgatctgtctatttcgttcatccatagttgcctgactccccgtcgtgtagataactacgatacgggagggcttaccatctggccccagtgctgcaatgataccgcgagagccacgctcaccggctccagatttatcagcaataaaccagccagccggaagggccgagcgcagaagtggtcctgcaactttatccgcctccatccagtctattaattgttgccgggaagctagagtaagtagttcgccagttaatagtttgcgcaacgttgttgccattgctacaggcatcgtggtgtcacgctcgtcgtttggtatggcttcattcagctccggttcccaacgatcaaggcgagttacatgatcccccatgttgtgcaaaaaagcggttagctccttcggtcctccgatcgttgtcagaagtaagttggccgcagtgttatcactcatggttatggcagcactgcataattctcttactgtcatgccatccgtaagatgcttttctgtgactggtgagtactcaaccaagtcattctgagaatagtgtatgcggcgaccgagttgctcttgcccggcgtcaatacgggataataccgcgccacatagcagaactttaaaagtgctcatcattggaaaacgttcttcggggcgaaaactctcaaggatcttaccgctgttgagatccagttcgatgtaacccactcgtgcacccaactgatcttcagcatcttttactttcaccagcgtttctgggtgagcaaaaacaggaaggcaaaatgccgcaaaaaagggaataagggcgacacggaaatgttgaatactcatactcttcctttttcaatattattgaagcatttatcagggttattgtctcatgagcggatacatatttgaatgtatttagaaaaataaacaaataggggttccgcgcacatttccccgaaaagtgccacctgacgtctaagaaaccattattatcatgacattaacctataaaaataggcgtatcacgaggccctttcgtc

SEQ ID NO: 2 - protein, 34 aa, Artificial Sequence
  Description of Artificial Sequence: Synthetic polypeptide
LTPDQVVAIASNIGGKQALETVQRLLPVLCQDHG

SEQ ID NO: 3 - protein, 34 aa, Artificial Sequence
  Description of Artificial Sequence: Synthetic polypeptide
LTPEQVVAIASNIGGKQALETVQRLLPVLCQAHG

SEQ ID NO: 4 - protein, 34 aa, Artificial Sequence
  Description of Artificial Sequence: Synthetic polypeptide
LTPDQVVAIASNIGGKQALETVQRLLPVLCQAHG

SEQ ID NO: 5 - protein, 34 aa, Artificial Sequence
  Description of Artificial Sequence: Synthetic polypeptide
LTPAQVVAIASNIGGKQALETVQRLLPVLCQDHG

SEQ ID NO: 6 - DNA, 102 bp, Artificial Sequence
  Description of Artificial Sequence: Synthetic polynucleotide
ctgaccccagaccaggtagtcgcaatcgcgtcgaacattgggggaaagcaagccctggaaaccgtgcaaaggttgttgccggtcctttgtcaagaccacggc

SEQ ID NO: 7 - DNA, 102 bp, Artificial Sequence
  Description of Artificial Sequence: Synthetic polynucleotide
cttacaccggagcaagtcgtggccattgcaagcaacatcggtggcaaacaggctcttgagacggttcagagacttctcccagttctctgtcaagcccacggg

SEQ ID NO: 8 - DNA, 102 bp, Artificial Sequence
  Description of Artificial Sequence: Synthetic polynucleotide
ctgactcccgatcaagttgtagcgattgcgtcgaacattggagggaaacaagcattggagactgtccaacggctccttcccgtgttgtgtcaagcccacggt

SEQ ID NO: 9 - DNA, 102 bp, Artificial Sequence
  Description of Artificial Sequence: Synthetic polynucleotide
ttgacgcctgcacaagtggtcgccatcgcctccaatattggcggtaagcaggcgctggaaacagtacagcgcctgctgcctgtactgtgccaggatcatgga

SEQ ID NO: 10 - DNA, 3269 bp, Artificial Sequence
  Description of Artificial Sequence: Synthetic polynucleotide
  modified_base (1483)..(1491): a, c, t, g, unknown or other
gacggatcgggagatctcccgatcccctatggtcgactctcagtacaatctgctctgatgccgcatagttaagccagtatctgctccctgcttgtgtgttggaggtcgctgagtagtgcgcgagcaaaatttaagctacaacaaggcaaggcttgaccgacaattgcatgaagaatctgcttagggttaggcgttttgcgctgcttcgcgatgtacgggccagatatacgcgttgacattgattattgactagttattaatagtaatcaattacggggtcattagttcatagcccatatatggagttccgcgttacataacttacggtaaatggcccgcctggctgaccgcccaacgacccccgcccattgacgtcaataatgacgtatgttcccatagtaacgccaatagggactttccattgacgtcaatgggtggactatttacggtaaactgcccacttggcagtacatcaagtgtatcatatgccaagtacgccccctattgacgtcaatgacggtaaatggcccgcctggcattatgcccagtacatgaccttatgggactttcctacttggcagtacatctacgtattagtcatcgctattaccatggtgatgcggttttggcagtacatcaatgggcgtggatagcggtttgactcacggggatttccaagtctccaccccattgacgtcaatgggagtttgttttggcaccaaaatcaacgggactttccaaaatgtcgtaacaactccgccccattgacgcaaatgggcggtaggcgtgtacggtgggaggtctatataagcagagctctctggctaactagagaacccactgcttactggcttatcgaaattaatacgactcactatagggagacccaagctggctagcaccatggactacaaagaccatgacggtgattataaagatcatgacatcgattacaaggatgacgatgacaagatggcccccaagaagaagaggaaggtgggcattcaccgcggggtacctatggtggacttgaggacactcggttattcgcaacagcaacaggagaaaatcaagcctaaggtcaggagcaccgtcgcgcaacaccacgaggcgcttgtggggcatggcttcactcatgcgcatattgtcgcgctttcacagcaccctgcggcgcttgggacggtggctgtcaaataccaagatatgattgcggccctgcccgaagccacgcacgaggcaattgtaggggtcggtaaacagtggtcgggagcgcgagcacttgaggcgctgctgactgtggcgggtgagcttagggggcctccgctccagctcgacaccgggcagctgctgaagatcgcgaagagagggggagtaacagcggtagaggcagtgcacgcctggcgcaatgcgctcaccggggcccccttgaacagagacgattaatgcgtctcgctgacacccgaacaggtggtcgccattgctnnnnnnnnnggaggacggccagccttggagtccatcgtagcccaattgtccaggcccgatcccgcgttggctgcgttaacgaatgaccatctggtggcgttggcatgtcttggtggacgacccgcgctcgatgcagtcaaaaagggtctgcctcatgctcccgcattgatcaaaagaaccaaccggcggattcccgagagaacttcccatcgagtcgcgggatcccaactagtcaaaagtgaactggaggagaagaaatctgaacttcgtcataaattgaaatatgtgcctcatgaatatattgaattaattgaaattgccagaaattccactcaggatagaattcttgaaatgaaggtaatggaattttttatgaaagtttatggatatagaggtaaacatttgggtggatcaaggaaaccggacggagcaatttatactgtcggatctcctattgattacggtgtgatcgtggatactaaagcttatagcggaggttataatctgccaattggccaagcagatgaaatgcaacgatatgtcgaagaaaatcaaacacgaaacaaacatatcaaccctaatgaatggtggaaagtctatccatcttctgtaacggaatttaagtttttatttgtgagtggtcactttaaaggaaactacaaagctcagcttacacgattaaatcatatcactaattgtaatggagctgttcttagtgtagaagagcttttaattggtggagaaatgattaaagccggcacattaaccttagaggaagtcagacggaaatttaataacggcgagataaacttttaagggcccttcgaaggtaagcctatccctaaccctctcctcggtctcgattctacgcgtaccggtcatcatcaccatcaccattgagtttaaacccgctgatcagcctcgactgtgccttctagttgccagccatctgttgtttgcccctcccccgtgccttccttgaccctggaaggtgccactcccactgtcctttcctaataaaatgaggaaattgcatcgcattgtctgagtaggtgtcattctattctggggggtggggtggggcaggacagcaagggggaggattgggaagacaatagcaggcatgctggggatgcggtgggctctatggcttctgaggcggaaagaaccagctggggctctagggggtatccccacgcgccctgtagcggcgcattaagcgcggcgggtgtggtggttacgcgcagcgtgaccgctacacttgccagcgccctagcgcccgctcctttcgctttcttcccttcctttctcgccacgttcgccggctttccccgtcaagctctaaatcggggcatccctttagggttccgatttagtgctttacggcacctcgaccccaaaaaacttgattagggtgatggttcacgtagtgggccatcgccctgatagacggtttttcgccctttgacgttggagtccacgttctttaatagtggactcttgttccaaactggaacaacactcaaccctatctcggtctattcttttgatttataagggattttggggatttcggcctattggttaaaaaatgagctgatttaacaaaaatttaacgcgaattaattctgtggaatgtgtgtcagttagggtgtggaaagtccccaggctccccaggcaggcagaagtatgcaaagcatgcatctcaattagtcagcaaccaggtgtggaaagtccccaggctccccagcaggcagaagtatgcaaagcatgcatctcaattagtc

SEQ ID NO: 11 - DNA, 3178 bp, Artificial Sequence
  Description of Artificial Sequence: Synthetic polynucleotide
agcaaccatagtcccgcccctaactccgcccatcccgcccctaactccgcccagttccgcccattctccgccccatggctgactaattttttttatttatgcagaggccgaggccgcctctgcctctgagctattccagaagtagtgaggaggcttttttggaggcctaggcttttgcaaaaagctcccgggagcttgtatatccattttcggatctgatcagcacgtgttgacaattaatcatcggcatagtatatcggcatagtataatacgacaaggtgaggaactaaaccatggccaagcctttgtctcaagaagaatccaccctcattgaaagagcaacggctacaatcaacagcatccccatctctgaagactacagcgtcgccagcgcagctctctctagcgacggccgcatcttcactggtgtcaatgtatatcattttactgggggaccttgtgcagaactcgtggtgctgggcactgctgctgctgcggcagctggcaacctgacttgtatcgtcgcgatcggaaatgagaacaggggcatcttgagcccctgcggacggtgtcgacaggtgcttctcgatctgcatcctgggatcaaagcgatagtgaaggacagtgatggacagccgacggcagttgggattcgtgaattgctgccctctggttatgtgtgggagggctaagcacttcgtggccgaggagcaggactgacacgtgctacgagatttcgattccaccgccgccttctatgaaaggttgggcttcggaatcgttttccgggacgccggctggatgatcctccagcgcggggatctcatgctggagttcttcgcccaccccaacttgtttattgcagcttataatggttacaaataaagcaatagcatcacaaatttcacaaataaagcatttttttcactgcattctagttgtggtttgtccaaactcatcaatgtatcttatcatgtctgtataccgtcgacctctagctagagcttggcgtaatcatggtcatagctgtttcctgtgtgaaattgttatccgctcacaattccacacaacatacgagccggaagcataaagtgtaaagcctggggtgcctaatgagtgagctaactcacattaattgcgttgcgctcactgcccgctttccagtcgggaaacctgtcgtgccagctgcattaatgaatcggccaacgcgcggggagaggcggtttgcgtattgggcgctcttccgcttcctcgctcactgactcgctgcgctcggtcgttcggctgcggcgagcggtatcagctcactcaaaggcggtaatacggttatccacagaatcaggggataacgcaggaaagaacatgtgagcaaaaggccagcaaaaggccaggaaccgtaaaaaggccgcgttgctggcgtttttccataggctccgcccccctgacgagcatcacaaaaatcgacgctcaagtcagaggtggcgaaacccgacaggactataaagataccaggcgtttccccctggaagctccctcgtgcgctctcctgttccgaccctgccgcttaccggatacctgtccgcctttctcccttcgggaagcgtggcgctttctcaatgctcacgctgtaggtatctcagttcggtgtaggtcgttcgctccaagctgggctgtgtgcacgaaccccccgttcagcccgaccgctgcgccttatccggtaactatcgtcttgagtccaacccggtaagacacgacttatcgccactggcagcagccactggtaacaggattagcagagcgaggtatgtaggcggtgctacagagttcttgaagtggtggcctaactacggctacactagaaggacagtatttggtatctgcgctctgctgaagccagttaccttcggaaaaagagttggtagctcttgatccggcaaacaaaccaccgctggtagcggtggtttttttgtttgcaagcagcagattacgcgcagaaaaaaaggatctcaagaagatcctttgatcttttctacggggtctgacgctcagtggaacgaaaactcacgttaagggattttggtcatgagattatcaaaaaggatcttcacctagatccttttaaattaaaaatgaagttttaaatcaatctaaagtatatatgagtaaacttggtctgacagttaccaatgcttaatcagtgaggcacctatctcagcgatctgtctatttcgttcatccatagttgcctgactccccgtcgtgtagataactacgatacgggagggcttaccatctggccccagtgctgcaatgataccgcgagacccacgctcaccggctccagatttatcagcaataaaccagccagccggaagggccgagcgcagaagtggtcctgcaactttatccgcctccatccagtctattaattgttgccgggaagctagagtaagtagttcgccagttaatagtttgcgcaacgttgttgccattgctacaggcatcgtggtgtcacgctcgtcgtttggtatggcttcattcagctccggttcccaacgatcaaggcgagttacatgatcccccatgttgtgcaaaaaagcggttagctccttcggtcctccgatcgttgtcagaagtaagttggccgcagtgttatcactcatggttatggcagcactgcataattctcttactgtcatgccatccgtaagatgcttttctgtgactggtgagtactcaaccaagtcattctgagaatagtgtatgcggcgaccgagttgctcttgcccggcgtcaatacgggataataccgcgccacatagcagaactttaaaagtgctcatcattggaaaacgttcttcggggcgaaaactctcaaggatcttaccgctgttgagatccagttcgatgtaacccactcgtgcacccaactgatcttcagcatcttttactttcaccagcgtttctgggtgagcaaaaacaggaaggcaaaatgccgcaaaaaagggaataagggcgacacggaaatgttgaatactcatactcttcctttttcaatattattgaagcatttatcagggttattgtctcatgagcggatacatatttgaatgtatttagaaaaataaacaaataggggttccgcgcacatttccccgaaaagtgccacctgacgtc

SEQ ID NO: 12 - DNA, 111 bp, Homo sapiens
ctacggcgtgcagtgcttcagccgctaccccgaccacatgaagcagcacgacttcttcaagtccgccatgcccgaaggctacgtccaggagcgcaccatcttcttcaagga

SEQ ID NO: 13 - DNA, 108 bp, Homo sapiens
ctacggcgtgcagtgcttcagccgctaccccgacatgaagcagcacgacttcttcaagtccgccatgcccgaaggctacgtccaggagcgcaccatcttcttcaagga

SEQ ID NO: 14 - DNA, 95 bp, Homo sapiens
ctacggcgtgcagtgcttcagccgaagcagcacgacttcttcaagtccgccatgcccgaaggctacgtccaggagcgcaccatcttcttcaagga

SEQ ID NO: 15 - DNA, 90 bp, Homo sapiens
ctacggcgtgcagtgcttcagccgctacgacttcttcaagtccgccatgcccgaaggctacgtccaggagcgcaccatcttcttcaagga

SEQ ID NO: 16 - DNA, 89 bp, Homo sapiens
  modified_base (61)..(61): a, c, t, g, unknown or other
ctacggcgtgcagtgcttcagccgcacgacttcttccagtccgccatgcccgaaggctacntccaggagcgcaccatcttcttcaagga

SEQ ID NO: 17 - DNA, 80 bp, Homo sapiens
ctacggcgtgcagtgcttcagcacttcaagtccgccatgcccgaaggctacgtccaggagcgcaccatcttcttcaagga

SEQ ID NO: 18 - DNA, 78 bp, Homo sapiens
ctacggcgtgcagcacgacttcttcaagtccgccatgcccgaaggctacgtccaggagcgcaccatcttcttcaagga

SEQ ID NO: 19 - DNA, 78 bp, Homo sapiens; identical to SEQ ID NO: 18

SEQ ID NO: 20 - DNA, 60 bp, Homo sapiens
ctacggcgtgcagtgcttgcccgaaggctacgtccaggagcgcaccatcttcttcaagga

SEQ ID NO: 21 - DNA, 57 bp, Homo sapiens
ctacggcgtgcagtgcttcagccgctacgtccaggagcgcaccatcttcttcaagga

SEQ ID NO: 22 - DNA, 51 bp, Homo sapiens
ctacgccatgcccgaaggctacgtccaggagcgcaccatcttcttcaagga

SEQ ID NO: 23 - DNA, 27 bp, Homo sapiens
ctacggcgtgcagtgcttcttcaagga

SEQ ID NO: 24 - DNA, 113 bp, Homo sapiens
ctacggcgtgcagtgcttcagccgctaccccgacaccacatgaagcagcacgacttcttcaagtccgccatgcccgaaggctacgtccaggagcgcaccatcttcttcaagga

SEQ ID NO: 25 - DNA, 2328 bp, Artificial Sequence
  Description of Artificial Sequence: Synthetic polynucleotide
tctagagctagcaccatggactacaaagaccatgacggtgattataaagatcatgacatcgattacaaggatgacgatgacaagatggcccccaagaagaagaggaaggtgggcattcaccgcggggtacctatggtggacttgaggacactcggttattcgcaacagcaacaggagaaaatcaagcctaaggtcaggagcaccgtcgcgcaacaccacgaggcgcttgtggggcatggcttcactcatgcgcatattgtcgcgctttcacagcaccctgcggcgcttgggacggtggctgtcaaataccaagatatgattgcggccctgcccgaagccacgcacgaggcaattgtaggggtcggtaaacagtggtcgggagcgcgagcacttgaggcgctgctgactgtggcgggtgagcttagggggcctccgctccagctcgacaccgggcagctgctgaagatcgcgaagagagggggagtaacagcggtagaggcagtgcacgcctggcgcaatgcgctcaccggggcccccttgaacctgaccccagaccaggtagtcgcaatcgcgaacaataatgggggaaagcaagccctggaaaccgtgcaaaggttgttgccggtcctttgtcaagaccacggccttacaccggagcaagtcgtggccattgcatcccacgacggtggcaaacaggctcttgagacggttcagagacttctcccagttctctgtcaagcccacgggctgactcccgatcaagttgtagcgattgcgtcgaacattggagggaaacaagcattggagactgtccaacggctccttcccgtgttgtgtcaagcccacggtttgacgcctgcacaagtggtcgccatcgccaacaacaacggcggtaagcaggcgctggaaacagtacagcgcctgctgcctgtactgtgccaggatcatggactgaccccagaccaggtagtcgcaatcgcgtcaaacggagggggaaagcaagccctggaaaccgtgcaaaggttgttgccggtcctttgtcaagaccacggccttacaccggagcaagtcgtggccattgcaaataataacggtggcaaacaggctcttgagacggttcagagacttctcccagttctctgtcaagcccacgggctgactcccgatcaagttgtagcgattgcgtcgcatgacggagggaaacaagcattggagactgtccaacggctccttcccgtgttgtgtcaagcccacggtttgacgcctgcacaagtggtcgccatcgcctcgaatggcggcggtaagcaggcgctggaaacagtacagcgcctgctgcctgtactgtgccaggatcatggactgaccccagaccaggtagtcgcaatcgcgtcaaacggagggggaaagcaagccctggaaaccgtgcaaaggttgttgccggtcctttgtcaagaccacggccttacaccggagcaagtcgtggccattgcatcccacgacggtggcaaacaggctcttgagacggttcagagacttctcccagttctctgtcaagcccacgggctgactcccgatcaagttgtagcgattgcgtcgaacattggagggaaacaagcattggagactgtccaacggctccttcccgtgttgtgtcaagcccacggtttgacgcctgcacaagtggtcgccatcgccaacaacaacggcggtaagcaggcgctggaaacagtacagcgcctgctgcctgtactgtgccaggatcatggactgaccccagaccaggtagtcgcaatcgcgtcacatgacgggggaaagcaagccctggaaaccgtgcaaaggttgttgccggtcctttgtcaagaccacggccttacaccggagcaagtcgtggccattgcatcccacgacggtggcaaacaggctcttgagacggttcagagacttctcccagttctctgtcaagcccacgggctgactcccgatcaagttgtagcgattgcgaataacaatggagggaaacaagcattggagactgtccaacggctccttcccgtgttgtgtcaagcccacggtctgacacccgaacaggtggtcgccattgcttcccacgacggaggacggccagccttggagtccatcgtagcccaattgtccaggcccgatcccgcgttggctgcgttaacgaatgaccatctggtggcgttggcatgtcttggtggacgacccgcgctcgatgcagtcaaaaagggtctgcctcatgctcccgcattgatcaaaagaaccaaccggcggattcccgagagaacttcccatcgagtcgcgggatcc

SEQ ID NO: 26 - protein, 771 aa, Artificial Sequence
  Description of Artificial Sequence: Synthetic polypeptide
MDYKDHDGDYKDHDIDYKDDDDKMAPKKKRKVGIHRGVPMVDLRTLGYSQQQQEKIKPKVRSTVAQHHEALVGHGFTHAHIVALSQHPAALGTVAVKYQDMIAALPEATHEAIVGVGKQWSGARALEALLTVAGELRGPPLQLDTGQLLKIAKRGGVTAVEAVHAWRNALTGAPLNLTPDQVVAIANNNGGKQALETVQRLLPVLCQDHGLTPEQVVAIASHDGGKQALETVQRLLPVLCQAHGLTPDQVVAIASNIGGKQALETVQRLLPVLCQAHGLTPAQVVAIANNNGGKQALETVQRLLPVLCQDHGLTPDQVVAIASNGGGKQALETVQRLLPVLCQDHGLTPEQVVAIANNNGGKQALETVQRLLPVLCQAHGLTPDQVVAIASHDGGKQALETVQRLLPVLCQAHGLTPAQVVAIASNGGGKQALETVQRLLPVLCQDHGLTPDQVVAIASNGGGKQALETVQRLLPVLCQDHGLTPEQVVAIASHDGGKQALETVQRLLPVLCQAHGLTPDQVVAIASNIGGKQALETVQRLLPVLCQAHGLTPAQVVAIANNNGGKQALETVQRLLPVLCQDHGLTPDQVVAIASHDGGKQALETVQRLLPVLCQDHGLTPEQVVAIASHDGGKQALETVQRLLPVLCQAHGLTPDQVVAIANNNGGKQALETVQRLLPVLCQAHGLTPEQVVAIASHDGGRPALESIVAQLSRPDPALAALTNDHLVALACLGGRPALDAVKKGLPHAPALIKRTNRRIPERTSHRVAGS

SEQ ID NO: 27 - DNA, 2430 bp, Artificial Sequence
  Description of Artificial Sequence: Synthetic polynucleotide
tctagagctagcaccatggactacaaagaccatgacggtgattataaagatcatgacatcgattacaaggatgacgatgacaagatggcccccaagaagaagaggaaggtgggcattcaccgcggggtacctatggtggacttgaggacactcggttattcgcaacagcaacaggagaaaatcaagcctaaggtcaggagcaccgtcgcgcaacaccacgaggcgcttgtggggcatggcttcactcatgcgcatattgtcgcgctttcacagcaccctgcggcgcttgggacggtggctgtcaaataccaagatatgattgcggccctgcccgaagccacgcacgaggcaattgtaggggtcggtaaacagtggtcgggagcgcgagcacttgaggcgctgctgactgtggcgggtgagcttagggggcctccgctccagctcgacaccgggcagctgctgaagatcgcgaagagagggggagtaacagcggtagaggcagtgcacgcctggcgcaatgcgctcaccggggcccccttgaacctgaccccagaccaggtagtcgcaatcgcgaacaataatgggggaaagcaagccctggaaaccgtgcaaaggttgttgccggtcctttgtcaagaccacggccttacaccggagcaagtcgtggccattgcatcccacgacggtggcaaacaggctcttgagacggttcagagacttctcccagttctctgtcaagcccacgggctgactcccgatcaagttgtagcgattgcgtcgaacattggagggaaacaagcattggagactgtccaacggctccttcccgtgttgtgtcaagcccacggtttgacgcctgcacaagtggtcgccatcgccaacaacaacggcggtaagcaggcgctggaaacagtacagcgcctgctgcctgtactgtgccaggatcatggactgaccccagaccaggtagtcgcaatcgcgtcaaacggagggggaaagcaagccctggaaaccgtgcaaaggttgttgccggtcctttgtcaagaccacggccttacaccggagcaagtcgtggccattgcaaataataacggtggcaaacaggctcttgagacggttcagagacttctcccagttctctgtcaagcccacgggctgactcccgatcaagttgtagcgattgcgtcgcatgacggagggaaacaagcattggagactgtccaacggctccttcccgtgttgtgtcaagcccacggtttgacgcctgcacaagtggtcgccatcgcctcgaatggcggcggtaagcaggcgctggaaacagtacagcgcctgctgcctgtactgtgccaggatcatggactgaccccagaccaggtagtcgcaatcgcgtcaaacggagggggaaagcaagccctggaaaccgtgcaaaggttgttgccggtcctttgtcaagaccacggccttacaccggagcaagtcgtggccattgcatcccacgacggtggcaaacaggctcttgagacggttcagagacttctcccagttctctgtcaagcccacgggctgactcccgatcaagttgtagcgattgcgtcgaacattggagggaaacaagcattggagactgtccaacggctccttcccgtgttgtgtcaagcccacggtttgacgcctgcacaagtggtcgccatcgccaacaacaacggcggtaagcaggcgctggaaacagtacagcgcctgctgcctgtactgtgccaggatcatggactgaccccagaccaggtagtcgcaatcgcgtcacatgacgggggaaagcaagccctggaaaccgtgcaaaggttgttgccggtcctttgtcaagaccacggccttacaccggagcaagtcgtggccattgcatcccacgacggtggcaaacaggctcttgagacggttcagagacttctcccagttctctgtcaagcccacgggctgactcccgatcaagttgtagcgattgcgaataacaatggagggaaacaagcattggagactgtccaacggctccttcccgtgttgtgtcaagcccacggtttgacgcctgcacaagtggtcgccatcgccagccatgatggcggtaagcaggcgctggaaacagtacagcgcctgctgcctgtactgtgccaggatcatggactgacacccgaacaggtggtcgccattgcttctaatgggggaggacggccagccttggagtccatcgtagcccaattgtccaggcccgatcccgcgttggctgcgttaacgaatgaccatctggtggcgttggcatgtcttggtggacgacccgcgctcgatgcagtcaaaaagggtctgcctcatgctcccgcattgatcaaaagaaccaaccggcggattcccgagagaacttcccatcgagtcgcgggatcc

SEQ ID NO: 28 - protein, 805 aa, Artificial Sequence
  Description of Artificial Sequence: Synthetic polypeptide
MDYKDHDGDYKDHDIDYKDDDDKMAPKKKRKVGIHRGVPMVDLRTLGYSQQQQEKIKPKVRSTVAQHHEALVGHGFTHAHIVALSQHPAALGTVAVKYQDMIAALPEATHEAIVGVGKQWSGARALEALLTVAGELRGPPLQLDTGQLLKIAKRGGVTAVEAVHAWRNALTGAPLNLTPDQVVAIANNNGGKQALETVQRLLPVLCQDHGLTPEQVVAIASHDGGKQALETVQRLLPVLCQAHGLTPDQVVAIASNIGGKQALETVQRLLPVLCQAHGLTPAQVVAIANNNGGKQALETVQRLLPVLCQDHGLTPDQVVAIASNGGGKQALETVQRLLPVLCQDHGLTPEQVVAIANNNGGKQALETVQRLLPVLCQAHGLTPDQVVAIASHDGGKQALETVQRLLPVLCQAHGLTPAQVVAIASNGGGKQALETVQRLLPVLCQDHGLTPDQVVAIASNGGGKQALETVQRLLPVLCQDHGLTPEQVVAIASHDGGKQALETVQRLLPVLCQAHGLTPDQVVAIASNIGGKQALETVQRLLPVLCQAHGLTPAQVVAIANNNGGKQALETVQRLLPVLCQDHGLTPDQVVAIASHDGGKQALETVQRLLPVLCQDHGLTPEQVVAIASHDGGKQALETVQRLLPVLCQAHGLTPDQVVAIANNNGGKQALETVQRLLPVLCQAHGLTPAQVVAIASHDGGKQALETVQRLLPVLCQDHGLTPEQVVAIASNGGGRPALESIVAQLSRPDPALAALTNDHLVALACLGGRPALDAVKKGLPHAPALIKRTNRRIPERTSHRVAGS

SEQ ID NO: 29 - DNA, 2430 bp, Artificial Sequence
  Description of Artificial Sequence: Synthetic polynucleotide
tctagagctagcaccatggactacaaagaccatgacggtgattataaagatcatgacatcgattacaaggatgacgatgacaagatggcccccaagaagaagaggaaggtgggcattcaccgcggggtacctatggtggacttgaggacactcggttattcgcaacagcaacaggagaaaatcaagcctaaggtcaggagcaccgtcgcgcaacaccacgaggcgcttgtggggcatggcttcactcatgcgcatattgtcgcgctttcacagcaccctgcggcgcttgggacggtggctgtcaaataccaagatatgattgcggccctgcccgaagccacgcacgaggcaattgtaggggtcggtaaacagtggtcgggagcgcgagcacttgaggcgctgctgactgtggcgggtgagcttagggggcctccgctccagctcgacaccgggcagctgctgaagatcgcgaagagagggggagtaacagcggtagaggcagtgcacgcctggcgcaatgcgctcaccggggcccccttgaacctgaccccagaccaggtagtcgcaatcgcgtcaaacggagggggaaagcaagccctggaaaccgtgcaaaggttgttgccggtcctttgtcaagaccacggccttacaccggagcaagtcgtggccattgcaaataataacggtggcaaacaggctcttgagacggttcagagacttctcccagttctctgtcaagcccacgggctgactcccgatcaagttgtagcgattgcgtcgaacattggagggaaacaagcattggagactgtccaacggctccttcccgtgttgtgtcaagcccacggtttgacgcctgcacaagtggtcgccatcgcctccaatattggcggtaagcaggcgctggaaacagtacagcgcctgctgcctgtactgtgccaggatcatggactgaccccagaccaggtagtcgcaatcgcgaacaataatgggggaaagcaagccctggaaaccgtgcaaaggttgttgccggtcctttgtcaagaccacggccttacaccggagcaagtcgtggccattgcaagcaacatcggtggcaaacaggctcttgagacggttcagagacttctcccagttctctgtcaagcccacgggctgactcccgatcaagttgtagcgattgcgtcgaacattggagggaaacaagcattggagactgtccaacggctccttcccgtgttgtgtcaagcccacggtttgacgcctgcacaagtggtcgccatcgccaacaacaacggcggtaagcaggcgctggaaacagtacagcgcctgctgcctgtactgtgccaggatcatggactgaccccagaccaggtagtcgcaatcgcgtcaaacggagggggaaagcaagccctggaaaccgtgcaaaggttgttgccggtcctttgtcaagaccacggccttacaccggagcaagtcgtggccattgcatcccacgacggtggcaaacaggctcttgagacggttcagagacttctcccagttctctgtcaagcccacgggctgactcccgatcaagttgtagcgattgcgaataacaatggagggaaacaagcattggagactgtccaacggctccttcccgtgttgtgtcaagcccacggtttgacgcctgcacaagtggtcgccatcgcctcgaatggcggcggtaagcaggcgctggaaacagtacagcgcctgctgcctgtactgtgccaggatcatggactgaccccagaccaggtagtcgcaatcgcgaacaataatgggggaaagcaagccctggaaaccgtgcaaaggttgttgccggtcctttgtcaagaccacggccttacaccggagcaagtcgtggccattgcatcccacgacggtggcaaacaggctcttgagacggttcagagacttctcccagttctctgtcaagcccacgggctgactcccgatcaagttgtagcgattgcgtccaacggtggagggaaacaagcattggagactgtccaacggctccttcccgtgttgtgtcaagcccacggtttgacgcctgcacaagtggtcgccatcgccaacaacaacggcggtaagcaggcgctggaaacagtacagcgcctgctgcctgtactgtgccaggatcatggactgacacccgaacaggtggtcgccattgcttcccacgacggaggacggccagccttggagtccatcgtagcccaattgtccaggcccgatcccgcgttggctgcgttaacgaatgaccatctggtggcgttggcatgtcttggtggacgacccgcgctcgatgcagtcaaaaagggtctgcctcatgctcccgcattgatcaaaagaaccaaccggcggattcccgagagaacttcccatcgagtcgcgggatcc

SEQ ID NO: 30 - protein, 805 aa, Artificial Sequence
  Description of Artificial Sequence: Synthetic polypeptide
MDYKDHDGDYKDHDIDYKDDDDKMAPKKKRKVGIHRGVPMVDLRTLGYSQQQQEKIKPKVRSTVAQHHEALVGHGFTHAHIVALSQHPAALGTVAVKYQDMIAALPEATHEAIVGVGKQWSGARALEALLTVAGELRGPPLQLDTGQLLKIAKRGGVTAVEAVHAWRNALTGAPLNLTPDQVVAIASNGGGKQALETVQRLLPVLCQDHGLTPEQVVAIANNNGGKQALETVQRLLPVLCQAHGLTPDQVVAIASNIGGKQALETVQRLLPVLCQAHGLTPAQVVAIASNIGGKQALETVQRLLPVLCQDHGLTPDQVVAIANNNGGKQALETVQRLLPVLCQDHGLTPEQVVAIASNIGGKQALETVQRLLPVLCQAHGLTPDQVVAIASNIGGKQALETVQRLLPVLCQAHGLTPAQVVAIANNNGGKQALETVQRLLPVLCQDHGLTPDQVVAIASNGGGKQALETVQRLLPVLCQDHGLTPEQVVAIASHDGGKQALETVQRLLPVLCQAHGLTPDQVVAIANNNGGKQALETVQRLLPVLCQAHGLTPAQVVAIASNGGGKQALETVQRLLPVLCQDHGLTPDQVVAIANNNGGKQALETVQRLLPVLCQDHGLTPEQVVAIASHDGGKQALETVQRLLPVLCQAHGLTPDQVVAIASNGGGKQALETVQRLLPVLCQAHGLTPAQVVAIANNNGGKQALETVQRLLPVLCQDHGLTPEQVVAIASHDGGRPALESIVAQLSRPDPALAALTNDHLVALACLGGRPALDAVKKGLPHAPALIKRTNRRIPERTSHRVAGS

SEQ ID NO: 31 - DNA, 2430 bp, Artificial Sequence
  Description of Artificial Sequence: Synthetic polynucleotide
tctagagctagcaccatggactacaaagaccatgacggtgattataaagatcatgacatcgattacaaggatgacgatgacaagatggcccccaagaagaagaggaaggtgggcattcaccgcggggtacctatggtggacttgaggacactcggttattcgcaacagcaacaggagaaaatcaagcctaaggtcaggagcaccgtcgcgcaacaccacgaggcgcttgtggggcatggcttcactcatgcgcatattgtcgcgctttcacagcaccctgcggcgcttgggacggtggctgtcaaataccaagatatgattgcggccctgcccgaagccacgcacgaggcaattgtaggggtcggtaaacagtggtcgggagcgcgagcacttgaggcgctgctgactgtggcgggtgagcttagggggcctccgctccagctcgacaccgggcagctgctgaagatcgcgaagagagggggagtaacagcggtagaggcagtgcacgcctggcgcaatgcgctcaccggggcccccttgaacctgaccccagaccaggtagtcgcaatcgcgaacaataatgggggaaagcaagccctggaaaccgtgcaaaggttgttgccggtcctttgtcaagaccacggccttacaccggagcaagtcgtggccattgcaagcaacatcggtggcaaacaggctcttgagacggttcagagacttctcccagttctctgtcaagcccacgggctgactcccgatcaagttgtagcgattgcgtcgaacattggagggaaacaagcattggagactgtccaacggctccttcccgtgttgtgtcaagcccacggtttgacgcctgcacaagtggtcgccatcgccaacaacaacggcggtaagcaggcgctggaaacagtacagcgcctgctgcctgtactgtgccaggatcatggactgaccccagaccaggtagtcgcaatcgcgtcgaacattgggggaaagcaagccctggaaaccgtgcaaaggttgttgccggtcctttgtcaagaccacggccttacaccggagcaagtcgtggccattgcaagcaacatcggtggcaaacaggctcttgagacggttcagagacttctcccagttctctgtcaagcccacgggctgactcccgatcaagttgtagcgattgcgaataacaatggagggaaacaagcattggagactgtccaacggctccttcccgtgttgtgtcaagcccacggtttgacgcctgcacaagtggtcgccatcgcctcgaatggcggcggtaagcaggcgctggaaacagtacagcgcctgctgcctgtactgtgccaggatcatggactgaccccagaccaggtagtcgcaatcgcgtcacatgacgggggaaagcaagccctggaaaccgtgcaaaggttgttgccggtcctttgtcaagaccacggccttacaccggagcaagtcgtggccattgcaaataataacggtggcaaacaggctcttgagacggttcagagacttctcccagttctctgtcaagcccacgggctgactcccgatcaagttgtagcgattgcgtccaacggtggagggaaacaagcattggagactgtccaacggctccttcccgtgttgtgtcaagcccacggtttgacgcctgcacaagtggtcgccatcgccaacaacaacggcggtaagcaggcgctggaaacagtacagcgcctgctgcctgtactgtgccaggatcatggactgaccccagaccaggtagtcgcaatcgcgtcacatgacgggggaaagcaagccctggaaaccgtgcaaaggttgttgccggtcctttgtcaagaccacggccttacaccggagcaagtcgtggccattgcaagcaatgggggtggcaaacaggctcttgagacggttcagagacttctcccagttctctgtcaagcccacgggctgactcccgatcaagttgtagcgattgcgaataacaatggagggaaacaagcattggagactgtccaacggctccttcccgtgttgtgtcaagcccacggtttgacgcctgcacaagtggtcgccatcgccagccatgatggcggtaagcaggcgctggaaacagtacagcgcctgctgcctgtactgtgccaggatcatggactgacacccgaacaggtggtcgccattgcttctaatgggggaggacggccagccttggagtccatcgtagcccaattgtccaggcccgatcccgcgttggctgcgttaacgaatgaccatctggtggcgttggcatgtcttggtggacgacccgcgctcgatgcagtcaaaaagggtctgcctcatgctcccgcattgatcaaaagaaccaaccggcggattcccgagagaacttcccatcgagtcgcgggatcc

SEQ ID NO: 32 - protein, 805 aa, Artificial Sequence
  Description of Artificial Sequence: Synthetic polypeptide
MDYKDHDGDYKDHDIDYKDDDDKMAPKKKRKVGIHRGVPMVDLRTLGYSQQQQEKIKPKVRSTVAQHHEALVGHGFTHAHIVALSQHPAALGTVAVKYQDMIAALPEATHEAIVGVGKQWSGARALEALLTVAGELRGPPLQLDTGQLLKIAKRGGVTAVEAVHAWRNALTGAPLNLTPDQVVAIANNNGGKQALETVQRLLPVLCQDHGLTPEQVVAIASNIGGKQALETVQRLLPVLCQAHGLTPDQVVAIASNIGGKQALETVQRLLPVLCQAHGLTPAQVVAIANNNGGKQALETVQRLLPVLCQDHGLTPDQVVAIASNIGGKQALETVQRLLPVLCQDHGLTPEQVVAIASNIGGKQALETVQRLLPVLCQAHGLTPDQVVAIANNNGGKQALETVQRLLPVLCQAHGLTPAQVVAIASNGGGKQALETVQRLLPVLCQDHGLTPDQVVAIASHDGGKQALETVQRLLPVLCQDHGLTPEQVVAIANNNGGKQALETVQRLLPVLCQAHGLTPDQVVAIASNGGGKQALETVQRLLPVLCQAHGLTPAQVVAIANNNGGKQALETVQRLLPVLCQDHGLTPDQVVAIASHDGGKQALETVQRLLPVLCQDHGLTPEQVVAIASNGGGKQALETVQRLLPVLCQAHGLTPDQVVAIANNNGGKQALETVQRLLPVLCQAHGLTPAQVVAIASHDGGKQALETVQRLLPVLCQDHGLTPEQVVAIASNGGGRPALESIVAQLSRPDPALAALTNDHLVALACLGGRPALDAVKKGLPHAPALIKRTNRRIPERTSHRVAGS

SEQ ID NO: 33 - DNA, 2328 bp, Artificial Sequence
  Description of Artificial Sequence: Synthetic polynucleotide
tctagagctagcaccatggactacaaagaccatgacggtgattataaagatcatgacatcgattacaaggatgacgatgacaagatggcccccaagaagaagaggaaggtgggcattcaccgcggggtacctatggtggacttgaggacactcggttattcgcaacagcaacaggagaaaatcaagcctaaggtcaggagcaccgtcgcgcaacaccacgaggcgcttgtggggcatggcttcactcatgcgcatattgtcgcgctttcacagcaccctgcggcgcttgggacggtggctgtcaaataccaagatatgattgcggccctgcccgaagccacgcacgaggcaattgtaggggtcggtaaacagtggtcgggagcgcgagcacttgaggcgctgctgactgtggcgggtgagcttagggggcctccgctccagctcgacaccgggcagctgctgaagatcgcgaagagagggggagtaacagcggtagaggcagtgcacgcctggcgcaatgcgctcaccggggcccccttgaacctgaccccagaccaggtagtcgcaatcgcgtcacatgacgggggaaagcaagccctggaaaccgtgcaaaggttgttgccggtcctttgtcaagaccacggccttacaccggagcaagtcgtggccattgcaaataataacggtggcaaacaggctcttgagacggttcagagacttctcccagttctctgtcaagcccacgggctgactcccgatcaagttgtagcgattgcgtcgaacattggagggaaacaagcattggagactgtccaacggctccttcccgtgttgtgtcaagcccacggtttgacgcctgcacaagtggtcgccatcgccaacaacaacggcggtaagcaggcgctggaaacagtacagcgcctgctgcctgtactgtgccaggatcatggactgaccccagaccaggtagtcgcaatcgcgtcacatgacgggggaaagcaagccctggaaaccgtgcaaaggttgttgccggtcctttgtcaagaccacggccttacaccggagcaagtcgtggccattgcaagcaatgggggtggcaaacaggctcttgagacggttcagagacttctcccagttctctgtcaagcccacgggctgactcccgatcaagttgtagcgattgcgaataacaatggagggaaacaagcattggagactgtccaacggctccttcccgtgttgtgtcaagcccacggtttgacgcctgcacaagtggtcgccatcgcctccaatattggcggtaagcaggcgctggaaacagtacagcgcctgctgcctgtactgtgccaggatcatggactgaccccagaccaggtagtcgcaatcgcgtcgaacattgggggaaagcaagccctggaaaccgtgcaaaggttgttgccggtcctttgtcaagaccacggccttacaccggagcaagtcgtggccattgcaaataataacggtggcaaacaggctcttgagacggttcagagacttctcccagttctctgtcaagcccacgggctgactcccgatcaagttgtagcgattgcgaataacaatggagggaaacaagcattggagactgtccaacggctccttcccgtgttgtgtcaagcccacggtttgacgcctgcacaagtggtcgccatcgccaacaacaacggcggtaagcaggcgctggaaacagtacagcgcctgctgcctgtactgtgccaggatcatggactgaccccagaccaggtagtcgcaatcgcgtcacatgacgggggaaagcaagccctggaaaccgtgcaaaggttgttgccggtcctttgtcaagaccacggccttacaccggagcaagtcgtggccattgcaagcaacatcggtggcaaacaggctcttgagacggttcagagacttctcccagttctctgtcaagcccacgggctgactcccgatcaagttgtagcgattgcgtccaacggtggagggaaacaagcattggagactgtccaacggctccttcccgtgttgtgtcaagcccacggtctgacacccgaacaggtggtcgccattgcttcccacgacggaggacggccagccttggagtccatcgtagcccaattgtccaggcccgatcccgcgttggctgcgttaacgaatgaccatctggtggcgttggcatgtcttggtggacgacccgcgctcgatgcagtcaaaaagggtctgcctcatgctcccgcattgatcaaaagaaccaaccggcggattcccgagagaacttcccatcgagtcgcgggatcc

SEQ ID NO: 34 - protein, 771 aa, Artificial Sequence
  Description of Artificial Sequence: Synthetic polypeptide
MDYKDHDGDYKDHDIDYKDDDDKMAPKKKRKVGIHRGVPMVDLRTLGYSQQQQEKIKPKVRSTVAQHHEALVGHGFTHAHIVALSQHPAALGTVAVKYQDMIAALPEATHEAIVGVGKQWSGARALEALLTVAGELRGPPLQLDTGQLLKIAKRGGVTAVEAVHAWRNALTGAPLNLTPDQVVAIASHDGGKQALETVQRLLPVLCQDHGLTPEQVVAIANNNGGKQALETVQRLLPVLCQAHGLTPDQVVAIASNIGGKQALETVQRLLPVLCQAHGLTPAQVVAIANNNGGKQALETVQRLLPVLCQDHGLTPDQVVAIASHDGGKQALETVQRLLPVLCQDHGLTPEQVVAIASNGGGKQALETVQRLLPVLCQAHGLTPDQVVAIANNNGGKQALETVQRLLPVLCQAHGLTPAQVVAIASNIGGKQALETVQRLLPVLCQDHGLTPDQVVAIASNIGGKQALETVQRLLPVLCQDHGLTPEQVVAIANNNGGKQALETVQRLLPVLCQAHGLTPDQVVAIANNNGGKQALETVQRLLPVLCQAHGLTPAQVVAIANNNGGKQALETVQRLLPVLCQDHGLTPDQVVAIASHDGGKQALETVQRLLPVLCQDHGLTPEQVVAIASNIGGKQALETVQRLLPVLCQAHGLTPDQVVAIASNGGGKQALETVQRLLPVLCQAHGLTPEQVVAIASHDGGRPALESIVAQLSRPDPALAALTNDHLVALACLGGRPALDAVKKGLPHAPALIKRTNRRIPERTSHRVAGS

SEQ ID NO: 35 - DNA, 2430 bp, Artificial Sequence
  Description of Artificial Sequence: Synthetic polynucleotide
tctagagctagcaccatggactacaaagaccatgacggtgattataaagatcatgacatcgattacaaggatgacgatgacaagatggcccccaagaagaagaggaaggtgggcattcaccgcggggtacctatggtggacttgaggacactcggttattcgcaacagcaacaggagaaaatcaagcctaaggtcaggagcaccgtcgcgcaacaccacgaggcgcttgtggggcatggcttcactcatgcgcatattgtcgcgctttcacagcaccctgcggcgcttgggacggtggctgtcaaataccaagatatgattgcggccctgcccgaagccacgcacgaggcaattgtaggggtcggtaaacagtggtcgggagcgcgagcacttgaggcgctgctgactgtggcgggtgagcttagggggcctccgctccagctcgacaccgggcagctgctgaagatcgcgaagagagggggagtaacagcggtagaggcagtgcacgcctggcgcaatgcgctcaccggggcccccttgaacctgaccccagaccaggtagtcgcaatcgcgtcacatgacgggggaaagcaagccctggaaaccgtgcaaaggttgttgccggtcctttgtcaagaccacggccttacaccggagcaagtcgtggccattgcaaataataacggtggcaaacaggctcttgagacggttcagagacttctcccagttctctgtcaagcccacgggctgactcccgatcaagttgtagcgattgcgtcgaacattggagggaaacaagcattggagactgtccaacggctccttcccgtgttgtgtcaagcccacggtttgacgcctgcacaagtggtcgccatcgccaacaacaacggcggtaagcaggcgctggaaacagtacagcgcctgctgcctgtactgtgccaggatcatggactgaccccagaccaggtagtcgcaatcgcgtcacatgacgggggaaagcaagccctggaaaccgtgcaaaggttgttgccggtcctttgtcaagaccacggccttacaccggagcaagtcgtggccattgcaagcaatgggggtggcaaacaggctcttgagacggttcagagacttctcccagttctctgtcaagcccacgggctgactcccgatcaagttgtagcgattgcgaataacaatggagggaaacaagcattggagactgtccaacggctccttcccgtgttgtgtcaagcccacggtttgacgcctgcacaagtggtcgccatcgcctccaatattggcggtaagcaggcgctggaaacagtacagcgcctgctgcctgtactgtgccaggatcatggactgaccccagaccaggtagtcgcaatcgcgtcgaacattgggggaaagcaagccctggaaaccgtgcaaaggttgttgccggtcctttgtcaagaccacggccttacaccggagcaagtcgtggccattgcaaataataacggtggcaaacaggctcttgagacggttcagagacttctcccagttctctgtcaagcccacgggctgactcccgatcaagttgtagcgattgcgaataacaatggagggaaacaagcattggagactgtccaacggctccttcccgtgttgtgtcaagcccacggtttgacgcctgcacaagtggtcgccatcgccaacaacaacggcggtaagcaggcgctggaaacagtacagcgcctgctgcctgtactgtgccaggatcatggactgaccccagaccaggtagtcgcaatcgcgtcacatgacgggggaaagcaagccctggaaaccgtgcaaaggttgttgccggtcctttgtcaagaccacggccttacaccggagcaagtcgtggccattgcaagcaacatcggtggcaaacaggctcttgagacggttcagagacttctcccagttctctgtcaagcccacgggctgactcccgatcaagttgtagcgattgcgtccaacggtggagggaaacaagcattggagactgtccaacggctccttcccgtgttgtgtcaagcccacggtttgacgcctgcacaagtggtcgccatcgccagccatgatggcggtaagcaggcgctggaaacagtacagcgcctgctgcctgtactgtgccaggatcatggactgacacccgaacaggtggtcgccattgctaataataacggaggacggccagccttggagtccatcgtagcccaattgtccaggcccgatcccgcgttggctgcgttaacgaatgaccatctggtggcgttggcatgtcttggtggacgacccgcgctcgatgcagtcaaaaagggtctgcctcatgctcccgcattgatcaaaagaaccaaccggcggattcccgagagaacttcccatcgagtcgcgggatcc

SEQ ID NO: 36 - protein, 805 aa, Artificial Sequence
  Description of Artificial Sequence: Synthetic polypeptide
MDYKDHDGDYKDHDIDYKDDDDKMAPKKKRKVGIHRGVPMVDLRTLGYSQQQQEKIKPKVRSTVAQHHEALVGHGFTHAHIVALSQHPAALGTVAVKYQDMIAALPEATHEAIVGVGKQWSGARALEALLTVAGELRGPPLQLDTGQLLKIAKRGGVTAVEAVHAWRNALTGAPLNLTPDQVVAIASHDGGKQALETVQRLLPVLCQDHGLTPEQVVAIANNNGGKQALETVQRLLPVLCQAHGLTPDQVVAIASNIGGKQALETVQRLLPVLCQAHGLTPAQVVAIANNNGGKQALETVQRLLPVLCQDHGLTPDQVVAIASHDGGKQALETVQRLLPVLCQDHGLTPEQVVAIASNGGGKQALETVQRLLPVLCQAHGLTPDQVVAIANNNGGKQALETVQRLLPVLCQAHGLTPAQVVAIASNIGGKQALETVQRLLPVLCQDHGLTPDQVVAIASNIGGKQALETVQRLLPVLCQDHGLTPEQVVAIANNNGGKQALETVQRLLPVLCQAHGLTPDQVVAIANNNGGKQALETVQRLLPVLCQAHGLTPAQVVAIANNNGGKQALETVQRLLPVLCQDHGLTPDQVVAIASHDGGKQALETVQRLLPVLCQDHGLTPEQVVAIASNIGGKQALETVQRLLPVLCQAHGLTPDQVVAIASNGGGKQALETVQRLLPVLCQAHGLTPAQVVAIASHDGGKQALETVQRLLPVLCQDHGLTPEQVVAIANNNGGRPALESIVAQLSRPDPALAALTNDHLVALACLGGRPALDAVKKGLPHAPALIKRTNRRIPERTSHRVAGS

SEQ ID NO: 37 - DNA, 2430 bp, Artificial Sequence
  Description of Artificial Sequence: Synthetic polynucleotide
tctagagctagcaccatggactacaaagaccatgacggtgattataaagatcatgacatcgattacaaggatgacgatgacaagatggcccccaagaagaagaggaaggtgggcattcaccgcggggtacctatggtggacttgaggacactcggttattcgcaacagcaacaggagaaaatcaagcctaaggtcaggagcaccgtcgcgcaacaccacgaggcgcttgtggggcatggcttcactcatgcgcatattgtcgcgctttcacagcaccctgcggcgcttgggacggtggctgtcaaataccaagatatgattgcggccctgcccgaagccacgcacgaggcaattgtaggggtcggtaaacagtggtcgggagcgcgagcacttgaggcgctgctgactgtggcgggtgagcttagggggcctccgctccagctcgacaccgggcagctgctgaagatcgcgaagagagggggagtaacagcggtagaggcagtgcacgcctggcgcaatgcgctcaccggggcccccttgaacctgaccccagaccaggtagtcgcaatcgcgtcaaacggagggggaaagcaagccctggaaaccgtgcaaaggttgttgccggtcctttgtcaagaccacggccttacaccggagcaagtcgtggccattgcaaataataacggtggcaaacaggctcttgagacggttcagagacttctcccagttctctgtcaagcccacgggctgactcccgatcaagttgtagcgattgcgtccaacggtggagggaaacaagcattggagactgtccaacggctccttcccgtgttgtgtcaagcccacggtttgacgcctgcacaagtggtcgccatcgccaacaacaacggcggtaagcaggcgctggaaacagtacagcgcctgctgcctgtactgtgccaggatcatggactgaccccagaccaggtagtcgcaatcgcgtcacatgacgggggaaagcaagccctggaaaccgtgcaaaggttgttgccggtcctttgtcaagaccacggccttacaccggagcaagtcgtggccattgcatcccacgacggtggcaaacaggctcttgagacggttcagagacttctcccagttctctgtcaagcccacgggctgactcccgatcaagttgtagcgattgcgtcgcatgacggagggaaacaagcattggagactgtccaacggctccttcccgtgttgtgtcaagcccacggtttgacgcctgcacaagtggtcgccatcgccagccatgatggcggtaagcaggcgctggaaacagtacagcgcctgctgcctgtactgtgccaggatcatggactgaccccagaccaggtagtcgcaatcgcgtcgaacattgggggaaagcaagccctggaaaccgtgcaaaggttgttgccggtcctttgtcaagaccacggccttacaccggagcaagtcgtggccattgcaaataataacggtggcaaacaggctcttgagacggttcagagacttctcccagttctctgtcaagcccacgggctgactcccgatcaagttgtagcgattgcgaataacaatggagggaaacaagcattggagactgtccaacggctccttcccgtgttgtgtcaagcccacggtttgacgcctgcacaagtggtcgccatcgcctccaatattggcggtaagcaggcgctggaaacagtacagcgcctgctgcctgtactgtgccaggatcatggactgaccccagaccaggtagtcgcaatcgcgtcaaacggagggggaaagcaagccctggaaaccgtgcaaaggttgttgccggtcctttgtcaagaccacggccttacaccggagcaagtcgtggccattgcaaataataacggtggcaaacaggctcttgagacggttcagagacttctcccagttctctgtcaagcccacgggctgactcccgatcaagttgtagcgattgcgtccaacggtggagggaaacaagcattggagactgtccaacggctccttcccgtgttgtgtcaagcccacggtttgacgcctgcacaagtggtcgccatcgcctcgaatggcggcggtaagcaggcgctggaaacagtacagcgcctgctgcctgtactgtgccaggatcatggactgacacccgaacaggtggtcgccattgctaataataacggaggacggccagccttggagtccatcgtagcccaattgtccaggcccgatcccgcgttggctgcgttaacgaatgaccatctggtggcgttggcatgtcttggtggacgacccgcgctcgatgcagtcaaaaagggtctgcctcatgctcccgcattgatcaaaagaaccaaccggcggattcccgagagaacttcccatcgagtcgcgggatcc

SEQ ID NO: 38 - protein, 805 aa, Artificial Sequence
  Description of Artificial Sequence: Synthetic polypeptide
MDYKDHDGDYKDHDIDYKDDDDKMAPKKKRKVGIHRGVPMVDLRTLGYSQQQQEKIKPKVRSTVAQHHEALVGHGFTHAHIVALSQHPAALGTVAVKYQDMIAALPEATHEAIVGVGKQWSGARALEALLTVAGELRGPPLQLDTGQLLKIAKRGGVTAVEAVHAWRNALTGAPLNLTPDQVVAIASNGGGKQALETVQRLLPVLCQDHGLTPEQVVAIANNNGGKQALETVQRLLPVLCQAHGLTPDQVVAIASNGGGKQALETVQRLLPVLCQAHGLTPAQVVAIANNNGGKQALETVQRLLPVLCQDHGLTPDQVVAIASHDGGKQALETVQRLLPVLCQDHGLTPEQVVAIASHDGGKQALETVQRLLPVLCQAHGLTPDQVVAIASHDGGKQALETVQRLLPVLCQAHGLTPAQVVAIASHDGGKQALETVQRLLPVLCQDHGLTPDQVVAIASNIGGKQALETVQRLLPVLCQDHGLTPEQVVAIANNNGGKQALETVQRLLPVLCQAHGLTPDQVVAIANNNGGKQALETVQRLLPVLCQAHGLTPAQVVAIASNIGGKQALETVQRLLPVLCQDHGLTPDQVVAIASNGGGKQALETVQRLLPVLCQDHGLTPEQVVAIANNNGGKQALETVQRLLPVLCQAHGLTPDQVVAIASNGGGKQALETVQRLLPVLCQAHGLTPAQVVAIASNGGGKQALETVQRLLPVLCQDHGLTPEQVVAIANNNGGRPALESIVAQLSRPDPALAALTNDHLVALACLGGRPALDAVKKGLPHAPALIKRTNRRIPERTSHRVAGS

SEQ ID NO: 39 - DNA, 2430 bp, Artificial Sequence
  Description of Artificial Sequence: Synthetic polynucleotide
tctagagctagcaccatggactacaaagaccatgacggtgattataaagatcatgacatcgattacaaggatgacgatgacaagatggcccccaagaagaagaggaaggtgggcattcaccgcggggtacctatggtggacttgaggacactcggttattcgcaacagcaacaggagaaaatcaagcctaaggtcaggagcaccgtcgcgcaacaccacgaggcgcttgtggggcatggcttcactcatgcgcatattgtcgcgctttcacagcaccctgcggcgcttgggacggtggctgtcaaataccaagatatgattgcggccctgcccgaagccacgcacgaggcaattgtaggggtcggtaaacagtggtcgggagcgcgagcacttgaggcgctgctgactgtggcgggtgagcttagggggcctccgctccagctcgacaccgggcagctgctgaagatcgcgaagagagggggagtaacagcggtagaggcagtgcacgcctggcgcaatgcgctcaccggggcccccttgaacctgaccccagaccaggtagtcgcaatcgcgaacaataatgggggaaagcaagccctggaaaccgtgcaaaggttgttgccggtcctttgtcaagaccacggccttacaccggagcaagtcgtggccattgcaagcaatgggggtggcaaacaggctcttgagacggttcagagacttctcccagttctctgtcaagcccacgggctgactcccgatcaagttgtagcgattgcgaataacaatggagggaaacaagcattggagactgtccaacggctccttcccgtgttgtgtcaagcccacggtttgacgcctgcacaagtggtcgccatcgccagccatgatggcggtaagcaggcgctggaaacagtacagcgcctgctgcctgtactgtgccaggatcatggactgaccccagaccaggtagtcgcaatcgcgtcacatgacgggggaaagcaagccctggaaaccgtgcaaaggttgttgccggtcctttgtcaagaccacggccttacaccggagcaagtcgtggccattgcatcccacgacggtggcaaacaggctcttgagacggttcagagacttctcccagttctctgtcaagcccacgggctgactcccgatcaagttgtagcgattgcgtcgcatgacggagggaaacaagcattggagactgtccaacggctccttcccgtgttgtgtcaagcccacggtttgacgcctgcacaagtggtcgccatcgcctccaatattggcggtaagcaggcgctggaaacagtacagcgcctgctgcctgtactgtgccaggatcatggactgaccccagaccaggtagtcgcaatcgcgaacaataatgggggaaagcaagccctggaaaccgtgcaaaggttgttgccggtcctttgtcaagaccacggccttacaccggagcaagtcgtggccattgcaaataataacggtggcaaacaggctcttgagacggttcagagacttctcccagttctctgtcaagcccacgggctgactcccgatcaagttgtagcgattgcgtcgaacattggagggaaacaagcattggagactgtccaacggctccttcccgtgttgtgtcaagcccacggtttgacgcctgcacaagtggtcgccatcgcctcgaatggcggcggtaagcaggcgctggaaacagtacagcgcctgctgcctgtactgtgccaggatcatggactgaccccagaccaggtagtcgcaatcgcgaacaataatgggggaaagcaagccctggaaaccgtgcaaaggttgttgccggtcctttgtcaagaccacggccttacaccggagcaagtcgtggccattgcaagcaatgggggtggcaaacaggctcttgagacggttcagagacttctcccagttctctgtcaagcccacgggctgactcccgatcaagttgtagcgattgcgtccaacggtggagggaaacaagcattggagactgtccaacggctccttcccgtgttgtgtcaagcccacggtttgacgcctgcacaagtggtcgccatcgccaacaacaacggcggtaagcaggcgctggaaacagtacagcgcctgctgcctgtactgtgccaggatcatggactgacacccgaacaggtggtcgccattgcttcccacgacggaggacggccagccttggagtccatcgtagcccaattgtccaggcccgatcccgcgttggctgcgttaacgaatgaccatctggtggcgttggcatgtcttggtggacgacccgcgctcgatgcagtcaaaaagggtctgcctcatgctcccgcattgatcaaaagaaccaaccggcggattcccgagagaacttcccatcgagtcgcgggatcc

SEQ ID NO: 40 - protein, 805 aa, Artificial Sequence
  Description of Artificial Sequence: Synthetic polypeptide
MDYKDHDGDYKDHDIDYKDDDDKMAPKKKRKVGIHRGVPMVDLRTLGYSQQQQEKIKPKVRSTVAQHHEALVGHGFTHAHIVALSQHPAALGTVAVKYQDMIAALPEATHEAIVGVGKQWSGARALEALLTVAGELRGPPLQLDTGQLLKIAKRGGVTAVEAVHAWRNALTGAPLNLTPDQVVAIANNNGGKQALETVQRLLPVLCQDHGLTPEQVVAIASNGGGKQALETVQRLLPVLCQAHGLTPDQVVAIANNNGGKQALETVQRLLPVLCQAHGLTPAQVVAIASHDGGKQALETVQRLLPVLCQDHGLTPDQVVAIASHDGGKQALETVQRLLPVLCQDHGLTPEQVVAIASHDGGKQALETVQRLLPVLCQAHGLTPDQVVAIASHDGGKQALETVQRLLPVLCQAHGLTPAQVVAIASNIGGKQALETVQRLLPVLCQDHGLTPDQVVAIANNNGGKQALETVQRLLPVLCQDHGLTPEQVVAIANNNGGKQALETVQRLLPVLCQAHGLTPDQVVAIASNIGGKQALETVQRLLPVLCQAHGLTPAQVVAIASNGGGKQALETVQRLLPVLCQDHGLTPDQVVAIANNNGGKQALETVQRLLPVLCQDHGLTPEQVVAIASNGGGKQALETVQRLLPVLCQAHGLTPDQVVAIASNGGGKQALETVQRLLPVLCQAHGLTPAQVVAIANNNGGKQALETVQRLLPVLCQDHGLTPEQVVAIASHDGGRPALESIVAQLSRPDPALAALTNDHLVALACLGGRPALDAVKKGLPHAPALIKRTNRRIPERTSHRVAGS

SEQ ID NO: 41 - DNA, 16 bp, Homo sapiens
gcagtgcttcagccgc

SEQ ID NO: 42 - DNA, 24 bp, Artificial Sequence
  Description of Artificial Sequence: Synthetic primer
tctagagaagacaagaacctgacc

SEQ ID NO: 43 - DNA, 24 bp, Artificial Sequence
  Description of Artificial Sequence: Synthetic primer
  5'-biotin
ggatccggtctcttaaggccgtgg

SEQ ID NO: 44 - DNA, 16 bp, Homo sapiens
gcagtgcttcagccgc

SEQ ID NO: 45 - DNA, 9 bp, Artificial Sequence
  Description of Artificial Sequence: Synthetic oligonucleotide
tctaacatc

SEQ ID NO: 46 - DNA, 9 bp, Artificial Sequence
  Description of Artificial Sequence: Synthetic oligonucleotide
tcccacgac

SEQ ID NO: 47 - DNA, 9 bp, Artificial Sequence
  Description of Artificial Sequence: Synthetic oligonucleotide
aataataac

SEQ ID NO: 48 - DNA, 9 bp, Artificial Sequence
  Description of Artificial Sequence: Synthetic oligonucleotide
tccaataaa

SEQ ID NO: 49 - DNA, 9 bp, Artificial Sequence
  Description of Artificial Sequence: Synthetic oligonucleotide
tctaatggg

SEQ ID NO: 50 - DNA, 17 bp, Homo sapiens
tgcagtgcttcagccgc

SEQ ID NO: 51 - DNA, 18 bp, Homo sapiens
tgcagtgcttcagccgct

SEQ ID NO: 52 - DNA, 18 bp, Homo sapiens
ttgaagaagtcgtgctgc

SEQ ID NO: 53 - DNA, 18 bp, Homo sapiens
tgaagaagtcgtgctgct

SEQ ID NO: 54 - DNA, 17 bp, Homo sapiens
tcgagctgaagggcatc

SEQ ID NO: 55 - DNA, 18 bp, Homo sapiens
tcgagctgaagggcatcg

SEQ ID NO: 56 - DNA, 18 bp, Homo sapiens
ttgtgccccaggatgttg

SEQ ID NO: 57 - DNA, 18 bp, Homo sapiens
tgtgccccaggatgttgc

SEQ ID NO: 58 - DNA, 137 bp, Artificial Sequence
  Description of Artificial Sequence: Synthetic polynucleotide
tctagagaagacaagaacctgaccccagaccaggtagtcgcaatcgcgtcgaacattgggggaaagcaagccctggaaaccgtgcaaaggttgttgccggtcctttgtcaagaccacggccttaagagaccggatcc

SEQ ID NO: 59 - DNA, 137 bp, Artificial Sequence
  Description of Artificial Sequence: Synthetic polynucleotide
tctagagaagacaagaacctgaccccagaccaggtagtcgcaatcgcgtcacatgacgggggaaagcaagccctggaaaccgtgcaaaggttgttgccggtcctttgtcaagaccacggccttaagagaccggatcc

SEQ ID NO: 60 - DNA, 137 bp, Artificial Sequence
  Description of Artificial Sequence: Synthetic polynucleotide
tctagagaagacaagaacctgaccccagaccaggtagtcgcaatcgcgtcgaacaaagggggaaagcaagccctggaaaccgtgcaaaggttgttgccggtcctttgtcaagaccacggccttaagagaccggatcc

SEQ ID NO: 61 - DNA, 137 bp, Artificial Sequence
  Description of Artificial Sequence: Synthetic polynucleotide
tctagagaagacaagaacctgaccccagaccaggtagtcgcaatcgcgaacaataatgggggaaagcaagccctggaaaccgtgcaaaggttgttgccggtcctttgtcaagaccacggccttaagagaccggatcc

SEQ ID NO: 62 - DNA, 137 bp, Artificial Sequence
  Description of Artificial Sequence: Synthetic polynucleotide
tctagagaagacaagaacctgaccccagaccaggtagtcgcaatcgcgtcaaacggagggggaaagcaagccctggaaaccgtgcaaaggttgttgccggtcctttgtcaagaccacggccttaagagaccggatcc

SEQ ID NO: 63 - DNA, 133 bp, Artificial Sequence
  Description of Artificial Sequence: Synthetic polynucleotide
tctagagaagacaacttacaccggagcaagtcgtggccattgcaagcaacatcggtggcaaacaggctcttgagacggttcagagacttctcccagttctctgtcaagcccacgggctgaagagaccggatcc

SEQ ID NO: 64 - DNA, 133 bp, Artificial Sequence
  Description of Artificial Sequence: Synthetic polynucleotide
tctagagaagacaacttacaccggagcaagtcgtggccattgcatcccacgacggtggcaaacaggctcttgagacggttcagagacttctcccagttctctgtcaagcccacgggctgaagagaccggatcc

SEQ ID NO: 65 - DNA, 133 bp, Artificial Sequence
  Description of Artificial Sequence: Synthetic polynucleotide
tctagagaagacaacttacaccggagcaagtcgtggccattgcatcaaataaaggtggcaaacaggctcttgagacggttcagagacttctcccagttctctgtcaagcccacgggctgaagagaccggatcc

SEQ ID NO: 66 - DNA, 133 bp, Artificial Sequence
  Description of Artificial Sequence: Synthetic polynucleotide
tctagagaagacaacttacaccggagcaagtcgtggccattgcaaataataacggtggcaaacaggctcttgagacggttcagagacttctcccagttctctgtcaagcccacgggctgaagagaccggatcc

SEQ ID NO: 67 - DNA, 133 bp, Artificial Sequence
  Description of Artificial Sequence: Synthetic polynucleotide
tctagagaagacaacttacaccggagcaagtcgtggccattgcaagcaatgggggtggcaaacaggctcttgagacggttcagagacttctcccagttctctgtcaagcccacgggctgaagagaccggatcc

SEQ ID NO: 68 - DNA, 133 bp, Artificial Sequence
  Description of Artificial Sequence: Synthetic polynucleotide
tctagagaagacaactgactcccgatcaagttgtagcgattgcgtcgaacattggagggaaacaagcattggagactgtccaacggctccttcccgtgttgtgtcaagcccacggtttgaagagaccggatcc

SEQ ID NO: 69 - DNA, 133 bp, Artificial Sequence
  Description of Artificial Sequence: Synthetic polynucleotide
tctagagaagacaactgactcccgatcaagttgtagcgattgcgtcgcatgacggagggaaacaagcattggagactgtccaacggctccttcccgtgttgtgtcaagcccacggtttgaagagaccggatcc

SEQ ID NO: 70 - DNA, 133 bp, Artificial Sequence
  Description of Artificial Sequence: Synthetic polynucleotide
tctagagaagacaactgactcccgatcaagttgtagcgattgcgtccaacaagggagggaaacaagcattggagactgtccaacggctccttcccgtgttgtgtcaagcccacggtttgaagagaccggatcc

SEQ ID NO: 71 - DNA, 133 bp, Artificial Sequence
  Description of Artificial Sequence: Synthetic polynucleotide
tctagagaagacaactgactcccgatcaagttgtagcgattgcgaataacaatggagggaaacaagcattggagactgtccaacggctccttcccgtgttgtgtcaagcccacggtttgaagagaccggatcc

SEQ ID NO: 72 - DNA, 133 bp, Artificial Sequence
  Description of Artificial Sequence: Synthetic polynucleotide
tctagagaagacaactgactcccgatcaagttgtagcgattgcgtccaacggtggagggaaacaagcattggagactgtccaacggctccttcccgtgttgtgtcaagcccacggtttgaagagaccggatcc

SEQ ID NO: 73 - DNA, 133 bp, Artificial Sequence
  Description of Artificial Sequence: Synthetic polynucleotide
tctagagaagacaattgacgcctgcacaagtggtcgccatcgcctccaatattggcggtaagcaggcgctggaaacagtacagcgcctgctgcctgtactgtgccaggatcatggactgaagagaccggatcc

SEQ ID NO: 74 - DNA, 133 bp, Artificial Sequence
  Description of Artificial Sequence: Synthetic polynucleotide
tctagagaagacaattgacgcctgcacaagtggtcgccatcgccagccatgatggcggtaagcaggcgctggaaacagtacagcgcctgctgcctgtactgtgccaggatcatggactgaagagaccggatcc

SEQ ID NO: 75 - DNA, 133 bp, Artificial Sequence
  Description of Artificial Sequence: Synthetic polynucleotide
tctagagaagacaattgacgcctgcacaagtggtcgccatcgccagcaataagggcggtaagcaggcgctggaaacagtacagcgcctgctgcctgtactgtgccaggatcatggactgaagagaccggatcc

SEQ ID NO: 76 - DNA, 133 bp, Artificial Sequence
  Description of Artificial Sequence: Synthetic polynucleotide
tctagagaagacaattgacgcctgcacaagtggtcgccatcgccaacaacaacggcggtaagcaggcgctggaaacagtacagcgcctgctgcctgtactgtgccaggatcatggactgaagagaccggatcc

SEQ ID NO: 77 - DNA, 133 bp, Artificial Sequence
  Description of Artificial Sequence: Synthetic polynucleotide
tctagagaagacaattgacgcctgcacaagtggtcgccatcgcctcgaatggcggcggtaagcaggcgctggaaacagtacagcgcctgctgcctgtactgtgccaggatcatggactgaagagaccggatcc

SEQ ID NO: 78 - DNA, 133 bp, Artificial Sequence
  Description of Artificial Sequence: Synthetic polynucleotide
tctagagaagacaactgaccccagaccaggtagtcgcaatcgcgtcgaacattgggggaaagcaagccctggaaaccgtgcaaaggttgttgccggtcctttgtcaagaccacggccttaagagaccggatcc

SEQ ID NO: 79 - DNA, 133 bp, Artificial Sequence
  Description of Artificial Sequence: Synthetic polynucleotide
tctagagaagacaactgaccccagaccaggtagtcgcaatcgcgtcacatgacgggggaaagcaagccctggaaaccgtgcaaaggttgttgccggtcctttgtcaagaccacggccttaagagaccggatcc

SEQ ID NO: 80 - DNA, 133 bp, Artificial Sequence
  Description of Artificial Sequence: Synthetic polynucleotide
tctagagaagacaactgaccccagaccaggtagtcgcaatcgcgtcgaacaaagggggaaagcaagccctggaaaccgtgcaaaggttgttgccggtcctttgtcaagaccacggccttaagagaccggatcc

SEQ ID NO: 81 - DNA, 133 bp, Artificial Sequence
  Description of Artificial Sequence: Synthetic polynucleotide
tctagagaagacaactgaccccagaccaggtagtcgcaatcgcgaacaataatgggggaaagcaagccctggaaaccgtgcaaaggttgttgccggtcctttgtcaagaccacggccttaagagaccggatcc

SEQ ID NO: 82 - DNA, 133 bp, Artificial Sequence
  Description of Artificial Sequence: Synthetic polynucleotide
tctagagaagacaactgaccccagaccaggtagtcgcaatcgcgtcaaacggagggggaaagcaagccctggaaaccgtgcaaaggttgttgccggtcctttgtcaagaccacggccttaagagaccggatcc

SEQ ID NO: 83 - DNA, 133 bp, Artificial Sequence
  Description of Artificial Sequence: Synthetic polynucleotide
tctagagaagacaactgactcccgatcaagttgtagcgattgcgtcgaacattggagggaaacaagcattggagactgtccaacggctccttcccgtgttgtgtcaagcccacggtctgaagagaccggatcc

SEQ ID NO: 84 - DNA, 133 bp, Artificial Sequence
  Description of Artificial Sequence: Synthetic polynucleotide
tctagagaagacaactgactcccgatcaagttgtagcgattgcgtcgcatgacggagggaaacaagcattggagactgtccaacggctccttcccgtgttgtgtcaagcccacggtctgaagagaccggatcc

SEQ ID NO: 85 - DNA, 133 bp, Artificial Sequence
  Description of Artificial Sequence: Synthetic polynucleotide
tctagagaagacaactgactcccgatcaagttgtagcgattgcgtccaacaagggagggaaacaagcattggagactgtccaacggctccttcccgtgttgtgtcaagcccacggtctgaagagaccggatcc

SEQ ID NO: 86 - DNA, 133 bp, Artificial Sequence
  Description of Artificial Sequence: Synthetic polynucleotide
tctagagaagacaactgactcccgatcaagttgtagcgattgcgaataacaatggagggaaacaagcattggagactgtccaacggctccttcccgtgttgtgtcaagcccacggtctgaagagaccggatcc

SEQ ID NO: 87 - DNA, 133 bp, Artificial Sequence
  Description of Artificial Sequence: Synthetic polynucleotide
tctagagaagacaactgactcccgatcaagttgtagcgattgcgtccaacggtggagggaaacaagcattggagactgtccaacggctccttcccgtgttgtgtcaagcccacggtctgaagagaccggatcc

SEQ ID NO: 88 - DNA, 133 bp, Artificial Sequence
  Description of Artificial Sequence: Synthetic polynucleotide
tctagagaagacaactgaccccagaccaggtagtcgcaatcgcgtcgaacattgggggaaagcaagccctggaaaccgtgcaaaggttgttgccggtcctttgtcaagaccacggcctgaagagaccggatcc

SEQ ID NO: 89 - DNA, 133 bp, Artificial Sequence
  Description of Artificial Sequence: Synthetic polynucleotide
tctagagaagacaactgaccccagaccaggtagtcgcaatcgcgtcacatgacgggggaaagcaagccctggaaaccgtgcaaaggttgttgccggtcctttgtcaagaccacggcctgaagagaccggatcc

SEQ ID NO: 90 - DNA, 133 bp, Artificial Sequence
  Description of Artificial Sequence: Synthetic polynucleotide
tctagagaagacaactgaccccagaccaggtagtcgcaatcgcgtcgaacaaagggggaaagcaagccctggaaaccgtgcaaaggttgttgccggtcctttgtcaagaccacggcctgaagagaccggatcc

SEQ ID NO: 91 - DNA, 133 bp, Artificial Sequence
  Description of Artificial Sequence: Synthetic polynucleotide
tctagagaagacaactgaccccagaccaggtagtcgcaatcgcgaacaataatgggggaaagcaagccctggaaaccgtgcaaaggttgttgccggtcctttgtcaagaccacggcctgaagagaccggatcc

SEQ ID NO: 92 - DNA, 133 bp, Artificial Sequence
  Description of Artificial Sequence: Synthetic polynucleotide
tctagagaagacaactgaccccagaccaggtagtcgcaatcgcgtcaaacggagggggaaagcaagccctggaaaccgtgcaaaggttgttgccggtcctttgtcaagaccacggcctgaagagaccggatcc

SEQ ID NO: 93 - DNA, 36 bp, Homo sapiens
tcgccaccatggtgagcaagggcgaggagctgttca

SEQ ID NO: 94 - DNA, 36 bp, Homo sapiens
tggtgcccatcctggtcgagctggacggcgacgtaa

SEQ ID NO: 95 - DNA, 36 bp, Homo sapiens
tctgcaccaccggcaagctgcccgtgccctggccca

SEQ ID NO: 96 - DNA, 36 bp, Homo sapiens
tggagtacaactacaacagccacaacgtctatatca

SEQ ID NO: 97 - DNA, 38 bp, Homo sapiens
ttcagcgtgtccggcgagggcgagggcgatgccaccta

SEQ ID NO: 98 - DNA, 38 bp, Homo sapiens
tgccacctacggcaagctgaccctgaagttcatctgca

SEQ ID NO: 99 - DNA, 38 bp, Homo sapiens
tggcccaccctcgtgaccaccctgacctacggcgtgca

SEQ ID NO: 100 - DNA, 38 bp, Homo sapiens
ttcaagatccgccacaacatcgaggacggcagcgtgca

SEQ ID NO: 101 - DNA, 40 bp, Homo sapiens
tagaggatccaccggtcgccaccatggtgagcaagggcga

SEQ ID NO: 102 - DNA, 40 bp, Homo sapiens
tccggcgagggcgagggcgatgccacctacggcaagctga

SEQ ID NO: 103 - DNA, 40 bp, Homo sapiens
tgacctacggcgtgcagtgcttcagccgctaccccgacca

SEQ ID NO: 104 - DNA, 40 bp, Homo sapiens
tccgccacaacatcgaggacggcagcgtgcagctcgccga

SEQ ID NO: 105 - DNA, 42 bp, Homo sapiens
tcctggtcgagctggacggcgacgtaaacggccacaagttca

SEQ ID NO: 106 - DNA, 42 bp, Homo sapiens
tcagccgctaccccgaccacatgaagcagcacgacttcttca

SEQ ID NO: 107 - DNA, 42 bp, Homo sapiens
tcttcaagtccgccatgcccgaaggctacgtccaggagcgca

SEQ ID NO: 108 - DNA, 42 bp, Homo sapiens
tcaaggaggacggcaacatcctggggcacaagctggagtaca

SEQ ID NO: 109 - DNA, 42 bp, Homo sapiens
tcaaggtgaacttcaagatccgccacaacatcgaggacggca

SEQ ID NO: 110 - DNA, 44 bp, Homo sapiens
tccaccggtcgccaccatggtgagcaagggcgaggagctgttca

SEQ ID NO: 111 - DNA, 44 bp, Homo sapiens
ttcagcgtgtccggcgagggcgagggcgatgccacctacggcaa

SEQ ID NO: 112 - DNA, 44 bp, Homo sapiens
ttcagccgctaccccgaccacatgaagcagcacgacttcttcaa

SEQ ID NO: 113 - DNA, 44 bp, Homo sapiens
tacaacagccacaacgtctatatcatggccgacaagcagaagaa

SEQ ID NO: 114 - DNA, 46 bp, Homo sapiens
tggtgcccatcctggtcgagctggacggcgacgtaaacggccacaa

SEQ ID NO: 115 - DNA, 46 bp, Homo sapiens
tgcccgaaggctacgtccaggagcgcaccatcttcttcaaggacga

SEQ ID NO: 116 - DNA, 46 bp, Homo sapiens
tgaaccgcatcgagctgaagggcatcgacttcaaggaggacggcaa

SEQ ID NO: 117 - DNA, 46 bp, Homo sapiens
tcaagatccgccacaacatcgaggacggcagcgtgcagctcgccga

SEQ ID NO: 118 - DNA, 48 bp, Homo sapiens
tgttcaccggggtggtgcccatcctggtcgagctggacggcgacgtaa

SEQ ID NO: 119 - DNA, 48 bp, Homo sapiens
tgcccatcctggtcgagctggacggcgacgtaaacggccacaagttca

SEQ ID NO: 120 - DNA, 48 bp, Homo sapiens
tgtccggcgagggcgagggcgatgccacctacggcaagctgaccctga

SEQ ID NO: 121 - DNA, 48 bp, Homo sapiens
tcatctgcaccaccggcaagctgcccgtgccctggcccaccctcgtga

SEQ ID NO: 122 - DNA, 48 bp, Homo sapiens
tctatatcatggccgacaagcagaagaacggcatcaaggtgaacttca

SEQ ID NO: 123 - DNA, 50 bp, Homo sapiens
tacggcgtgcagtgcttcagccgctaccccgaccacatgaagcagcacga

SEQ ID NO: 124 - DNA, 50 bp, Homo sapiens
taccccgaccacatgaagcagcacgacttcttcaagtccgccatgcccga

SEQ ID NO: 125 - DNA, 50 bp, Homo sapiens
tccgccatgcccgaaggctacgtccaggagcgcaccatcttcttcaagga

SEQ ID NO: 126 - DNA, 50 bp, Homo sapiens
ttcaaggaggacggcaacatcctggggcacaagctggagtacaactacaa

SEQ ID NO: 127 - DNA, 50 bp, Homo sapiens
tacaactacaacagccacaacgtctatatcatggccgacaagcagaagaa

SEQ ID NO: 128 - DNA, 52 bp, Homo sapiens
tcaccggggtggtgcccatcctggtcgagctggacggcgacgtaaacggcca

SEQ ID NO: 129 - DNA, 52 bp, Homo sapiens
taaacggccacaagttcagcgtgtccggcgagggcgagggcgatgccaccta

SEQ ID NO: 130 - DNA, 52 bp, Homo sapiens
tgcagtgcttcagccgctaccccgaccacatgaagcagcacgacttcttcaa

SEQ ID NO: 131 - DNA, 54 bp, Homo sapiens
tcagcgtgtccggcgagggcgagggcgatgccacctacggcaagctgaccctga

SEQ ID NO: 132 - DNA, 54 bp, Homo sapiens
tgaagttcatctgcaccaccggcaagctgcccgtgccctggcccaccctcgtga

SEQ ID NO: 133 - DNA, 54 bp, Homo sapiens
tcgtgaccaccctgacctacggcgtgcagtgcttcagccgctaccccgaccaca

SEQ ID NO: 134 - DNA, 54 bp, Homo sapiens
tcatggccgacaagcagaagaacggcatcaaggtgaacttcaagatccgccaca

SEQ ID NO: 135 - DNA, 56 bp, Homo sapiens
ttcaccggggtggtgcccatcctggtcgagctggacggcgacgtaaacggccacaa

SEQ ID NO: 136 - DNA, 56 bp, Homo sapiens
tgcaccaccggcaagctgcccgtgccctggcccaccctcgtgaccaccctgaccta

SEQ ID NO: 137 - DNA, 56 bp, Homo sapiens
ttcaagtccgccatgcccgaaggctacgtccaggagcgcaccatcttcttcaagga

SEQ ID NO: 138 - DNA, 56 bp, Homo sapiens
tatatcatggccgacaagcagaagaacggcatcaaggtgaacttcaagatccgcca

SEQ ID NO: 139 - DNA, 58 bp, Homo sapiens
ttcatctgcaccaccggcaagctgcccgtgccctggcccaccctcgtgaccaccctga

SEQ ID NO: 140 - DNA, 58 bp, Homo sapiens
tgaagttcgagggcgacaccctggtgaaccgcatcgagctgaagggcatcgacttcaa

SEQ ID NO: 141 - DNA, 52 bp, Homo sapiens
tacctattattactttatggggcagcagcctggaaaagtacttggggaccaa

SEQ ID NO: 142 - DNA, 52 bp, Homo sapiens
tgtgtcttgggatgagtgggtcagtgttctggtgctcacaggatggctggca

SEQ ID NO: 143 - DNA, 51 bp, Homo sapiens
tcctgtggctcctgccgctgctgctttccacggcagctgtgggctccggga

SEQ ID NO: 144 - DNA, 52 bp, Homo sapiens
tatgtacgcctccctgggctcgggtccggtcgcccctttgcccgcttctgta

SEQ ID NO: 145 - DNA, 54 bp, Homo sapiens
tgaattgggatgctgtttttaggtattctattcaaatttattttactgtcttta

SEQ ID NO: 146 - DNA, 52 bp, Homo sapiens
tccctcaccatgagtagcgctatgttggtgacttgcctcccggaccccagca

SEQ ID NO: 147 - DNA, 52 bp, Homo sapiens
tgtgcgatctccaagcactgaggggcagaaactcccggatcgggcgctgcca

SEQ ID NO: 148 - DNA, 52 bp, Homo sapiens
ttttcaagtgaagacaaaatggcctcgccggctgacagctgtatccagttca

SEQ ID NO: 149 - DNA, 53 bp, Homo sapiens
tacaattgaacaatgcctcagctatacatttacatcagattattgggagccta

SEQ ID NO: 150 - DNA, 52 bp, Homo sapiens
tccgaagctgacagatgggtattctttgacggggggtaggggcggaacctga

SEQ ID NO: 151 - DNA, 52 bp, Homo sapiens
ttagacttaggtaagtaatgcaatatggtagactggggagaactacaaacta

SEQ ID NO: 152 - DNA, 52 bp, Homo sapiens
tctgcaataaaaaatggcctccaacaaaactacattggtaagttaatgaaaa

SEQ ID NO: 153 - DNA, 52 bp, Homo sapiens
tggagctttcagcggtgggggagcgggtgttcgcggccgaagccctcctgaa

SEQ ID NO: 154 - DNA, 55 bp, Homo sapiens
tggaacaccagctcctgtgctgcgaagtggaaaccatccgccgcgcgtaccccga

SEQ ID NO: 155 - DNA, 52 bp, Homo sapiens
tgcttagcgtcctgcgacagtacaacatccagaagaaggagattgtggtgaa

SEQ ID NO: 156 - DNA, 52 bp, Homo sapiens
tgctgcaggtaccccggatcccctgacttgcgagggacgcattcgggccgca

SEQ ID NO: 157 - DNA, 49 bp, Homo sapiens
tcccttgatctgagaatggctacctctcgatatgagccagtggctgaaa

SEQ ID NO: 158 - DNA, 52 bp, Homo sapiens
tggcgtcgggcctgggctccccgtccccctgctcggcgggcagtgaggagga

SEQ ID NO: 159 - DNA, 52 bp, Homo sapiens
tgtgttggaagaagatggcagatccaggaatgatgagtctttttggcgagga

SEQ ID NO: 160 - DNA, 51 bp, Homo sapiens
tccagcgtggacaatggctactcaaggtttgtgtcattaaatctttagtta

SEQ ID NO: 161 - DNA, 54 bp, Homo sapiens
taatatcacaatgagttcaggcttatggagccaagaaaaagtcacttcacccta

SEQ ID NO: 162 - DNA, 50 bp, Homo sapiens
tcacacggaggacgcgatggctcccaagaaacgcccagaaacccagaaga

SEQ ID NO: 163 - DNA, 49 bp, Homo sapiens
tccggccggcgccatgaagtgagaagggggctgggggtcgcgctcgcta

SEQ ID NO: 164 - DNA, 55 bp, Homo sapiens
tccgggatcgccatgggaactcaatagaaaatcctcatcttctcactttgtttca

SEQ ID NO: 165 - DNA, 53 bp, Homo sapiens
tggcgtccacgggtgagtatggtggaactgcggtcgcgccggcggtagccgga

SEQ ID NO: 166 - DNA, 53 bp, Homo sapiens
tgacccaggcaggacacatgcaggccaaaaaacgctatttcatcctgctctca

SEQ ID NO: 167 - DNA, 52 bp, Homo sapiens
ttcctcccagggggatgtcctgcgcctcagggtccggtggtggcctgcggca

SEQ ID NO: 168 - DNA, 52 bp, Homo sapiens
tgcttttagaataatcatgggccagactgggaagaaatctgagaagggacca

SEQ ID NO: 169 - DNA, 52 bp, Homo sapiens
taggcgccaaggccatgtccgactcgtgggtcccgaactccgcctcgggcca

SEQ ID NO: 170 - DNA, 52 bp, Homo sapiens
tgaagggacatcaccttttcgctttttccaagatggctcaagattcagtaga

SEQ ID NO: 171 - DNA, 53 bp, Homo sapiens
tgccccggcatggcgacaccggacgcggggctccctggggctgagggcgtgga

SEQ ID NO: 172 - DNA, 50 bp, Homo sapiens
ttcgcgcacctcatggaatcccttctgcagcacctggatcgcttttccga

SEQ ID NO: 173 - DNA, 50 bp, Homo sapiens
tcggccaccatgtcccgccagaccacctctgtgggctccagctgcctgga

SEQ ID NO: 174 - DNA, 54 bp, Homo sapiens
tccccagaacagcactatgggcttctcttccgagctgtgcagcccccagggcca

SEQ ID NO: 175 - DNA, 51 bp, Homo sapiens
tctgctccccaccgaggacctctgcatgcaggcatgaatcccaggagccta

SEQ ID NO: 176 - DNA, 53 bp, Homo sapiens
tgtaccgagcacttcggctcctcgcgcgctcgcgtcccctcgtgcgggctcca

SEQ ID NO: 177 - DNA, 54 bp, Homo sapiens
tctccaaggcaccatgaatgccatcgtggctctctgccacttctgcgagctcca

SEQ ID NO: 178 - DNA, 56 bp, Homo sapiens
tccggaggccatgccggcgttggcgcgcgacggcggccagctgccgctgctcggta

SEQ ID NO: 179 - DNA, 55 bp, Homo sapiens
tgcagcggggcgccgcgctgtgcctgcgactgtggctctgcctgggactcctgga

SEQ ID NO: 180 - DNA, 49 bp, Homo sapiens
tcaccatggccgaggcgcctcaggtggtggagatcgacccggacttcga

SEQ ID NO: 181 - DNA, 54 bp, Homo sapiens
tctccgctcgaagtggagctggacccggagttcgagccccagagccgtccgcga

SEQ ID NO: 182 - DNA, 52 bp, Homo sapiens
tcctctgagacgccatgttcaactcgatgaccccaccaccaatcagtagcta

SEQ ID NO: 183 - DNA, 52 bp, Homo sapiens
tggcgcagacgcagggcacccggaggaaagtctgttactactacgacggtga

SEQ ID NO: 184 - DNA, 54 bp, Homo sapiens
tgcgctcacctccctgcggcctcctgaggtggtttggtggccccctcctcgcga

SEQ ID NO: 185 - DNA, 52 bp, Homo sapiens
tcctcaactatgacctcaaccggccaggattccaccacaaccaggcagcgaa

SEQ ID NO: 186 - DNA, 52 bp, Homo sapiens
tgagcgcacgcggtgagggcgcggggcagccgtccacttcagcccagggaca

SEQ ID NO: 187 - DNA, 53 bp, Homo sapiens
tccgtgctcctccacccccgctggatcgagcccaccgtcatgtttctctacga

SEQ ID NO: 188 - DNA, 49 bp, Homo sapiens
tgggcacggtgatggccaccactggggccctgggcaactactacgtgga

SEQ ID NO: 189 - DNA, 54 bp, Homo sapiens
tccagcagatcatgtcatgacgacttcgctgctcctgcatccacgctggccgga

SEQ ID NO: 190 - DNA, 52 bp, Homo sapiens
ttgacgagtgcggccagagcgcagccagcatgtacctgccgggctgcgccta

SEQ ID NO: 191 - DNA, 53 bp, Homo sapiens
tgcgggcagacggcgggggcgccggtggcgccccggcctcttcctcctcctca

SEQ ID NO: 192 - DNA, 52 bp, Homo sapiens
tctgaaaaagactctgcatgggaatggcctgccttacgatgacagaaatgga

SEQ ID NO: 193 - DNA, 55 bp, Homo sapiens
taccgcgatgagaggcgctcgcggcgcctgggattttctctgcgttctgctccta

SEQ ID NO: 194 - DNA, 52 bp, Homo sapiens
tgaaaatgactgaatataaacttgtggtagttggagctggtggcgtaggcaa

SEQ ID NO: 195 - DNA, 52 bp, Homo sapiens
tagggtccccggcgccaggccacccggccgtcagcagcatgcagggtaagga

SEQ ID NO: 196 - DNA, 52 bp, Homo sapiens
tccaagcgcgaaaaccccggatggtgaggagcaggtactggcccggcagcga

SEQ ID NO: 197 - DNA, 52 bp, Homo sapiens
ttattattacatggctttgccttactgaggcttcatcttgtcctctggtcca

SEQ ID NO: 198 - DNA, 52 bp, Homo sapiens
tctggcgccaaaatgtcgttcgtggcaggggttattcggcggctggacgaga

SEQ ID NO: 199 - DNA, 52 bp, Homo sapiens
tgaggaggtttcgacatggcggtgcagccgaaggagacgctgcagttggaga

SEQ ID NO: 200 - DNA, 54 bp, Homo sapiens
tcactgtcggcggccatgacaccgctcgtctcccgcctgagtcgtctgtgggta

SEQ ID NO: 201 - DNA, 52 bp, Homo sapiens
tgcttagacgctggatttttttcgggtagtggaaaaccaggtaagcaccgaa

SEQ ID NO: 202 - DNA, 52 bp, Homo sapiens
tcccgcagggagcggacatggactacgactcgtaccagcactatttctacga

SEQ ID NO: 203 - DNA, 50 bp, Homo sapiens
tgccgagctgctccacgtccaccatgccgggcatgatctgcaagaaccca

SEQ ID NO: 204 - DNA, 48 bp, Homo sapiens
tgaggagccggaccgatgtggaaactgctgcccgccgcgggcccggca

SEQ ID NO: 205 - DNA, 52 bp, Homo sapiens
tctttactgataatgtcaagttcatgttaccctcccaaccaaggagcattca

SEQ ID NO: 206 - DNA, 48 bp, Homo sapiens
tggagggccactgagccccgctacccgccccacagcctttcctaccca

SEQ ID NO: 207 - DNA, 52 bp, Homo sapiens
tcggcgcatgaaggaggtactcctcattttcgttctctctctctgtgcccca

SEQ ID NO: 208 - DNA, 52 bp, Homo sapiens
ttgcgctcggggcggccatgtcggccggcgaggtcgagcgcctagtgtcgga

SEQ ID NO: 209 - DNA, 52 bp, Homo sapiens
tctgcaggacaccatgcggcttccgggtgcgatgccagctctggccctcaaa

SEQ ID NO: 210 - DNA, 52 bp, Homo sapiens
tgagtactccgcctctaccccggctgaagcccgcccccgccgccacctatta

SEQ ID NO: 211 - DNA, 54 bp, Homo sapiens
tcgggtgttgcatccatggagcgagctgagagctcgaggtgagcggggctcgca

SEQ ID NO: 212 - DNA, 48 bp, Homo sapiens
tggaactgcttaatagaaacaggcttgtaattgtgagtccgcgctgca

SEQ ID NO: 213 - DNA, 51 bp, Homo sapiens
tcccagacatgacagccatcatcaaagagatcgttagcagaaacaaaagga

SEQ ID NO: 214 - DNA, 53 bp, Homo sapiens
tggcatggccagcaacagcagctcctgcccgacacctgggggcgggcacctca

SEQ ID NO: 215 - DNA, 52 bp, Homo sapiens
tgctgggtgagaagggctgtggctgcgttttagagaagcgttgggtactgga

SEQ ID NO: 216 - DNA, 52 bp, Homo sapiens
tgcgggacgtgcgggagcggctgcaggcgtgggagcgcgcgttccgacggca

SEQ ID NO: 217 - DNA, 52 bp, Homo sapiens
tcagaatacagttatggccacccaggtaatggggcagtcttctggaggagga

SEQ ID NO: 218 - DNA, 53 bp, Homo sapiens
tgagttctgccggccgccggctcccgcaggggccagggcgaagttggcgccga

SEQ ID NO: 219 - DNA, 52 bp, Homo sapiens
ttctttatttccagcaatgtctcaggctgtgcagacaaacggaactcaacca

SEQ ID NO: 220 - DNA, 52 bp, Homo sapiens
ttcaggaggaagcgatggcttcagacagcatatttgagtcatttccttcgta

SEQ ID NO: 221 - DNA, 52 bp, Homo sapiens
tctccttgaggcgccggttgccggccacaacccttggcggagcctgcctgca

SEQ ID NO: 222 - DNA, 54 bp, Homo sapiens
tgttgctgaggtgacttcagtgggactgggagttggtgcctgcggccctccgga

SEQ ID NO: 223 - DNA, 53 bp, Homo sapiens
tcaggaacgagatggcggttctctggaggctgagtgccgtttgcggtgcccta

SEQ ID NO: 224 - DNA, 52 bp, Homo sapiens
tgcagaggacaaaagcatgtcttcccttcctgggtgcattggtttggatgca

SEQ ID NO: 225 - DNA, 54 bp, Homo sapiens
ttacgcggcggggctgtcgccgtacgcggacaagggcaagtgcggcctcccgga

SEQ ID NO: 226 - DNA, 52 bp, Homo sapiens
tttggtaagaacatgtcgtccatcttgccattcacgccgccagttgtgaaga

SEQ ID NO: 227 - DNA, 53 bp, Homo sapiens
tggtgacggcggcaacatgtctgtggctttcgcggccccgaggcagcgaggca

SEQ ID NO: 228 - DNA, 48 bp, Homo sapiens
tggcgcctcagaagcacggcggtgggggagggggcggctcggggccca

SEQ ID NO: 229 - DNA, 52 bp, Homo sapiens
tcatgtctcatgcggccgaaccagctcgggatggcgtagaggccagcgcgga

SEQ ID NO: 230 - DNA, 53 bp, Homo sapiens
tcgggggctgctcaggggcctgtggccgctgcacatcgtcctgtggacgcgta

SEQ ID NO: 231 - DNA, 53 bp, Homo sapiens
ttccgcccgcccaggatggaggcgcccgccagcgcgcagaccccgcacccgca

SEQ ID NO: 232 - DNA, 53 bp, Homo sapiens
ttgccgtcccaagcaatggatgatttgatgctgtccccggacgatattgaaca

SEQ ID NO: 233 - DNA, 52 bp, Homo sapiens
tcctggtccaccatggccaaaccaacaagcaaagattcaggcttgaaggaga

SEQ ID NO: 234 - DNA, 52 bp, Homo sapiens
tctggatcgcggagggaatgccccggagggcggagaactgggacgaggccga

SEQ ID NO: 235 - DNA, 52 bp, Homo sapiens
tgggccagagatggcggcggccgacggggctttgccggaggcggcggcttta

SEQ ID NO: 236 - DNA, 55 bp, Homo sapiens
tgcccagacaagcaacatggctcggaaacgcgcggccggcggggagccgcgggga

SEQ ID NO: 237 - DNA, 24 bp, Artificial Sequence
  Description of Artificial Sequence: Synthetic primer
  5'-biotin
tctagagaagacaagaacctgacc

SEQ ID NO: 238 - DNA, 24 bp, Artificial Sequence
  Description of Artificial Sequence: Synthetic primer
ggatccggtctcttaaggccgtgg

SEQ ID NO: 239 - DNA, 28 bp, Artificial Sequence
  Description of Artificial Sequence: Synthetic primer
gacggtggctgtcaaataccaagatatg

SEQ ID NO: 240 - DNA, 30 bp, Artificial Sequence
  Description of Artificial Sequence: Synthetic primer
tctcctccagttcacttttgactagttggg

SEQ ID NO: 241 - DNA, 20 bp, Artificial Sequence
  Description of Artificial Sequence: Synthetic primer
agtaacagcggtagaggcag

SEQ ID NO: 242 - DNA, 20 bp, Artificial Sequence
  Description of Artificial Sequence: Synthetic primer
attgggctacgatggactcc

SEQ ID NO: 243 - DNA, 25 bp, Artificial Sequence
  Description of Artificial Sequence: Synthetic primer
ttaattcaatatattcatgaggcac

SEQ ID NO: 244 - DNA, 5656 bp, Artificial Sequence
  Description of Artificial Sequence: Synthetic polynucleotide
  modified_base (901)..(910): a, c, t, g, unknown or other
gacggatcgggagatctcccgatcccctatggtcgactctcagtacaatctgctctgatgccgcatagttaagccagtatctgctccctgcttgtgtgttggaggtcgctgagtagtgcgcgagcaaaatttaagctacaacaaggcaaggcttgaccgacaattgcatgaagaatctgcttagggttaggcgttttgcgctgcttcgcgatgtacgggccagatatacgcgttgacattgattattgactagttattaatagtaatcaattacggggtcattagttcatagcccatatatggagttccgcgttacataacttacggtaaatggcccgcctggctgaccgcccaacgacccccgcccattgacgtcaataatgacgtatgttcccatagtaacgccaatagggactttccattgacgtcaatgggtggactatttacggtaaactgcccacttggcagtacatcaagtgtatcatatgccaagtacgccccctattgacgtcaatgacggtaaatggcccgcctggcattatgcccagtacatgaccttatgggactttcctacttggcagtacatctacgtattagtcatcgctattaccatggtgatgcggttttggcagtacatcaatgggcgtggatagcggtttgactcacggggatttccaagtctccaccccattgacgtcaatgggagtttgttttggcaccaaaatcaacgggactttccaaaatgtcgtaacaactccgccccattgacgcaaatgggcggtaggcgtgtacggtgggaggtctatataagcagagctctctggctaactagagaacccactgcttactggcttatcgaaattaatacgactcactatagggagacccaagctggctagcnnnnnnnnnnggatcccaactagtcaaaagtgaactggaggagaagaaatctgaacttcgtcataaattgaaatatgtgcctcatgaatatattgaattaattgaaattgccagaaattccactcaggatagaattcttgaaatgaaggtaatggaattttttatgaaagtttatggatatagaggtaaacatttgggtggatcaaggaaaccggacggagcaatttatactgtcggatctcctattgattacggtgtgatcgtggatactaaagcttatagcggaggttataatctgccaattggccaagcagatgaaatgcaacgatatgtcgaagaaaatcaaacacgaaacaaacatatcaaccctaatgaatggtggaaagtctatccatcttctgtaacggaatttaagtttttatttgtgagtggtcactttaaaggaaactacaaagctcagcttacacgattaaatcatatcactaattgtaatggagctgttcttagtgtagaagagcttttaattggtggagaaatgattaaagccggcacattaaccttagaggaagtcagacggaaatttaataacggcgagataaacttttaagggcccttcgaaggtaagcctatccctaaccctctcctcggtctcgattctacgcgtaccggtcatcatcaccatcaccattgagtttaaacccgctgatcagcctcgactgtgccttctagttgccagccatctgttgtttgcccctcccccgtgccttccttgaccctggaaggtgccactcccactgtcctttcctaataaaatgaggaaattgcatcgcattgtctgagtaggtgtcattctattctggggggtggggtggggcaggacagcaagggggaggattgggaagacaatagcaggcatgctggggatgcggtgggctctatggcttctgaggcggaaagaaccagctggggctctagggggtatccccacgcgccctgtagcggcgcattaagcgcggcgggtgtggtggttacgcgcagcgtgaccgctacacttgccagcgccctagcgcccgctcctttcgctttcttcccttcctttctcgccacgttcgccggctttccccgtcaagctctaaatcggggcatccctttagggttccgatttagtgctttacggcacctcgaccccaaaaaacttgattagggtgatggttcacgtagtgggccatcgccctgatagacggtttttcgccctttgacgttggagtccacgttctttaatagtggactcttgttccaaactggaacaacactcaaccctatctcggtctattcttttgatttataagggattttggggatttcggcctattggttaaaaaatgagctgatttaacaaaaatttaacgcgaattaattctgtggaatgtgtgtcagttagggtgtggaaagtccccaggctccccaggcaggcagaagtatgcaaagcatgcatctcaattagtcagcaaccaggtgtggaaagtccccaggctccccagcaggcagaagtatgcaaagcatgcatctcaattagtcagcaaccatagtcccgcccctaactccgcccatcccgcccctaactccgcccagttccgcccattctccgccccatggctgactaattttttttatttatgcagaggccgaggccgcctctgcctctgagctattccagaagtagtgaggaggcttttttggaggcctaggcttttgcaaaaagctcccgggagcttgtatatccattttcggatctgatcagcacgtgttgacaattaatcatcggcatagtatatcggcatagtataatacgacaaggtgaggaactaaaccatggccaagcctttgtctcaagaagaatccaccctcattgaaagagcaacggctacaatcaacagcatccccatctctgaagactacagcgtcgccagcgcagctctctctagcgacggccgcatcttcactggtgtcaatgtatatcattttactgggggaccttgtgcagaactcgtggtgctgggcactgctgctgctgcggcagctggcaacctgacttgtatcgtcgcgatcggaaatgagaacaggggcatcttgagcccctgcggacggtgtcgacaggtgcttctcgatctgcatcctgggatcaaagcgatagtgaaggacagtgatggacagccgacggcagttgggattcgtgaattgctgccctctggttatgtgtgggagggctaagcacttcgtggccgaggagcaggactgacacgtgctacgagatttcgattccaccgccgccttctatgaaaggttgggcttcggaatcgttttccgggacgccggctggatgatcctccagcgcggggatctcatgctggagttcttcgcccaccccaacttgtttattgcagcttataatggttacaaataaagcaatagcatcacaaatttcacaaataaagcatttttttcactgcattctagttgtggtttgtccaaactcatcaatgtatcttatcatgtctgtataccgtcgacctctagctagagcttggcgtaatcatggtcatagctgtttcctgtgtgaaattgttatccgctcacaattccacacaacatacgagccggaagcataaagtgtaaagcctggggtgcctaatgagtgagctaactcacattaattgcgttgcgctcactgcccgctttccagtcgggaaacctgtcgtgccagctgcattaatgaatcggccaacgcgcggggagaggcggtttgcgtattgggcgctcttccgcttcctcgctcactgactcgctgcgctcggtcgttcggctgcggcgagcggtatcagctcactcaaaggcggtaatacggttatccacagaatcaggggataacgcaggaaagaacatgtgagcaaaaggccagcaaaaggccaggaaccgtaaaaaggccgcgttgctggcgtttttccataggctccgcccccctgacgagcatcacaaaaatcgacgctcaagtcagaggtggcgaaacccgacaggactataaagataccaggcgtttccccctggaagctccctcgtgcgctctcctgttccgaccctgccgcttaccggatacctgtccgcctttctcccttcgggaagcgtggcgctttctcaatgctcacgctgtaggtatctcagttcggtgtaggtcgttcgctccaagctgggctgtgtgcacgaaccccccgttcagcccgaccgctgcgccttatccggtaactatcgtcttgagtccaacccggtaagacacgacttatcgccactggcagcagccactggtaacaggattagcagagcgaggtatgtaggcggtgctacagagttcttgaagtggtggcctaactacggctacactagaaggacagtatttggtatctgcgctctgctgaagccagttaccttcggaaaaagagttggtagctcttgatccggcaaacaaaccaccgctggtagcggtggtttttttgtttgcaagcagcagattacgcgcagaaaaaaaggatctcaagaagatcctttgatcttttctacggggtctgacgctcagtggaacgaaaactcacgttaagggattttggtcatgagattatcaaaaaggatcttcacctagatccttttaaattaaaaatgaagttttaaatcaatctaaagtatatatgagtaaacttggtctgacagttaccaatgcttaatcagtgaggcacctatctcagcgatctgtctatttcgttcatccatagttgcctgactccccgtcgtgtagataactacgatacgggagggcttaccatctggccccagtgctgcaatgataccgcgagacccacgctcaccggctccagatttatcagcaataaaccagccagccggaagggccgagcgcagaagtggtcctgcaactttatccgcctccatccagtctattaattgttgccgggaagctagagtaagtagttcgccagttaatagtttgcgcaacgttgttgccattgctacaggcatcgtggtgtcacgctcgtcgtttggtatggcttcattcagctccggttcccaacgatcaaggcgagttacatgatcccccatgttgtgcaaaaaagcggttagctccttcggtcctccgatcgttgtcagaagtaagttggccgcagtgttatcactcatggttatggcagcactgcataattctcttactgtcatgccatccgtaagatgcttttctgtgactggtgagtactcaaccaagtcattctgagaatagtgtatgcggcgaccgagttgctcttgcccggcgtcaatacgggataataccgcgccacatagcagaactttaaaagtgctcatcattggaaaacgttcttcggggcgaaaactctcaaggatcttaccgctgttgagatccagttcgatgtaacccactcgtgcacccaactgatcttcagcatcttttactttcaccagcgtttctgggtgagcaaaaacaggaaggcaaaatgccgcaaaaaagggaataagggcgacacggaaatgttgaatactcatactcttcctttttcaatattattgaagcatttatcagggttattgtctcatgagcggatacatatttgaatgtatttagaaaaataaacaaataggggttccgcgcacatttccccgaaaagtgccacctgacgtc

SEQ ID NO: 245 - DNA, 2424 bp, Artificial Sequence
  Description of Artificial Sequence: Synthetic polynucleotide
gctagcaccatggactacaaagaccatgacggtgattataaagatcatgacatcgattacaaggatgacgatgacaagatggcccccaagaagaagaggaaggtgggcattcaccgcggggtacctatggtggacttgaggacactcggttattcgcaacagcaacaggagaaaatcaagcctaaggtcaggagcaccgtcgcgcaacaccacgaggcgcttgtggggcatggcttcactcatgcgcatattgtcgcgctttcacagcaccctgcggcgcttgggacggtggctgtcaaataccaagatatgattgcggccctgcccgaagccacgcacgaggcaattgtaggggtcggtaaacagtggtcgggagcgcgagcacttgaggcgctgctgactgtggcgggtgagcttagggggcctccgctccagctcgacaccgggcagctgctgaagatcgcgaagagagggggagtaacagcggtagaggcagtgcacgcctggcgcaatgcgctcaccggggcccccttgaacctgaccccagaccaggtagtcgcaatcgcgtcgaacattgggggaaagcaagccctggaaaccgtgcaaaggttgttgccggtcctttgtcaagaccacggccttacaccggagcaagtcgtggccattgcaagcaatgggggtggcaaacaggctcttgagacggttcagagacttctcccagttctctgtcaagcccacgggctgactcccgatcaagttgtagcgattgcgaataacaatggagggaaacaagcattggagactgtccaacggctccttcccgtgttgtgtcaagcccacggtttgacgcctgcacaagtggtcgccatcgcctcgaatggcggcggtaagcaggcgctggaaacagtacagcgcctgctgcctgtactgtgccaggatcatggactgaccccagaccaggtagtcgcaatcgcgtcgaacattgggggaaagcaagccctggaaaccgtgcaaaggttgttgccggtcctttgtcaagaccacggccttacaccggagcaagtcgtggccattgcatcccacgacggtggcaaacaggctcttgagacggttcagagacttctcccagttctctgtcaagcccacgggctgactcccgatcaagttgtagcgattgcgaataacaatggagggaaacaagcattggagactgtccaacggctccttcccgtgttgtgtcaagcccacggtttgacgcctgcacaagtggtcgccatcgccagccatgatggcggtaagcaggcgctggaaacagtacagcgcctgctgcctgtactgtgccaggatcatggactgaccccagaccaggtagtcgcaatcgcgtcacatgacgggggaaagcaagccctggaaaccgtgcaaaggttgttgccggtcctttgtcaagaccacggccttacaccggagcaagtcgtggccattgcaagcaatgggggtggcaaacaggctcttgagacggttcagagacttctcccagttctctgtcaagcccacgggctgactcccgatcaagttgtagcgattgcgtcgcatgacggagggaaacaagcattggagactgtccaacggctccttcccgtgttgtgtcaagcccacggtttgacgcctgcacaagtggtcgccatcgccagccatgatggcggtaagcaggcgctggaaacagtacagcgcctgctgcctgtactgtgccaggatcatggactgaccccagaccaggtagtcgcaatcgcgtcacatgacgggggaaagcaagccctggaaaccgtgcaaaggttgttgccggtcctttgtcaagaccacggccttacaccggagcaagtcgtggccattgcaagcaatgggggtggcaaacaggctcttgagacggttcagagacttctcccagttctctgtcaagcccacgggctgactcccgatcaagttgtagcgattgcgaataacaatggagggaaacaagcattggagactgtccaacggctccttcccgtgttgtgtcaagcccacggtttgacgcctgcacaagtggtcgccatcgccaacaacaacggcggtaagcaggcgctggaaacagtacagcgcctgctgcctgtactgtgccaggatcatggactgacacccgaacaggtggtcgccattgctaataataacggaggacggccagccttggagtccatcgtagcccaattgtccaggcccgatcccgcgttggctgcgttaacgaatgaccatctggtggcgttggcatgtcttggtggacgacccgcgctcgatgcagtcaaaaagggtctgcctcatgctcccgcattgatcaaaagaaccaaccggcggattcccgagagaacttcccatcgagtcgcgggatcc

SEQ ID NO: 246 - protein, 808 aa, Artificial Sequence
  Description of Artificial Sequence: Synthetic polypeptide
ASTMDYKDHDGDYKDHDIDYKDDDDKMAPKKKRKVGIHRGVPMVDLRTLGYSQQQQEKIKPKVRSTVAQHHEALVGHGFTHAHIVALSQHPAALGTVAVKYQDMIAALPEATHEAIVGVGKQWSGARALEALLTVAGELRGPPLQLDTGQLLKIAKRGGVTAVEAVHAWRNALTGAPLNLTPDQVVAIASNIGGKQALETVQRLLPVLCQDHGLTPEQVVAIASNGGGKQALETVQRLLPVLCQAHGLTPDQVVAIANNNGGKQALETVQRLLPVLCQAHGLTPAQVVAIASNGGGKQALETVQRLLPVLCQDHGLTPDQVVAIASNIGGKQALETVQRLLPVLCQDHGLTPEQVVAIASHDGGKQALETVQRLLPVLCQAHGLTPDQVVAIANNNGGKQALETVQRLLPVLCQAHGLTPAQVVAIASHDGGKQALETVQRLLPVLCQDHGLTPDQVVAIASHDGGKQALETVQRLLPVLCQDHGLTPEQVVAIASNGGGKQALETVQRLLPVLCQAHGLTPDQVVAIASHDGGKQALETVQRLLPVLCQAHGLTPAQVVAIASHDGGKQALETVQRLLPVLCQDHGLTPDQVVAIASHDGGKQALETVQRLLPVLCQDHGLTPEQVVAIASNGGGKQALETVQRLLPVLCQAHGLTPDQVVAIANNNGGKQALETVQRLLPVLCQAHGLTPAQVVAIANNNGGKQALETVQRLLPVLCQDHGLTPEQVVAIANNNGGRPALESIVAQLSRPDPALAALTNDHLVALACLGGRPALDAVKKGLPHAPALIKRTNRRIPERTSHRVAGS

SEQ ID NO: 247 - DNA, 2424 bp, Artificial Sequence
  Description of Artificial Sequence: Synthetic polynucleotide
gctagcaccatggactacaaagaccatgacggtgattataaagatcatgacatcgattacaaggatgacgatgacaagatggcccccaagaagaagaggaaggtgggcattcaccgcggggtacctatggtggacttgaggacactcggttattcgcaacagcaacaggagaaaatcaagcctaaggtcaggagcaccgtcgcgcaacaccacgaggcgcttgtggggcatggcttcactcatgcgcatattgtcgcgctttcacagcaccctgcggcgcttgggacggtggctgtcaaataccaagatatgattgcggccctgcccgaagccacgcacgaggcaattgtaggggtcggtaaacagtggtcgggagcgcgagcacttgaggcgctgctgactgtggcgggtgagcttagggggcctccgctccagctcgacaccgggcagctgctgaagatcgcgaagagagggggagtaacagcggtagaggcagtgcacgcctggcgcaatgcgctcaccggggcccccttgaacctgaccccagaccaggtagtcgcaatcgcgtcgaacattgggggaaagcaagccctggaaaccgtgcaaaggttgttgccggtcctttgtcaagaccacggccttacaccggagcaagtcgtggccattgcatcccacgacggtggcaaacaggctcttgagacggttcagagacttctcccagttctctgtcaagcccacgggctgactcccgatcaagttgtagcgattgcgtcgaacattggagggaaacaagcattggagactgtccaacggctccttcccgtgttgtgtcaagcccacggtttgacgcctgcacaagtggtcgccatcgccaacaacaacggcggtaagcaggcgctggaaacagtacagcgcctgctgcctgtactgtgccaggatcatggactgaccccagaccaggtagtcgcaatcgcgtcgaacattgggggaaagcaagccctggaaaccgtgcaaaggttgttgccggtcctttgtcaagaccacggccttacaccggagcaagtcgtggccattgcaagcaacatcggtggcaaacaggctcttgagacggttcagagacttctcccagttctctgtcaagcccacgggctgactcccgatcaagttgtagcgattgcgaataacaatggagggaaacaagcattggagactgtccaacggctccttcccgtgttgtgtcaagcccacggtttgacgcctgcacaagtggtcgccatcgccagccatgatggcggtaagcaggcgctggaaacagtacagcgcctgctgcctgtactgtgccaggatcatggactgaccccagaccaggtagtcgcaatcgcgaacaataatgggggaaagcaagccctggaaaccgtgcaaaggttgttgccggtcctttgtcaagaccacggccttacaccggagcaagtcgtggccattgcaaataataacggtggcaaacaggctcttgagacggttcagagacttctcccagttctctgtcaagcccacgggctgactcccgatcaagttgtagcgattgcgaataacaatggagggaaacaagcattggagactgtccaacggctccttcccgtgttgtgtcaagcccacggtttgacgcctgcacaagtggtcgccatcgccagccatgatggcggtaagcaggcgctggaaacagtacagcgcctgctgcctgtactgtgccaggatcatggactgaccccagaccaggtagtcgcaatcgcgtcgaacattgggggaaagcaagccctggaaaccgtgcaaaggttgttgccggtcctttgtcaagaccacggccttacaccggagcaagtcgtggccattgcaagcaacatcggtggcaaacaggctcttgagacggttcagagacttctcccagttctctgtcaagcccacgggctgactcccgatcaagttgtagcgattgcgtcgaacattggagggaaacaagcattggagactgtccaacggctccttcccgtgttgtgtcaagcccacggtttgacgcctgcacaagtggtcgccatcgccaacaacaacggcggtaagcaggcgctggaaacagtacagcgcctgctgcctgtactgtgccaggatcatggactgacacccgaacaggtggtcgccattgctaataataacggaggacggccagccttggagtccatcgtagcccaattgtccaggcccgatcccgcgttggctgcgttaacgaatgaccatctggtggcgttggcatgtcttggtggacgacccgcgctcgatgcagtcaaaaagggtctgcctcatgctcccgcattgatcaaaagaaccaaccggcggattcccgagagaacttcccatcgagtcgcgggatcc

SEQ ID NO: 248 - protein, 808 aa, Artificial Sequence
  Description of Artificial Sequence: Synthetic polypeptide
ASTMDYKDHDGDYKDHDIDYKDDDDKMAPKKKRKVGIHRGVPMVDLRTLGYSQQQQEKIKPKVRSTVAQHHEALVGHGFTHAHIVALSQHPAALGTVAVKYQDMIAALPEATHEAIVGVGKQWSGARALEALLTVAGELRGPPLQLDTGQLLKIAKRGGVTAVEAVHAWRNALTGAPLNLTPDQVVAIASNIGGKQALETVQRLLPVLCQDHGLTPEQVVAIASHDGGKQALETVQRLLPVLCQAHGLTPDQVVAIASNIGGKQALETVQRLLPVLCQAHGLTPAQVVAIANNNGGKQALETVQRLLPVLCQDHGLTPDQVVAIASNIGGKQALETVQRLLPVLCQDHGLTPEQVVAIASNIGGKQALETVQRLLPVLCQAHGLTPDQVVAIANNNGGKQALETVQRLLPVLCQAHGLTPAQVVAIASHDGGKQALETVQRLLPVLCQDHGLTPDQVVAIANNNGGKQALETVQRLLPVLCQDHGLTPEQVVAIANNNGGKQALETVQRLLPVLCQAHGLTPDQVVAIANNNGGKQALETVQRLLPVLCQAHGLTPAQVVAIASHDGGKQALETVQRLLPVLCQDHGLTPDQVVAIASNIGGKQALETVQRLLPVLCQDHGLTPEQVVAIASNIGGKQALETVQRLLPVLCQAHGLTPDQVVAIASNIGGKQALETVQRLLPVLCQAHGLTPAQVVAIANNNGGKQALETVQRLLPVLCQDHGLTPEQVVAIANNNGGRPALESIVAQLSRPDPALAALTNDHLVALACLGGRPALDAVKKGLPHAPALIKRTNRRIPERTSHRVAGS

SEQ ID NO: 249 - DNA, 2424 bp, Artificial Sequence
  Description of Artificial Sequence: Synthetic polynucleotide
gctagcaccatggactacaaagaccatgacggtgattataaagatcatgacatcgattacaaggatgacgatgacaagatggcccccaagaagaagaggaaggtgggcattcaccgcggggtacctatggtggacttgaggacactcggttattcgcaacagcaacaggagaaaatcaagcctaaggtcaggagcaccgtcgcgcaacaccacgaggcgcttgtggggcatggcttcactcatgcgcatattgtcgcgctttcacagcaccctgcggcgcttgggacggtggctgtcaaataccaagatatgattgcggccctgcccgaagccacgcacgaggcaattgtaggggtcggtaaacagtggtcgggagcgcgagcacttgaggcgctgctgactgtggcgggtgagcttagggggcctccgctccagctcgacaccgggcagctgctgaagatcgcgaagagagggggagtaacagcggtagaggcagtgcacgcctggcgcaatgcgctcaccggggcccccttgaacctgaccccagaccaggtagtcgcaatcgcgtcacatgacgggggaaagcaagccctggaaaccgtgcaaaggttgttgccggtcctttgtcaagaccacggccttacaccggagcaagtcgtggccattgcatcccacgacggtggcaaacaggctcttgagacggttcagagacttctcccagttctctgtcaagcccacgggctgactcccgatcaagttgtagcgattgcgaataacaatggagggaaacaagcattggagactgtccaacggctccttcccgtgttgtgtcaagcccacggtttgacgcctgcacaagtggtcgccatcgcctccaatattggcggtaagcaggcgctggaaacagtacagcgcctgctgcctgtactgtgccaggatcatggactgaccccagaccaggtagtcgcaatcgcgtcgaacattgggggaaagcaagccctggaaaccgtgcaaaggttgttgccggtcctttgtcaagaccacggccttacaccggagcaagtcgtggccattgcaaataataacggtggcaaacaggctcttgagacggttcagagacttctcccagttctctgtcaagcccacgggctgactcccgatcaagttgtagcgattgcgtcgcatgacggagggaaacaagcattggagactgtccaacggctccttcccgtgttgtgtcaagcccacggtttgacgcctgcacaagtggtcgccatcgcctcgaatggcggcggtaagcaggcgctggaaacagtacagcgcctgctgcctgtactgtgccaggatcatggactgaccccagaccaggtagtcgcaatcgcgaacaataatgggggaaagcaagccctggaaaccgtgcaaaggttgttgccggtcctttgtcaagaccacggccttacaccggagcaagtcgtggccattgcaagcaacatcggtggcaaacaggctcttgagacggttcagagacttctcccagttctctgtcaagcccacgggctgactcccgatcaagttgtagcgattgcgtcgcatgacggagggaaacaagcattggagactgtccaacggctccttcccgtgttgtgtcaagcccacggtttgacgcctgcacaagtggtcgccatcgcctccaatattggcggtaagcaggcgctggaaacagtacagcgcctgctgcctgtactgtgccaggatcatggactgaccccagaccaggtagtcgcaatcgcgaacaataatgggggaaagcaagccctggaaaccgtgcaaaggttgttgccggtcctttgtcaagaccacggccttacaccggagcaagtcgtggccattgcaagcaacatcggtggcaaacaggctcttgagacggttcagagacttctcccagttctctgtcaagcccacgggctgactcccgatcaagttgtagcgattgcgtccaacggtggagggaaacaagcattggagactgtccaacggctccttcccgtgttgtgtcaagcccacggtttgacgcctgcacaagtggtcgccatcgccaacaacaacggcggtaagcaggcgctggaaacagtacagcgcctgctgcctgtactgtgccaggatcatggactgacacccgaacaggtggtcgccattgctaataataacggaggacggccagccttggagtccatcgtagcccaattgtccaggcccgatcccgcgttggctgcgttaacgaatgaccatctggtggcgttggcatgtcttggtggacgacccgcgctcgatgcagtcaaaaagggtctgcctcatgctcccgcattgatcaaaagaaccaaccggcggattcccgagagaacttcccatcgagtcgcgggatcc

SEQ ID NO: 250 - protein, 808 aa, Artificial Sequence
  Description of Artificial Sequence: Synthetic polypeptide
ASTMDYKDHDGDYKDHDIDYKDDDDKMAPKKKRKVGIHRGVPMVDLRTLGYSQQQQEKIKPKVRSTVAQHHEALVGHGFTHAHIVALSQHPAALGTVAVKYQDMIAALPEATHEAIVGVGKQWSGARALEALLTVAGELRGPPLQLDTGQLLKIAKRGGVTAVEAVHAWRNALTGAPLNLTPDQVVAIASHDGGKQALETVQRLLPVLCQDHGLTPEQVVAIASHDGGKQALETVQRLLPVLCQAHGLTPDQVVAIANNNGGKQALETVQRLLPVLCQAHGLTPAQVVAIASNIGGKQALETVQRLLPVLCQDHGLTPDQVVAIASNIGGKQALETVQRLLPVLCQDHGLTPEQVVAIANNNGGKQALETVQRLLPVLCQAHGLTPDQVVAIASHDGGKQALETVQRLLPVLCQAHGLTPAQVVAIASNGGGKQALETVQRLLPVLCQDHGLTPDQVVAIANNNGGKQALETVQRLLPVLCQDHGLTPEQVVAIASNIGGKQALETVQRLLPVLCQAHGLTPDQVVAIASHDGGKQALETVQRLLPVLCQAHGLTPAQVVAIASNIGGKQALETVQRLLPVLCQDHGLTPDQVVAIANNNGGKQALETVQRLLPVLCQDHGLTPEQVVAIASNIGGKQALETVQRLLPVLCQAHGLTPDQVVAIASNGGGKQALETVQRLLPVLCQAHGLTPAQVVAIANNNGGKQALETVQRLLPVLCQDHGLTPEQVVAIANNNGGRPALESIVAQLSRPDPALAALTNDHLVALACLGGRPALDAVKKGLPHAPALIKRTNRRIPERTSHRVAGS

SEQ ID NO: 251 - DNA, 2424 bp, Artificial Sequence
  Description of Artificial Sequence: Synthetic polynucleotide
gctagcaccatggactacaaagaccatgacggtgattataaagatcatgacatcgattacaaggatgacgatgacaagatggcccccaagaagaagaggaaggtgggcattcaccgcggggtacctatggtggacttgaggacactcggttattcgcaacagcaacaggagaaaatcaagcctaaggtcaggagcaccgtcgcgcaacaccacgaggcgcttgtggggcatggcttcactcatgcgcatattgtcgcgctttcacagcaccctgcggcgcttgggacggtggctgtcaaataccaagatatgattgcggccctgcccgaagccacgcacgaggcaattgtaggggtcggtaaacagtggtcgggagcgcgagcacttgaggcgctgctgactgtggcgggtgagcttagggggcctccgctccagctcgacaccgggcagctgctgaagatcgcgaagagagggggagtaacagcggtagaggcagtgcacgcctggcgcaatgcgctcaccggggcccccttgaacctgaccccagaccaggtagtcgcaatcgcgtcacatgacgggggaaagcaagccctggaaaccgtgcaaaggttgttgccggtcctttgtcaagaccacggccttacaccggagcaagtcgtggccattgcaagcaacatcggtggcaaacaggctcttgagacggttcagagacttctcccagttctctgtcaagcccacgggctgactcccgatcaagttgtagcgattgcgaataacaatggagggaaacaagcattggagactgtccaacggctccttcccgtgttgtgtcaagcccacggtttgacgcctgcacaagtggtcgccatcgccaacaacaacggcggtaagcaggcgctggaaacagtacagcgcctgctgcctgtactgtgccaggatcatggactgaccccagaccaggtagtcgcaatcgcgtcaaacggagggggaaagcaagccctggaaaccgtgcaaaggttgttgccggtcctttgtcaagaccacggccttacaccggagcaagtcgtggccattgcaagcaatgggggtggcaaacaggctcttgagacggttcagagacttctcccagttctctgtcaagcccacgggctgactcccgatcaagttgtagcgattgcgtcgcatgacggagggaaacaagcattggagactgtccaacggctccttcccgtgttgtgtcaagcccacggtttgacgcctgcacaagtggtcgccatcgccagccatgatggcggtaagcaggcgctggaaacagtacagcgcctgctgcctgtactgtgccaggatcatggactgaccccagaccaggtagtcgcaatcgcgaacaataatgggggaaagcaagccctggaaaccgtgcaaaggttgttgccggtcctttgtcaagaccacggccttacaccggagcaagtcgtggccattgcatcccacgacggtggcaaacaggctcttgagacggttcagagacttctcccagttctctgtcaagcccacgggctgactcccgatcaagttgtagcgattgcgtcgcatgacggagggaaacaagcattggagactgtccaacggctccttcccgtgttgtgtcaagcccacggtttgacgcctgcacaagtggtcgccatcgccagccatgatggcggtaagcaggcgctggaaacagtacagcgcctgctgcctgtactgtgccaggatcatggactgaccccagaccaggtagtcgcaatcgcgtcacatgacgggggaaagcaagccctggaaaccgtgcaaaggttgttgccggtcctttgtcaagaccacggccttacaccggagcaagtcgtggccattgcaagcaatgggggtggcaaacaggctcttgagacggttcagagacttctcccagttctctgtcaagcccacgggctgactcccgatcaagttgtagcgattgcgtcgaacattggagggaaacaagcattggagactgtccaacggctccttcccgtgttgtgtcaagcccacggtttgacgcctgcacaagtggtcgccatcgccagccatgatggcggtaagcaggcgctggaaacagtacagcgcctgctgcctgtactgtgccaggatcatggactgacacccgaacaggtggtcgccattgcttcccacgacggaggacggccagccttggagtccatcgtagcccaattgtccaggcccgatcccgcgttggctgcgttaacgaatgaccatctggtggcgttggcatgtcttggtggacgacccgcgctcgatgcagtcaaaaagggtctgcctcatgctcccgcattgatcaaaagaaccaaccggcggattcccgagagaacttcccatcgagtcgcgggatcc

SEQ ID NO: 252 - protein, 808 aa, Artificial Sequence
  Description of Artificial Sequence: Synthetic polypeptide
ASTMDYKDHDGDYKDHDIDYKDDDDKMAPKKKRKVGIHRGVPMVDLRTLGYSQQQQEKIKPKVRSTVAQHHEALVGHGFTHAHIVALSQHPAALGTVAVKYQDMIAALPEATHEAIVGVGKQWSGARALEALLTVAGELRGPPLQLDTGQLLKIAKRGGVTAVEAVHAWRNALTGAPLNLTPDQVVAIASHDGGKQALETVQRLLPVLCQDHGLTPEQVVAIASNIGGKQALETVQRLLPVLCQAHGLTPDQVVAIANNNGGKQALETVQRLLPVLCQAHGLTPAQVVAIANNNGGKQALETVQRLLPVLCQDHGLTPDQVVAIASNGGGKQALETVQRLLPVLCQDHGLTPEQVVAIASNGGGKQALETVQRLLPVLCQAHGLTPDQVVAIASHDGGKQALETVQRLLPVLCQAHGLTPAQVVAIASHDGGKQALETVQRLLPVLCQDHGLTPDQVVAIANNNGGKQALETVQRLLPVLCQDHGLTPEQVVAIASHDGGKQALETVQRLLPVLCQAHGLTPDQVVAIASHDGGKQALETVQRLLPVLCQAHGLTPAQVVAIASHDGGKQALETVQRLLPVLCQDHGLTPDQVVAIASHDGGKQALETVQRLLPVLCQDHGLTPEQVVAIASNGGGKQALETVQRLLPVLCQAHGLTPDQVVAIASNIGGKQALETVQRLLPVLCQAHGLTPAQVVAIASHDGGKQALETVQRLLPVLCQDHGLTPEQVVAIASHDGGRPALESIVAQLSRPDPALAALTNDHLVALACLGGRPALDAVKKGLPHAPALIKRTNRRIPERTSHRVAGS

SEQ ID NO: 253 - DNA, 2424 bp, Artificial Sequence
  Description of Artificial Sequence: Synthetic polynucleotide
gctagcaccatggactacaaagaccatgacggtgattataaagatcatgacatcgattacaaggatgacgatgacaagatggcccccaagaagaagaggaaggtgggcattcaccgcggggtacctatggtggacttgaggacactcggttattcgcaacagcaacaggagaaaatcaagcctaaggtcaggagcaccgtcgcgcaacaccacgaggcgcttgtggggcatggcttcactcatgcgcatattgtcgcgctttcacagcaccctgcggcgcttgggacggtggctgtcaaataccaagatatgattgcggccctgcccgaagccacgcacgaggcaattgtaggggtcggtaaacagtggtcgggagcgcgagcacttgaggcgctgctgactgtggcgggtgagcttagggggcctccgctccagctcgacaccgggcagctgctgaagatcgcgaagagagggggagtaacagcggtagaggcagtgcacgcctggcgcaatgcgctcaccggggcccccttgaacctgaccccagaccaggtagtcgcaatcgcgtcaaacggagggggaaagcaagccctggaaaccgtgcaaaggttgttgccggtcctttgtcaagaccacggccttacaccggagcaagtcgtggccattgcaagcaacatcggtggcaaacaggctcttgagacggttcagagacttctcccagttctctgtcaagcccacgggctgactcccgatcaagttgtagcgattgcgaataacaatggagggaaacaagcattggagactgtccaacggctccttcccgtgttgtgtcaagcccacggtttgacgcctgcacaagtggtcgccatcgcctccaatattggcggtaagcaggcgctggaaacagtacagcgcctgctgcctgtactgtgccaggatcatggactgaccccagaccaggtagtcgcaatcgcgtcacatgacgggggaaagcaagccctggaaaccgtgcaaaggttgttgccggtcctttgtcaagaccacggccttacaccggagcaagtcgtggccattgcaagcaatgggggtggcaaacaggctcttgagacggttcagagacttctcccagttctctgtcaagcccacgggctgactcccgatcaagttgtagcgattgcgtccaacggtggagggaaacaagcattggagactgtccaacggctccttcccgtgttgtgtcaagcccacggtttgacgcctgcacaagtggtcgccatcgcctccaatattggcggtaagcaggcgctggaaacagtacagcgcctgctgcctgtactgtgccaggatcatggactgaccccagaccaggtagtcgcaatcgcgaacaataatgggggaaagcaagccctggaaaccgtgcaaaggttgttgccggtcctttgtcaagaccacggccttacaccggagcaagtcgtggccattgcaaataataacggtggcaaacaggctcttgagacggttcagagacttctcccagttctctgtcaagcccacgggctgactcccgatcaagttgtagcgattgcgtccaacggtggagggaaacaagcattggagactgtccaacggctccttcccgtgttgtgtcaagcccacggtttgacgcctgcacaagtggtcgccatcgcctccaatattggcggtaagcaggcgctggaaacagtacagcgcctgctgcctgtactgtgccaggatcatggactgaccccagaccaggtagtcgcaatcgcgtcgaacattgggggaaagcaagccctggaaaccgtgcaaaggttgttgccggtcctttgtcaagaccacggccttacaccggagcaagtcgtggccattgcaaataataacggtggcaaacaggctcttgagacggttcagagacttctcccagttctctgtcaagcccacgggctgactcccgatcaagttgtagcgattgcgtccaacggtggagggaaacaagcattggagactgtccaacggctccttcccgtgttgtgtcaagcccacggtttgacgcctgcacaagtggtcgccatcgcctccaatattggcggtaagcaggcgctggaaacagtacagcgcctgctgcctgtactgtgccaggatcatggactgacacccgaacaggtggtcgccattgcttctaacatcggaggacggccagccttggagtccatcgtagcccaattgtccaggcccgatcccgcgttggctgcgttaacgaatgaccatctggtggcgttggcatgtcttggtggacgacccgcgctcgatgcagtcaaaaagggtctgcctcatgctcccgcattgatcaaaagaaccaaccggcggattcccgagagaacttcccatcgagtcgcgggatcc

SEQ ID NO: 254 - protein, 808 aa, Artificial Sequence
  Description of Artificial Sequence: Synthetic polypeptide
ASTMDYKDHDGDYKDHDIDYKDDDDKMAPKKKRKVGIHRGVPMVDLRTLGYSQQQQEKIKPKVRSTVAQHHEALVGHGFTHAHIVALSQHPAALGTVAVKYQDMIAALPEATHEAIVGVGKQWSGARALEALLTVAGELRGPPLQLDTGQLLKIAKRGGVTAVEAVHAWRNALTGAPLNLTPDQVVAIASNGGGKQALETVQRLLPVLCQDHGLTPEQVVAIASNIGGKQALETVQRLLPVLCQAHGLTPDQVVAIANNNGGKQALETVQRLLPVLCQAHGLTPAQVVAIASNIGGKQALETVQRLLPVLCQDHGLTPDQVVAIASHDGGKQALETVQRLLPVLCQDHGLTPEQVVAIASNGGGKQALETVQRLLPVLCQAHGLTPDQVVAIASNGGGKQALETVQRLLPVLCQAHGLTPAQVVAIASNIGGKQALETVQRLLPVLCQDHGLTPDQVVAIANNNGGKQALETVQRLLPVLCQDHGLTPEQVVAIANNNGGKQALETVQRLLPVLCQAHGLTPDQVVAIASNGGGKQALETVQRLLPVLCQAHGLTPAQVVAIASNIGGKQALETVQRLLPVLCQDHGLTPDQVVAIASNIGGKQALETVQRLLPVLCQDHGLTPEQVVAIANNNGGKQALETVQRLLPVLCQAHGLTPDQVVAIASNGGGKQALETVQRLLPVLCQAHGLTPAQVVAIASNIGGKQALETVQRLLPVLCQDHGLTPEQVVAIASNIGGRPALESIVAQLSRPDPALAALTNDHLVALACLGGRPALDAVKKGLPHAPALIKRTNRRIPERTSHRVAGS

SEQ ID NO: 255 - DNA, 2424 bp, Artificial Sequence
  Description of Artificial Sequence: Synthetic polynucleotide
gctagcaccatggactacaaagaccatgacggtgattataaagatcatgacatcgattacaaggatgacgatgacaagatggcccccaagaagaagaggaaggtgggcattcaccgcggggtacctatggtggacttgaggacactcggttattcgcaacagcaacaggagaaaatcaagcctaaggtcaggagcaccgtcgcgcaacaccacgaggcgcttgtggggcatggcttcactcatgcgcatattgtcgcgctttcacagcaccctgcggcgcttgggacggtggctgtcaaataccaagatatgattgcggccctgcccgaagccacgcacgaggcaattgtaggggtcggtaaacagtggtcgggagcgcgagcacttgaggcgctgctgactgtggcgggtgagcttagggggcctccgctccagctcgacaccgggcagctgctgaagatcgcgaagagagggggagtaacagcggtagaggcagtgcacgcctggcgcaatgcgctcaccggggcccccttgaacctgaccccagaccaggtagtcgcaatcgcgtcgaacattgggggaaagcaagccctggaaaccgtgcaaaggttgttgccggtcctttgtcaagaccacggccttacaccggagcaagtcgtggccattgcaaataataacggtggcaaacaggctcttgagacggttcagagacttctcccagttctctgtcaagcccacgggctgactcccgatcaagttgtagcgattgcgtccaacggtggagggaaacaagcattggagactgtccaacggctccttcccgtgttgtgtcaagcccacggtttgacgcctgcacaagtggtcgccatcgcctcgaatggcggcggtaagcaggcgctggaaacagtacagcgcctgctgcctgtactgtgccaggatcatggactgaccccagaccaggtagtcgcaatcgcgtcaaacggagggggaaagcaagccctggaaaccgtgcaaaggttgttgccggtcctttgtcaagaccacggccttacaccggagcaagtcgtggccattgcaaataataacggtggcaaacaggctcttgagacggttcagagacttctcccagttctctgtcaagcccacgggctgactcccgatcaagttgtagcgattgcgtccaacggtggagggaaacaagcattggagactgtccaacggctccttcccgtgttgtgtcaagcccacggtttgacgcctgcacaagtggtcgccatcgcctccaatattggcggtaagcaggcgctggaaacagtacagcgcctgctgcctgtactgtgccaggatcatggactgaccccagaccaggtagtcgcaatcgcgaacaataatgggggaaagcaagccctggaaaccgtgcaaaggttgttgccggtcctttgtcaagaccacggccttacaccggagcaagtcgtggccattgcaagcaatgggggtggcaaacaggctcttgagacggttcagagacttctcccagttctctgtcaagcccacgggctgactcccgatcaagttgtagcgattgcgtccaacggtggagggaaacaagcattggagactgtccaacggctccttcccgtgttgtgtcaagcccacggtttgacgcctgcacaagtggtcgccatcgccagccatgatggcggtaagcaggcgctggaaacagtacagcgcctgctgcctgtactgtgccaggatcatggactgaccccagaccaggtagtcgcaatcgcgtcaaacggagggggaaagcaagccctggaaaccgtgcaaaggttgttgccggtcctttgtcaagaccacggccttacaccggagcaagtcgtggccattgcatcccacgacggtggcaaacaggctcttgagacggttcagagacttctcccagttctctgtcaagcccacgggctgactcccgatcaagttgtagcgattgcgtcgcatgacggagggaaacaagcattggagactgtccaacggctccttcccgtgttgtgtcaagcccacggtttgacgcctgcacaagtggtcgccatcgccagccatgatggcggtaagcaggcgctggaaacagtacagcgcctgctgcctgtactgtgccaggatcatggactgacacccgaacaggtggtcgccattgcttcccacgacggaggacggccagccttggagtccatcgtagcccaattgtccaggcccgatcccgcgttggctgcgttaacgaatgaccatctggtggcgttggcatgtcttggtggacgacccgcgctcgatgcagtcaaaaagggtctgcctcatgctcccgcattgatcaaaagaaccaaccggcggattcccgagagaacttcccatcgagtcgcgggatcc

SEQ ID NO: 256 - protein, 808 aa, Artificial Sequence
  Description of Artificial Sequence: Synthetic polypeptide
ASTMDYKDHDGDYKDHDIDYKDDDDKMAPKKKRKVGIHRGVPMVDLRTLGYSQQQQEKIKPKVRSTVAQHHEALVGHGFTHAHIVALSQHPAALGTVAVKYQDMIAALPEATHEAIVGVGKQWSGARALEALLTVAGELRGPPLQLDTGQLLKIAKRGGVTAVEAVHAWRNALTGAPLNLTPDQVVAIASNIGGKQALETVQRLLPVLCQDHGLTPEQVVAIANNNGGKQALETVQRLLPVLCQAHGLTPDQVVAIASNGGGKQALETVQRLLPVLCQAHGLTPAQVVAIASNGGGKQALETVQRLLPVLCQDHGLTPDQVVAIASNGGGKQALETVQRLLPVLCQDHGLTPEQVVAIANNNGGKQALETVQRLLPVLCQAHGLTPDQVVAIASNGGGKQALETVQRLLPVLCQAHGLTPAQVVAIASNIGGKQALETVQRLLPVLCQDHGLTPDQVVAIANNNGGKQALETVQRLLPVLCQDHGLTPEQVVAIASNGGGKQALETVQRLLPVLCQAHGLTPDQVVAIASNGGGKQALETVQRLLPVLCQAHGLTPAQVVAIASHDGGKQALETVQRLLPVLCQDHGLTPDQVVAIASNGGGKQALETVQRLLPVLCQDHGLTPEQVVAIASHDGGKQALETVQRLLPVLCQAHGLTPDQVVAIASHDGGKQALETVQRLLPVLCQAHGLTPAQVVAIASHDGGKQALETVQRLLPVLCQDHGLTPEQVVAIASHDGGRPALESIVAQLSRPDPALAALTNDHLVALACLGGRPALDAVKKGLPHAPALIKRTNRRIPERTSHRVAGS

SEQ ID NO: 257 - DNA, 2322 bp, Artificial Sequence
  Description of Artificial Sequence: Synthetic polynucleotide
gctagcaccatggactacaaagaccatgacggtgattataaagatcatgacatcgattacaaggatgacgatgacaagatggcccccaagaagaagaggaaggtgggcattcaccgcggggtacctatggtggacttgaggacactcggttattcgcaacagcaacaggagaaaatcaagcctaaggtcaggagcaccgtcgcgcaacaccacgaggcgcttgtggggcatggcttcactcatgcgcatattgtcgcgctttcacagcaccctgcggcgcttgggacggtggctgtcaaataccaagatatgattgcggccctgcccgaagccacgcacgaggcaattgtaggggtcggtaaacagtggtcgggagcgcgagcacttgaggcgctgctgactgtggcgggtgagcttagggggcctccgctccagctcgacaccgggcagctgctgaagatcgcgaagagagggggagtaacagcggtagaggcagtgcacgcctggcgcaatgcgctcaccggggcccccttgaacctgaccccagaccaggtagtcgcaatcgcgtcacatgacgggggaaagcaagccctggaaaccgtgcaaaggttgttgccggtcctttgtcaagaccacggccttacaccggagcaagtcgtggccattgcatcccacgacggtggcaaacaggctcttgagacggttcagagacttctcccagttctctgtcaagcccacgggctgactcccgatcaagttgtagcgattgcgaataacaatggagggaaacaagcattggagactgtccaacggctccttcccgtgttgtgtcaagcccacggtttgacgcctgcacaagtggtcgccatcgccaacaacaacggcggtaagcaggcgctggaaacagtacagcgcctgctgcctgtactgtgccaggatcatggactgaccccagaccaggtagtcgcaatcgcgtcacatgacgggggaaagcaagccctggaaaccgtgcaaaggttgttgccggtcctttgtcaagaccacggccttacaccggagcaagtcgtggccattgcatcccacgacggtggcaaacaggctcttgagacggttcagagacttctcccagttctctgtcaagcccacgggctgactcccgatcaagttgtagcgattgcgaataacaatggagggaaacaagcattggagactgtccaacggctccttcccgtgttgtgtcaagcccacggtttgacgcctgcacaagtggtcgccatcgccaacaacaacggcggtaagcaggcgctggaaacagtacagcgcctgctgcctgtactgtgccaggatcatggactgaccccagaccaggtagtcgcaatcgcgtcacatgacgggggaaagcaagccctggaaaccgtgcaaaggttgttgccggtcctttgtcaagaccacggccttacaccggagcaagtcgtggccattgcaaataataacggtggcaaacaggctcttgagacggttcagagacttctcccagttctctgtcaagcccacgggctgactcccgatcaagttgtagcgattgcgtcgcatgacggagggaaacaagcattggagactgtccaacggctccttcccgtgttgtgtcaagcccacggtttgacgcctgcacaagtggtcgccatcgccagccatgatggcggtaagcaggcgctggaaacagtacagcgcctgctgcctgtactgtgccaggatcatggactgaccccagaccaggtagtcgcaatcgcgtcgaacattgggggaaagcaagccctggaaaccgtgcaaaggttgttgccggtcctttgtcaagaccacggccttacaccggagcaagtcgtggccattgcaagcaatgggggtggcaaacaggctcttgagacggttcagagacttctcccagttctctgtcaagcccacgggctgactcccgatcaagttgtagcgattgcgaataacaatggagggaaacaagcattggagactgtccaacggctccttcccgtgttgtgtcaagcccacggtctgacacccgaacaggtggtcgccattgcttctaacatcggaggacggccagccttggagtccatcgtagcccaattgtccaggcccgatcccgcgttggctgcgttaacgaatgaccatctggtggcgttggcatgtcttggtggacgacccgcgctcgatgcagtcaaaaagggtctgcctcatgctcccgcattgatcaaaagaaccaaccggcggattcccgagagaacttcccatcgagtcgcgggatcc

SEQ ID NO: 258 - protein, 774 aa, Artificial Sequence
  Description of Artificial Sequence: Synthetic polypeptide
ASTMDYKDHDGDYKDHDIDYKDDDDKMAPKKKRKVGIHRGVPMVDLRTLGYSQQQQEKIKPKVRSTVAQHHEALVGHGFTHAHIVALSQHPAALGTVAVKYQDMIAALPEATHEAIVGVGKQWSGARALEALLTVAGELRGPPLQLDTGQLLKIAKRGGVTAVEAVHAWRNALTGAPLNLTPDQVVAIASHDGGKQALETVQRLLPVLCQDHGLTPEQVVAIASHDGGKQALETVQRLLPVLCQAHGLTPDQVVAIANNNGGKQALETVQRLLPVLCQAHGLTPAQVVAIANNNGGKQALETVQRLLPVLCQDHGLTPDQVVAIASHDGGKQALETVQRLLPVLCQDHGLTPEQVVAIASHDGGKQALETVQRLLPVLCQAHGLTPDQVVAIANNNGGKQALETVQRLLPVLCQAHGLTPAQVVAIANNNGGKQALETVQRLLPVLCQDHGLTPDQVVAIASHDGGKQALETVQRLLPVLCQDHGLTPEQVVAIANNNGGKQALETVQRLLPVLCQAHGLTPDQVVAIASHDGGKQALETVQRLLPVLCQAHGLTPAQVVAIASHDGGKQALETVQRLLPVLCQDHGLTPDQVVAIASNIGGKQALETVQRLLPVLCQDHGLTPEQVVAIASNGGGKQALETVQRLLPVLCQAHGLTPDQVVAIANNNGGKQALETVQRLLPVLCQAHGLTPEQVVAIASNIGGRPALESIVAQLSRPDPALAALTNDHLVALACLGGRPALDAVKKGLPHAPALIKRTNRRIPERTSHRVAGS

SEQ ID NO: 259 - DNA, 2220 bp, Artificial Sequence
  Description of Artificial Sequence: Synthetic polynucleotide
gctagcaccatggactacaaagaccatgacggtgattataaagatcatgacatcgattacaaggatgacgatgacaagatggcccccaagaagaagaggaaggtgggcattcaccgcggggtacctatggtggacttgaggacactcggttattcgcaacagcaacaggagaaaatcaagcctaaggtcaggagcaccgtcgcgcaacaccacgaggcgcttgtggggcatggcttcactcatgcgcatattgtcgcgctttcacagcaccctgcggcgcttgggacggtggctgtcaaataccaagatatgattgcggccctgcccgaagccacgcacgaggcaattgtaggggtcggtaaacagtggtcgggagcgcgagcacttgaggcgctgctgactgtggcgggtgagcttagggggcctccgctccagctcgacaccgggcagctgctgaagatcgcgaagagagggggagtaacagcggtagaggcagtgcacgcctggcgcaatgcgctcaccggggcccccttgaacctgaccccagaccaggtagtcgcaatcgcgtcgaacattgggggaaagcaagccctggaaaccgtgcaaaggttgttgccggtcctttgtcaagaccacggccttacaccggagcaagtcgtggccattgcaaataataacggtggcaaacaggctcttgagacggttcagagacttctcccagttctctgtcaagcccacgggctgactcccgatcaagttgtagcgattgcgtcgcatgacggagggaaacaagcattggagactgtccaacggctccttcccgtgttgtgtcaagcccacggtttgacgcctgcacaagtggtcgccatcgccaacaacaacggcggtaagcaggcgctggaaacagtacagcgcctgctgcctgtactgtgccaggatcatggactgaccccagaccaggtagtcgcaatcgcgtcgaacattgggggaaagcaagccctggaaaccgtgcaaaggttgttgccggtcctttgtcaagaccacggccttacaccggagcaagtcgtggccattgcaaataataacggtggcaaacaggctcttgagacggttcagagacttctcccagttctctgtcaagcccacgggctgactcccgatcaagttgtagcgattgcgtcgcatgacggagggaaacaagcattggagactgtccaacggctccttcccgtgttgtgtcaagcccacggtttgacgcctgcacaagtggtcgccatcgccaacaacaacggcggtaagcaggcgctggaaacagtacagcgcctgctgcctgtactgtgccaggatcatggactgaccccagaccaggtagtcgcaatcgcgtcacatgacgggggaaagcaagccctggaaaccgtgcaaaggttgttgccggtcctttgtcaagaccacggccttacaccggagcaagtcgtggccattgcaaataataacggtggcaaacaggctcttgagacggttcagagacttctcccagttctctgtcaagcccacgggctgactcccgatcaagttgtagcgattgcgtcgaacattggagggaaacaagcattggagactgtccaacggctccttcccgtgttgtgtcaagcccacggtttgacgcctgcacaagtggtcgccatcgccagccatgatggcggtaagcaggcgctggaaacagtacagcgcctgctgcctgtactgtgccaggatcatggactgaccccagaccaggtagtcgcaatcgcgtcacatgacgggggaaagcaagccctggaaaccgtgcaaaggttgttgccggtcctttgtcaagaccacggccttacaccggagcaagtcgtggccattgcatcccacgacggtggcaaacaggctcttgagacggttcagagacttctcccagttctctgtcaagcccacgggctgacacccgaacaggtggtcgccattgcttcccacgacggaggacggccagccttggagtccatcgtagcccaattgtccaggcccgatcccgcgttggctgcgttaacgaatgaccatctggtggcgttggcatgtcttggtggacgacccgcgctcgatgcagtcaaaaagggtctgcctcatgctcccgcattgatcaaaagaaccaaccggcggattcccgagagaacttcccatcgagtcgcgggatcc

SEQ ID NO: 260 - protein, 740 aa, Artificial Sequence
  Description of Artificial Sequence: Synthetic polypeptide
ASTMDYKDHDGDYKDHDIDYKDDDDKMAPKKKRKVGIHRGVPMVDLRTLGYSQQQQEKIKPKVRSTVAQHHEALVGHGFTHAHIVALSQHPAALGTVAVKYQDMIAALPEATHEAIVGVGKQWSGARALEALLTVAGELRGPPLQLDTGQLLKIAKRGGVTAVEAVHAWRNALTGAPLNLTPDQVVAIASNIGGKQALETVQRLLPVLCQDHGLTPEQVVAIANNNGGKQALETVQRLLPVLCQAHGLTPDQVVAIASHDGGKQALETVQRLLPVLCQAHGLTPAQVVAIANNNGGKQALETVQRLLPVLCQDHGLTPDQVVAIASNIGGKQALETVQRLLPVLCQDHGLTPEQVVAIANNNGGKQALETVQRLLPVLCQAHGLTPDQVVAIASHDGGKQALETVQRLLPVLCQAHGLTPAQVVAIANNNGGKQALETVQRLLPVLCQDHGLTPDQVVAIASHDGGKQALETVQRLLPVLCQDHGLTPEQVVAIANNNGGKQALETVQRLLPVLCQAHGLTPDQVVAIASNIGGKQALETVQRLLPVLCQAHGLTPAQVVAIASHDGGKQALETVQRLLPVLCQDHGLTPDQVVAIASHDGGKQALETVQRLLPVLCQDHGLTPEQVVAIASHDGGKQALETVQRLLPVLCQAHGLTPEQVVAIASHDGGRPALESIVAQLSRPDPALAALTNDHLVALACLGGRPALDAVKKGLPHAPALIKRTNRRIPERTSHRVAGS

SEQ ID NO: 261 - DNA, 2424 bp, Artificial Sequence
  Description of Artificial Sequence: Synthetic polynucleotide
gctagcaccatggactacaaagaccatgacggtgattataaagatcatgacatcgattacaaggatgacgatgacaagatggcccccaagaagaagaggaaggtgggcattcaccgcggggtacctatggtggacttgaggacactcggttattcgcaacagcaacaggagaaaatcaagcctaaggtcaggagcaccgtcgcgcaacaccacgaggcgcttgtggggcatggcttcactcatgcgcatattgtcgcgctttcacagcaccctgcggcgcttgggacggtggctgtcaaataccaagatatgattgcggccctgcccgaagccacgcacgaggcaattgtaggggtcggtaaacagtggtcgggagcgcgagcacttgaggcgctgctgactgtggcgggtgagcttagggggcctccgctccagctcgacaccgggcagctgctgaagatcgcgaagagagggggagtaacagcggtagaggcagtgcacgcctggcgcaatgcgctcaccggggcccccttgaacctgaccccagaccaggtagtcgcaatcgcgtcgaacattgggggaaagcaagccctggaaaccgtgcaaaggttgttgccggtcctttgtcaagaccacggccttacaccggagcaagtcgtggccattgcaaataataacggtggcaaacaggctcttgagacggttcagagacttctcccagttctctgtcaagcccacgggctgactcccgatcaagttgtagcgattgcgaataacaatggagggaaacaagcattggagactgtccaacggctccttcccgtgttgtgtcaagcccacggtttgacgcctgcacaagtggtcgccatcgccagccatgatggcggtaagcaggcgctggaaacagtacagcgcctgctgcctgtactgtgccaggatcatggactgaccccagaccaggtagtcgcaatcgcgaacaataatgggggaaagcaagccctggaaaccgtgcaaaggttgttgccggtcctttgtcaagaccacggccttacaccggagcaagtcgtggccattgcatcccacgacggtggcaaacaggctcttgagacggttcagagacttctcccagttctctgtcaagcccacgggctgactcccgatcaagttgtagcgattgcgtcgcatgacggagggaaacaagcattggagactgtccaacggctccttcccgtgttgtgtcaagcccacggtttgacgcctgcacaagtggtcgccatcgcctccaatattggcggtaagcaggcgctggaaacagtacagcgcctgctgcctgtactgtgccaggatcatggactgaccccagaccaggtagtcgcaatcgcgtcgaacattgggggaaagcaagccctggaaaccgtgcaaaggttgttgccggtcctttgtcaagaccacggccttacaccggagcaagtcgtggccattgcaaataataacggtggcaaacaggctcttgagacggttcagagacttctcccagttctctgtcaagcccacgggctgactcccgatcaagttgtagcgattgcgaataacaatggagggaaacaagcattggagactgtccaacggctccttcccgtgttgtgtcaagcccacggtttgacgcctgcacaagtggtcgccatcgccagccatgatggcggtaagcaggcgctggaaacagtacagcgcctgctgcctgtactgtgccaggatcatggactgaccccagaccaggtagtcgcaatcgcgtcacatgacgggggaaagcaagccctggaaaccgtgcaaaggttgttgccggtcctttgtcaagaccacggccttacaccggagcaagtcgtggccattgcaagcaacatcggtggcaaacaggctcttgagacggttcagagacttctcccagttctctgtcaagcccacgggctgactcccgatcaagttgtagcgattgcgtccaacggtggagggaaacaagcattggagactgtccaacggctccttcccgtgttgtgtcaagcccacggtttgacgcctgcacaagtggtcgccatcgccaacaacaacggcggtaagcaggcgctggaaacagtacagcgcctgctgcctgtactgtgccaggatcatggactgacacccgaacaggtggtcgccattgcttctaatgggggaggacggccagccttggagtccatcgtagcccaattgtccaggcccgatcccgcgttggctgcgttaacgaatgaccatctggtggcgttggcatgtcttggtggacgacccgcgctcgatgcagtcaaaaagggtctgcctcatgctcccgcattgatcaaaagaaccaaccggcggattcccgagagaacttcccatcgagtcgcgggatcc

SEQ ID NO: 262 - protein, 808 aa, Artificial Sequence
  Description of Artificial Sequence: Synthetic polypeptide
ASTMDYKDHDGDYKDHDIDYKDDDDKMAPKKKRKVGIHRGVPMVDLRTLGYSQQQQEKIKPKVRSTVAQHHEALVGHGFTHAHIVALSQHPAALGTVAVKYQDMIAALPEATHEAIVGVGKQWSGARALEALLTVAGELRGPPLQLDTGQLLKIAKRGGVTAVEAVHAWRNALTGAPLNLTPDQVVAIASNIGGKQALETVQRLLPVLCQDHGLTPEQVVAIANNNGGKQALETVQRLLPVLCQAHGLTPDQVVAIANNNGGKQALETVQRLLPVLCQAHGLTPAQVVAIASHDGGKQALETVQRLLPVLCQDHGLTPDQVVAIANNNGGKQALETVQRLLPVLCQDHGLTPEQVVAIASHDGGKQALETVQRLLPVLCQAHGLTPDQVVAIASHDGGKQALETVQRLLPVLCQAHGLTPAQVVAIASNIGGKQALETVQRLLPVLCQDHGLTPDQVVAIASNIGGKQALETVQRLLPVLCQDHGLTPEQVVAIANNNGGKQALETVQRLLPVLCQAHGLTPDQVVAIANNNGGKQALETVQRLLPVLCQAHGLTPAQVVAIASHDGGKQALETVQRLLPVLCQDHGLTPDQVVAIASHDGGKQALETVQRLLPVLCQDHGLTPEQVVAIASNIGGKQALETVQRLLPVLCQAHGLTPDQVVAIASNGGGKQALETVQRLLPVLCQAHGLTPAQVVAIANNNGGKQALETVQRLLPVLCQDHGLTPEQVVAIASNGGGRPALESIVAQLSRPDPALAALTNDHLVALACLGGRPALDAVKKGLPHAPALIKRTNRRIPERTSHRVAGS

SEQ ID NO: 263 - DNA, 2424 bp, Artificial Sequence
  Description of Artificial Sequence: Synthetic polynucleotide
gctagcaccatggactacaaagaccatgacggtgattataaagatcatgacatcgattacaaggatgacgatgacaagatggcccccaagaagaagaggaaggtgggcattcaccgcggggtacctatggtggacttgaggacactcggttattcgcaacagcaacaggagaaaatcaagcctaaggtcaggagcaccgtcgcgcaacaccacgaggcgcttgtggggcatggcttcactcatgcgcatattgtcgcgctttcacagcaccctgcggcgcttgggacggtggctgtcaaataccaagatatgattgcggccctgcccgaagccacgcacgaggcaattgtaggggtcggtaaacagtggtcgggagcgcgagcacttgaggcgctgctgactgtggcgggtgagcttagggggcctccgctccagctcgacaccgggcagctgctgaagatcgcgaagagagggggagtaacagcggtagaggcagtgcacgcctggcgcaatgcgctcaccggggcccccttgaacctgaccccagaccaggtagtcgcaatcgcgaacaataatgggggaaagcaagccctggaaaccgtgcaaaggttgttgccggtcctttgtcaagaccacggccttacaccggagcaagtcgtggccattgcaaataataacggtggcaaacaggctcttgagacggttcagagacttctcccagttctctgtcaagcccacgggctgactcccgatcaagttgtagcgattgcgtcgcatgacggagggaaacaagcattggagactgtccaacggctccttcccgtgttgtgtcaagcccacggtttgacgcctgcacaagtggtcgccatcgccagccatgatggcggtaagcaggcgctggaaacagtacagcgcctgctgcctgtactgtgccaggatcatggactgaccccagaccaggtagtcgcaatcgcgtcacatgacgggggaaagcaagccctggaaaccgtgcaaaggttgttgccggtcctttgtcaagaccacggccttacaccggagcaagtcgtggccattgcaaataataacggtggcaaacaggctcttgagacggttcagagacttctcccagttctctgtcaagcccacgggctgactcccgatcaagttgtagcgattgcgtcgaacattggagggaaacaagcattggagactgtccaacggctccttcccgtgttgtgtcaagcccacggtttgacgcctgcacaagtggtcgccatcgccaacaacaacggcggtaagcaggcgctggaaacagtacagcgcctgctgcctgtactgtgccaggatcatggactgaccccagaccaggtagtcgcaatcgcgaacaataatgggggaaagcaagccctggaaaccgtgcaaaggttgttgccggtcctttgtcaagaccacggccttacaccggagcaagtcgtggccattgcatcccacgacggtggcaaacaggctcttgagacggttcagagacttctcccagttctctgtcaagcccacgggctgactcccgatcaagttgtagcgattgcgaataacaatggagggaaacaagcattggagactgtccaacggctccttcccgtgttgtgtcaagcccacggtttgacgcctgcacaagtggtcgccatcgccaacaacaacggcggtaagcaggcgctggaaacagtacagcgcctgctgcctgtactgtgccaggatcatggactgaccccagaccaggtagtcgcaatcgcgtcgaacattgggggaaagcaagccctggaaaccgtgcaaaggttgttgccggtcctttgtcaagaccacggccttacaccggagcaagtcgtggccattgcaaataataacggtggcaaacaggctcttgagacggttcagagacttctcccagttctctgtcaagcccacgggctgactcccgatcaagttgtagcgattgcgtccaacggtggagggaaacaagcattggagactgtccaacggctccttcccgtgttgtgtcaagcccacggtttgacgcctgcacaagtggtcgccatcgcctcgaatggcggcggtaagcaggcgctggaaacagtacagcgcctgctgcctgtactgtgccaggatcatggactgacacccgaacaggtggtcgccattgcttcccacgacggaggacggccagccttggagtccatcgtagcccaattgtccaggcccgatcccgcgttggctgcgttaacgaatgaccatctggtggcgttggcatgtcttggtggacgacccgcgctcgatgcagtcaaaaagggtctgcctcatgctcccgcattgatcaaaagaaccaaccggcggattcccgagagaacttcccatcgagtcgcgggatcc

SEQ ID NO: 264 - protein, 808 aa, Artificial Sequence
  Description of Artificial Sequence: Synthetic polypeptide
ASTMDYKDHDGDYKDHDIDYKDDDDKMAPKKKRKVGIHRGVPMVDLRTLGYSQQQQEKIKPKVRSTVAQHHEALVGHGFTHAHIVALSQHPAALGTVAVKYQDMIAALPEATHEAIVGVGKQWSGARALEALLTVAGELRGPPLQLDTGQLLKIAKRGGVTAVEAVHAWRNALTGAPLNLTPDQVVAIANNNGGKQALETVQRLLPVLCQDHGLTPEQVVAIANNNGGKQALETVQRLLPVLCQAHGLTPDQVVAIASHDGGKQALETVQRLLPVLCQAHGLTPAQVVAIASHDGGKQALETVQRLLPVLCQDHGLTPDQVVAIASHDGGKQALETVQRLLPVLCQDHGLTPEQVVAIANNNGGKQALETVQRLLPVLCQAHGLTPDQVVAIASNIGGKQALETVQRLLPVLCQAHGLTPAQVVAIANNNGGKQALETVQRLLPVLCQDHGLTPDQVVAIANNNGGKQALETVQRLLPVLCQDHGLTPEQVVAIASHDGGKQALETVQRLLPVLCQAHGLTPDQVVAIANNNGGKQALETVQRLLPVLCQAHGLTPAQVVAIANNNGGKQALETVQRLLPVLCQDHGLTPDQVVAIASNIGGKQALETVQRLLPVLCQDHGLTPEQVVAIANNNGGKQALETVQRLLPVLCQAHGLTPDQVVAIASNGGGKQALETVQRLLPVLCQAHGLTPAQVVAIASNGGGKQALETVQRLLPVLCQDHGLTPEQVVAIASHDGGRPALESIVAQLSRPDPALAALTNDHLVALACLGGRPALDAVKKGLPHAPALIKRTNRRIPERTSHRVAGS

SEQ ID NO: 265 - DNA, 2424 bp, Artificial Sequence
  Description of Artificial Sequence: Synthetic polynucleotide
gctagcaccatggactacaaagaccatgacggtgattataaagatcatgacatcgattacaaggatgacgatgacaagatggcccccaagaagaagaggaaggtgggcattcaccgcggggtacctatggtggacttgaggacactcggttattcgcaacagcaacaggagaaaatcaagcctaaggtcaggagcaccgtcgcgcaacaccacgaggcgcttgtggggcatggcttcactcatgcgcatattgtcgcgctttcacagcaccctgcggcgcttgggacggtggctgtcaaataccaagatatgattgcggccctgcccgaagccacgcacgaggcaattgtaggggtcggtaaacagtggtcgggagcgcgagcacttgaggcgctgctgactgtggcgggtgagcttagggggcctccgctccagctcgacaccgggcagctgctgaagatcgcgaagagagggggagtaacagcggtagaggcagtgcacgcctggcgcaatgcgctcaccggggcccccttgaacctgaccccagaccaggtagtcgcaatcgcgaacaataatgggggaaagcaagccctggaaaccgtgcaaaggttgttgccggtcctttgtcaagaccacggccttacaccggagcaagtcgtggccattgcaagcaacatcggtggcaaacaggctcttgagacggttcagagacttctcccagttctctgtcaagcccacgggctgactcccgatcaagttgtagcgattgcgtcgaacattggagggaaacaagcattggagactgtccaacggctccttcccgtgttgtgtcaagcccacggtttgacgcctgcacaagtggtcgccatcgccaacaacaacggcggtaagcaggcgctggaaacagtacagcgcctgctgcctgtactgtgccaggatcatggactgaccccagaccaggtagtcgcaatcgcgaacaataatgggggaaagcaagccctggaaaccgtgcaaaggttgttgccggtcctttgtcaagaccacggccttacaccggagcaagtcgtggccattgcaaataataacggtggcaaacaggctcttgagacggttcagagacttctcccagttctctgtcaagcccacgggctgactcccgatcaagttgtagcgattgcgtcgaacattggagggaaacaagcattggagactgtccaacggctccttcccgtgttgtgtcaagcccacggtttgacgcctgcacaagtggtcgccatcgccagccatgatggcggtaagcaggcgctggaaacagtacagcgcctgctgcctgtactgtgccaggatcatggactgaccccagaccaggtagtcgcaatcgcgtcgaacattgggggaaagcaagccctggaaaccgtgcaaaggttgttgccggtcctttgtcaagaccacggccttacaccggagcaagtcgtggccattgcaagcaatgggggtggcaaacaggctcttgagacggttcagagacttctcccagttctctgtcaagcccacgggctgactcccgatcaagttgtagcgattgcgtcgcatgacggagggaaacaagcattggagactgtccaacggctccttcccgtgttgtgtcaagcccacggtttgacgcctgcacaagtggtcgccatcgcctccaatattggcggtaagcaggcgctggaaacagtacagcgcctgctgcctgtactgtgccaggatcatggactgaccccagaccaggtagtcgcaatcgcgtcacatgacgggggaaagcaagccctggaaaccgtgcaaaggttgttgccggtcctttgtcaagaccacggccttacaccggagcaagtcgtggccattgcatcccacgacggtggcaaacaggctcttgagacggttcagagacttctcccagttctctgtcaagcccacgggctgactcccgatcaagttgtagcgattgcgtccaacggtggagggaaacaagcattggagactgtccaacggctccttcccgtgttgtgtcaagcccacggtttgacgcctgcacaagtggtcgccatcgcctcgaatggcggcggtaagcaggcgctggaaacagtacagcgcctgctgcctgtactgtgccaggatcatggactgacacccgaacaggtggtcgccattgcttctaatgggggaggacggccagccttggagtccatcgtagcccaattgtccaggcccgatcccgcgttggctgcgttaacgaatgaccatctggtggcgttggcatgtcttggtggacgacccgcgctcgatgcagtcaaaaagggtctgcctcatgctcccgcattgatcaaaagaaccaaccggcggattcccgagagaacttcccatcgagtcgcgggatcc

SEQ ID NO: 266 - protein, 808 aa, Artificial Sequence
  Description of Artificial Sequence: Synthetic polypeptide
ASTMDYKDHDGDYKDHDIDYKDDDDKMAPKKKRKVGIHRGVPMVDLRTLGYSQQQQEKIKPKVRSTVAQHHEALVGHGFTHAHIVALSQHPAALGTVAVKYQDMIAALPEATHEAIVGVGKQWSGARALEALLTVAGELRGPPLQLDTGQLLKIAKRGGVTAVEAVHAWRNALTGAPLNLTPDQVVAIANNNGGKQALETVQRLLPVLCQDHGLTPEQVVAIASNIGGKQALETVQRLLPVLCQAHGLTPDQVVAIASNIGGKQALETVQRLLPVLCQAHGLTPAQVVAIANNNGGKQALETVQRLLPVLCQDHGLTPDQVVAIANNNGGKQALETVQRLLPVLCQDHGLTPEQVVAIANNNGGKQALETVQRLLPVLCQAHGLTPDQVVAIASNIGGKQALETVQRLLPVLCQAHGLTPAQVVAIASHDGGKQALETVQRLLPVLCQDHGLTPDQVVAIASNIGGKQALETVQRLLPVLCQDHGLTPEQVVAIASNGGGKQALETVQRLLPVLCQAHGLTPDQVVAIASHDGGKQALETVQRLLPVLCQAHGLTPAQVVAIASNIGGKQALETVQRLLPVLCQDHGLTPDQVVAIASHDGGKQALETVQRLLPVLCQDHGLTPEQVVAIASHDGGKQALETVQRLLPVLCQAHGLTPDQVVAIASNGGGKQALETVQRLLPVLCQAHGLTPAQVVAIASNGGGKQALETVQRLLPVLCQDHGLTPEQVVAIASNGGGRPALESIVAQLSRPDPALAALTNDHLVALACLGGRPALDAVKKGLPHAPALIKRTNRRIPERTSHRVAGS

SEQ ID NO: 267 - DNA, 2322 bp, Artificial Sequence
  Description of Artificial Sequence: Synthetic polynucleotide
gctagcaccatggactacaaagaccatgacggtgattataaagatcatgacatcgattacaaggatgacgatgacaagatggcccccaagaagaagaggaaggtgggcattcaccgcggggtacctatggtggacttgaggacactcggttattcgcaacagcaacaggagaaaatcaagcctaaggtcaggagcaccgtcgcgcaacaccacgaggcgcttgtggggcatggcttcactcatgcgcatattgtcgcgctttcacagcaccctgcggcgcttgggacggtggctgtcaaataccaagatatgattgcggccctgcccgaagccacgcacgaggcaattgtaggggtcggtaaacagtggtcgggagcgcgagcacttgaggcgctgctgactgtggcgggtgagcttagggggcctccgctccagctcgacaccgggcagctgctgaagatcgcgaagagagggggagtaacagcggtagaggcagtgcacgcctggcgcaatgcgctcaccggggcccccttgaacctgaccccagaccaggtagtcgcaatcgcgtcacatgacgggggaaagcaagccctggaaaccgtgcaaaggttgttgccggtcctttgtcaagaccacggccttacaccggagcaagtcgtggccattgcaagcaatgggggtggcaaacaggctcttgagacggttcagagacttctcccagttctctgtcaagcccacgggctgactcccgatcaagttgtagcgattgcgtcgaacattggagggaaacaagcattggagactgtccaacggctccttcccgtgttgtgtcaagcccacggtttgacgcctgcacaagtggtcgccatcgccagccatgatggcggtaagcaggcgctggaaacagtacagcgcctgctgcctgtactgtgccaggatcatggactgaccccagaccaggtagtcgcaatcgcgtcaaacggagggggaaagcaagccctggaaaccgtgcaaaggttgttgccggtcctttgtcaagaccacggccttacaccggagcaagtcgtggccattgcaaataataacggtggcaaacaggctcttgagacggttcagagacttctcccagttctctgtcaagcccacgggctgactcccgatcaagttgtagcgattgcgtcgaacattggagggaaacaagcattggagactgtccaacggctccttcccgtgttgtgtcaagcccacggtttgacgcctgcacaagtggtcgccatcgcctccaatattggcggtaagcaggcgctggaaacagtacagcgcctgctgcctgtactgtgccaggatcatggactgaccccagaccaggtagtcgcaatcgcgtcaaacggagggggaaagcaagccctggaaaccgtgcaaaggttgttgccggtcctttgtcaagaccacggccttacaccggagcaagtcgtggccattgcatcccacgacggtggcaaacaggctcttgagacggttcagagacttctcccagttctctgtcaagcccacgggctgactcccgatcaagttgtagcgattgcgtccaacggtggagggaaacaagcattggagactgtccaacggctccttcccgtgttgtgtcaagcccacggtttgacgcctgcacaagtggtcgccatcgcctcgaatggcggcggtaagcaggcgctggaaacagtacagcgcctgctgcctgtactgtgccaggatcatggactgaccccagaccaggtagtcgcaatcgcgaacaataatgggggaaagcaagccctggaaaccgtgcaaaggttgttgccggtcctttgtcaagaccacggccttacaccggagcaagtcgtggccattgcaagcaacatcggtggcaaacaggctcttgagacggttcagagacttctcccagttctctgtcaagcccacgggctgactcccgatcaagttgtagcgattgcgaataacaatggagggaaacaagcattggagactgtccaacggctccttcccgtgttgtgtcaagcccacggtctgacacccgaacaggtggtcgccattgcttcccacgacggaggacggccagccttggagtccatcgtagcccaattgtccaggcccgatcccgcgttggctgcgttaacgaatgaccatctggtggcgttggcatgtcttggtggacgacccgcgctcgatgcagtcaaaaagggtctgcctcatgctcccgcattgatcaaaagaaccaaccggcggattcccgagagaacttcccatcgagtcgcgggatcc

SEQ ID NO: 268 - protein, 774 aa, Artificial Sequence
  Description of Artificial Sequence: Synthetic polypeptide
ASTMDYKDHDGDYKDHDIDYKDDDDKMAPKKKRKVGIHRGVPMVDLRTLGYSQQQQEKIKPKVRSTVAQHHEALVGHGFTHAHIVALSQHPAALGTVAVKYQDMIAALPEATHEAIVGVGKQWSGARALEALLTVAGELRGPPLQLDTGQLLKIAKRGGVTAVEAVHAWRNALTGAPLNLTPDQVVAIASHDGGKQALETVQRLLPVLCQDHGLTPEQVVAIASNGGGKQALETVQRLLPVLCQAHGLTPDQVVAIASNIGGKQALETVQRLLPVLCQAHGLTPAQVVAIASHDGGKQALETVQRLLPVLCQDHGLTPDQVVAIASNGGGKQALETVQRLLPVLCQDHGLTPEQVVAIANNNGGKQALETVQRLLPVLCQAHGLTPDQVVAIASNIGGKQALETVQRLLPVLCQAHGLTPAQVVAIASNIGGKQALETVQRLLPVLCQDHGLTPDQVVAIASNGGGKQALETVQRLLPVLCQDHGLTPEQVVAIASHDGGKQALETVQRLLPVLCQAHGLTPDQVVAIASNGGGKQALETVQRLLPVLCQAHGLTPAQVVAIASNGGGKQALETVQRLLPVLCQDHGLTPDQVVAIANNNGGKQALETVQRLLPVLCQDHGLTPEQVVAIASNIGGKQALETVQRLLPVLCQAHGLTPDQVVAIANNNGGKQALETVQRLLPVLCQAHGLTPEQVVAIASHDGGRPALESIVAQLSRPDPALAALTNDHLVALACLGGRPALDAVKKGLPHAPALIKRTNRRIPERTSHRVAGS

SEQ ID NO: 269 - DNA, 2220 bp, Artificial Sequence
  Description of Artificial Sequence: Synthetic polynucleotide
gctagcaccatggactacaaagaccatgacggtgattataaagatcatgacatcgattacaaggatgacgatgacaagatggcccccaagaagaagaggaaggtgggcattcaccgcggggtacctatggtggacttgaggacactcggttattcgcaacagcaacaggagaaaatcaagcctaaggtcaggagcaccgtcgcgcaacaccacgaggcgcttgtggggcatggcttcactcatgcgcatattgtcgcgctttcacagcaccctgcggcgcttgggacggtggctgtcaaataccaagatatgattgcggccctgcccgaagccacgcacgaggcaattgtaggggtcggtaaacagtggtcgggagcgcgagcacttgaggcgctgctgactgtggcgggtgagcttagggggcctccgctccagctcgacaccgggcagctgctgaagatcgcgaagagagggggagtaacagcggtagaggcagtgcacgcctggcgcaatgcgctcaccggggcccccttgaacctgaccccagaccaggtagtcgcaatcgcgtcacatgacgggggaaagcaagccctggaaaccgtgcaaaggttgttgccggtcctttgtcaagaccacggccttacaccggagcaagtcgtggccattgcaaataataacggtggcaaacaggctcttgagacggttcagagacttctcccagttctctgtcaagcccacgggctgactcccgatcaagttgtagcgattgcgaataacaatggagggaaacaagcattggagactgtccaacggctccttcccgtgttgtgtcaagcccacggtttgacgcctgcacaagtggtcgccatcgccagccatgatggcggtaagcaggcgctggaaacagtacagcgcctgctgcctgtactgtgccaggatcatggactgaccccagaccaggtagtcgcaatcgcgtcacatgacgggggaaagcaagccctggaaaccgtgcaaaggttgttgccggtcctttgtcaagaccacggccttacaccggagcaagtcgtggccattgcaagcaacatcggtggcaaacaggctcttgagacggttcagagacttctcccagttctctgtcaagcccacgggctgactcccgatcaagttgtagcgattgcgtcgcatgacggagggaaacaagcattggagactgtccaacggctccttcccgtgttgtgtcaagcccacggtttgacgcctgcacaagtggtcgccatcgccagccatgatggcggtaagcaggcgctggaaacagtacagcgcctgctgcctgtactgtgccaggatcatggactgaccccagaccaggtagtcgcaatcgcgtcgaacattgggggaaagcaagccctggaaaccgtgcaaaggttgttgccggtcctttgtcaagaccacggccttacaccggagcaagtcgtggccattgcaagcaatgggggtggcaaacaggctcttgagacggttcagagacttctcccagttctctgtcaagcccacgggctgactcccgatcaagttgtagcgattgcgaataacaatggagggaaacaagcattggagactgtccaacggctccttcccgtgttgtgtcaagcccacggtttgacgcctgcacaagtggtcgccatcgcctcgaatggcggcggtaagcaggcgctggaaacagtacagcgcctgctgcctgtactgtgccaggatcatggactgaccccagaccaggtagtcgcaatcgcgtcacatgacgggggaaagcaagccctggaaaccgtgcaaaggttgttgccggtcctttgtcaagaccacggccttacaccggagcaagtcgtggccattgcatcccacgacggtggcaaacaggctcttgagacggttcagagacttctcccagttctctgtcaagcccacgggctgacacccgaacaggtggtcgccattgcttcccacgacggaggacggccagccttggagtccatcgtagcccaattgtccaggcccgatcccgcgttggctgcgttaacgaatgaccatctggtggcgttggcatgtcttggtggacgacccgcgctcgatgcagtcaaaaagggtctgcctcatgctcccgcattgatcaaaagaaccaaccggcggattcccgagagaacttcccatcgagtcgcgggatcc

SEQ ID NO: 270 - protein, 740 aa, Artificial Sequence
  Description of Artificial Sequence: Synthetic polypeptide
ASTMDYKDHDGDYKDHDIDYKDDDDKMAPKKKRKVGIHRGVPMVDLRTLGYSQQQQEKIKPKVRSTVAQHHEALVGHGFTHAHIVALSQHPAALGTVAVKYQDMIAALPEATHEAIVGVGKQWSGARALEALLTVAGELRGPPLQLDTGQLLKIAKRGGVTAVEAVHAWRNALTGAPLNLTPDQVVAIASHDGGKQALETVQRLLPVLCQDHGLTPEQVVAIANNNGGKQALETVQRLLPVLCQAHGLTPDQVVAIANNNGGKQALETVQRLLPVLCQAHGLTPAQVVAIASHDGGKQALETVQRLLPVLCQDHGLTPDQVVAIASHDGGKQALETVQRLLPVLCQDHGLTPEQVVAIASNIGGKQALETVQRLLPVLCQAHGLTPDQVVAIASHDGGKQALETVQRLLPVLCQAHGLTPAQVVAIASHDGGKQALETVQRLLPVLCQDHGLTPDQVVAIASNIGGKQALETVQRLLPVLCQDHGLTPEQVVAIASNGGGKQALETVQRLLPVLCQAHGLTPDQVVAIANNNGGKQALETVQRLLPVLCQAHGLTPAQVVAIASNGGGKQALETVQRLLPVLCQDHGLTPDQVVAIASHDGGKQALETVQRLLPVLCQDHGLTPEQVVAIASHDGGKQALETVQRLLPVLCQAHGLTPEQVVAIASHDGGRPALESIVAQLSRPDPALAALTNDHLVALACLGGRPALDAVKKGLPHAPALIKRTNRRIPERTSHRVAGS

SEQ ID NO: 271 - DNA, 2424 bp, Artificial Sequence
  Description of Artificial Sequence: Synthetic polynucleotide
gctagcaccatggactacaaagaccatgacggtgattataaagatcatgacatcgattacaaggatgacgatgacaagatggcccccaagaagaagaggaaggtgggcattcaccgcggggtacctatggtggacttgaggacactcggttattcgcaacagcaacaggagaaaatcaagcctaaggtcaggagcaccgtcgcgcaacaccacgaggcgcttgtggggcatggcttcactcatgcgcatattgtcgcgctttcacagcaccctgcggcgcttgggacggtggctgtcaaataccaagatatgattgcggccctgcccgaagccacgcacgaggcaattgtaggggtcggtaaacagtggtcgggagcgcgagcacttgaggcgctgctgactgtggcgggtgagcttagggggcctccgctccagctcgacaccgggcagctgctgaagatcgcgaagagagggggagtaacagcggtagaggcagtgcacgcctggcgcaatgcgctcaccggggcccccttgaacctgaccccagaccaggtagtcgcaatcgcgtcacatgacgggggaaagcaagccctggaaaccgtgcaaaggttgttgccggtcctttgtcaagaccacggccttacaccggagcaagtcgtggccattgcatcccacgacggtggcaaacaggctcttgagacggttcagagacttctcccagttctctgtcaagcccacgggctgactcccgatcaagttgtagcgattgcgtcgaacattggagggaaacaagcattggagactgtccaacggctccttcccgtgttgtgtcaagcccacggtttgacgcctgcacaagtggtcgccatcgccaacaacaacggcggtaagcaggcgctggaaacagtacagcgcctgctgcctgtactgtgccaggatcatggactgaccccagaccaggtagtcgcaatcgcgaacaataatgggggaaagcaagccctggaaaccgtgcaaaggttgttgccggtcctttgtcaagaccacggccttacaccggagcaagtcgtggccattgcatcccacgacggtggcaaacaggctcttgagacggttcagagacttctcccagttctctgtcaagcccacgggctgactcccgatcaagttgtagcgattgcgtcgaacattggagggaaacaagcattggagactgtccaacggctccttcccgtgttgtgtcaagcccacggtttgacgcctgcacaagtggtcgccatcgccaacaacaacggcggtaagcaggcgctggaaacagtacagcgcctgctgcctgtactgtgccaggatcatggactgaccccagaccaggtagtcgcaatcgcgtcacatgacgggggaaagcaagccctggaaaccgtgcaaaggttgttgccggtcctttgtcaagaccacggccttacaccggagcaagtcgtggccattgcaagcaatgggggtggcaaacaggctcttgagacggttcagagacttctcccagttctctgtcaagcccacgggctgactcccgatcaagttgtagcgattgcgaataacaatggagggaaacaagcattggagactgtccaacggctccttcccgtgttgtgtcaagcccacggtttgacgcctgcacaagtggtcgccatcgccaacaacaacggcggtaagcaggcgctggaaacagtacagcgcctgctgcctgtactgtgccaggatcatggactgaccccagaccaggtagtcgcaatcgcgtcgaacattgggggaaagcaagccctggaaaccgtgcaaaggttgttgccggtcctttgtcaagaccacggccttacaccggagcaagtcgtggccattgcaaataataacggtggcaaacaggctcttgagacggttcagagacttctcccagttctctgtcaagcccacgggctgactcccgatcaagttgtagcgattgcgtcgcatgacggagggaaacaagcattggagactgtccaacggctccttcccgtgttgtgtcaagcccacggtttgacgcctgcacaagtggtcgccatcgccagccatgatggcggtaagcaggcgctggaaacagtacagcgcctgctgcctgtactgtgccaggatcatggactgacacccgaacaggtggtcgccattgcttcccacgacggaggacggccagccttggagtccatcgtagcccaattgtccaggcccgatcccgcgttggctgcgttaacgaatgaccatctggtggcgttggcatgtcttggtggacgacccgcgctcgatgcagtcaaaaagggtctgcctcatgctcccgcattgatcaaaagaaccaaccggcggattcccgagagaacttcccatcgagtcgcgggatcc

SEQ ID NO: 272 - protein, 808 aa, Artificial Sequence
  Description of Artificial Sequence: Synthetic polypeptide
ASTMDYKDHDGDYKDHDIDYKDDDDKMAPKKKRKVGIHRGVPMVDLRTLGYSQQQQEKIKPKVRSTVAQHHEALVGHGFTHAHIVALSQHPAALGTVAVKYQDMIAALPEATHEAIVGVGKQWSGARALEALLTVAGELRGPPLQLDTGQLLKIAKRGGVTAVEAVHAWRNALTGAPLNLTPDQVVAIASHDGGKQALETVQRLLPVLCQDHGLTPEQVVAIASHDGGKQALETVQRLLPVLCQAHGLTPDQVVAIASNIGGKQALETVQRLLPVLCQAHGLTPAQVVAIANNNGGKQALETVQRLLPVLCQDHGLTPDQVVAIANNNGGKQALETVQRLLPVLCQDHGLTPEQVVAIASHDGGKQALETVQRLLPVLCQAHGLTPDQVVAIASNIGGKQALETVQRLLPVLCQAHGLTPAQVVAIANNNGGKQALETVQRLLPVLCQDHGLTPDQVVAIASHDGGKQALETVQRLLPVLCQDHGLTPEQVVAIASNGGGKQALETVQRLLPVLCQAHGLTPDQVVAIANNNGGKQALETVQRLLPVLCQAHGLTPAQVVAIANNNGGKQALETVQRLLPVLCQDHGLTPDQVVAIASNIGGKQALETVQRLLPVLCQDHGLTPEQVVAIANNNGGKQALETVQRLLPVLCQAHGLTPDQVVAIASHDGGKQALETVQRLLPVLCQAHGLTPAQVVAIASHDGGKQALETVQRLLPVLCQDHGLTPEQVVAIASHDGGRPALESIVAQLSRPDPALAALTNDHLVALACLGGRPALDAVKKGLPHAPALIKRTNRRIPERTSHRVAGS

SEQ ID NO: 273 - DNA, 2424 bp, Artificial Sequence
  Description of Artificial Sequence: Synthetic polynucleotide
gctagcaccatggactacaaagaccatgacggtgattataaagatcatgacatcgattacaaggatgacgatgacaagatggcccccaagaagaagaggaaggtgggcattcaccgcggggtacctatggtggacttgaggacactcggttattcgcaacagcaacaggagaaaatcaagcctaaggtcaggagcaccgtcgcgcaacaccacgaggcgcttgtggggcatggcttcactcatgcgcatattgtcgcgctttcacagcaccctgcggcgcttgggacggtggctgtcaaataccaagatatgattgcggccctgcccgaagccacgcacgaggcaattgtaggggtcggtaaacagtggtcgggagcgcgagcacttgaggcgctgctgactgtggcgggtgagcttagggggcctccgctccagctcgacaccgggcagctgctgaagatcgcgaagagagggggagtaacagcggtagaggcagtgcacgcctggcgcaatgcgctcaccggggcccccttgaacctgaccccagaccaggtagtcgcaatcgcgtcacatgacgggggaaagcaagccctggaaaccgtgcaaaggttgttgccggtcctttgtcaagaccacggccttacaccggagcaagtcgtggccattgcaagcaatgggggtggcaaacaggctcttgagacggttcagagacttctcccagttctctgtcaagcccacgggctgactcccgatcaagttgtagcgattgcgaataacaatggagggaaacaagcattggagactgtccaacggctccttcccgtgttgtgtcaagcccacggtttgacgcctgcacaagtggtcgccatcgcctccaatattggcggtaagcaggcgctggaaacagtacagcgcctgctgcctgtactgtgccaggatcatggactgaccccagaccaggtagtcgcaatcgcgtcgaacattgggggaaagcaagccctggaaaccgtgcaaaggttgttgccggtcctttgtcaagaccacggccttacaccggagcaagtcgtggccattgcaagcaacatcggtggcaaacaggctcttgagacggttcagagacttctcccagttctctgtcaagcccacgggctgactcccgatcaagttgtagcgattgcgtcgaacattggagggaaacaagcattggagactgtccaacggctccttcccgtgttgtgtcaagcccacggtttgacgcctgcacaagtggtcgccatcgcctccaatattggcggtaagcaggcgctggaaacagtacagcgcctgctgcctgtactgtgccaggatcatggactgaccccagaccaggtagtcgcaatcgcgaacaataatgggggaaagcaagccctggaaaccgtgcaaaggttgttgccggtcctttgtcaagaccacggccttacaccggagcaagtcgtggccattgcaagcaacatcggtggcaaacaggctcttgagacggttcagagacttctcccagttctctgtcaagcccacgggctgactcccgatcaagttgtagcgattgcgtcgcatgacggagggaaacaagcattggagactgtccaacggctccttcccgtgttgtgtcaagcccacggtttgacgcctgcacaagtggtcgccatcgcctcgaatggcggcggtaagcaggcgctggaaacagtacagcgcctgctgcctgtactgtgccaggatcatggactgaccccagaccaggtagtcgcaatcgcgtcacatgacgggggaaagcaagccctggaaaccgtgcaaaggttgttgccggtcctttgtcaagaccacggccttacaccggagcaagtcgtggccattgcaagcaatgggggtggcaaacaggctcttgagacggttcagagacttctcccagttctctgtcaagcccacgggctgactcccgatcaagttgtagcgattgcgaataacaatggagggaaacaagcattggagactgtccaacggctccttcccgtgttgtgtcaagcccacggtttgacgcctgcacaagtggtcgccatcgccagccatgatggcggtaagcaggcgctggaaacagtacagcgcctgctgcctgtactgtgccaggatcatggactgacacccgaacaggtggtcgccattgcttctaacatcggaggacggccagccttggagtccatcgtagcccaattgtccaggcccgatcccgcgttggctgcgttaacgaatgaccatctggtggcgttggcatgtcttggtggacgacccgcgctcgatgcagtcaaaaagggtctgcctcatgctcccgcattgatcaaaagaaccaaccggcggattcccgagagaacttcccatcgagtcgcgggatcc

SEQ ID NO: 274 - protein, 808 aa, Artificial Sequence
  Description of Artificial Sequence: Synthetic polypeptide
ASTMDYKDHDGDYKDHDIDYKDDDDKMAPKKKRKVGIHRGVPMVDLRTLGYSQQQQEKIKPKVRSTVAQHHEALVGHGFTHAHIVALSQHPAALGTVAVKYQDMIAALPEATHEAIVGVGKQWSGARALEALLTVAGELRGPPLQLDTGQLLKIAKRGGVTAVEAVHAWRNALTGAPLNLTPDQVVAIASHDGGKQALETVQRLLPVLCQDHGLTPEQVVAIASNGGGKQALETVQRLLPVLCQAHGLTPDQVVAIANNNGGKQALETVQRLLPVLCQAHGLTPAQVVAIASNIGGKQALETVQRLLPVLCQDHGLTPDQVVAIASNIGGKQALETVQRLLPVLCQDHGLTPEQVVAIASNIGGKQALETVQRLLPVLCQAHGLTPDQVVAIASNIGGKQALETVQRLLPVLCQAHGLTPAQVVAIASNIGGKQALETVQRLLPVLCQDHGLTPDQVVAIANNNGGKQALETVQRLLPVLCQDHGLTPEQVVAIASNIGGKQALETVQRLLPVLCQAHGLTPDQVVAIASHDGGKQALETVQRLLPVLCQAHGLTPAQVVAIASNGGGKQALETVQRLLPVLCQDHGLTPDQVVAIASHDGGKQALETVQRLLPVLCQDHGLTPEQVVAIASNGGGKQALETVQRLLPVLCQAHGLTPDQVVAIANNNGGKQALETVQRLLPVLCQAHGLTPAQVVAIASHDGGKQALETVQRLLPVLCQDHGLTPEQVVAIASNIGGRPALESIVAQLSRPDPALAALTNDHLVALACLGGRPALDAVKKGLPHAPALIKRTNRRIPERTSHRVAGS

SEQ ID NO: 275 - DNA, 2424 bp, Artificial Sequence
  Description of Artificial Sequence: Synthetic polynucleotide
gctagcaccatggactacaaagaccatgacggtgattataaagatcatgacatcgattacaaggatgacgatgacaagatggcccccaagaagaagaggaaggtgggcattcaccgcggggtacctatggtggacttgaggacactcggttattcgcaacagcaacaggagaaaatcaagcctaaggtcaggagcaccgtcgcgcaacaccacgaggcgcttgtggggcatggcttcactcatgcgcatattgtcgcgctttcacagcaccctgcggcgcttgggacggtggctgtcaaataccaagatatgattgcggccctgcccgaagccacgcacgaggcaattgtaggggtcggtaaacagtggtcgggagcgcgagcacttgaggcgctgctgactgtggcgggtgagcttagggggcctccgctccagctcgacaccgggcagctgctgaagatcgcgaagagagggggagtaacagcggtagaggcagtgcacgcctggcgcaatgcgctcaccggggcccccttgaacctgaccccagaccaggtagtcgcaatcgcgtcacatgacgggggaaagcaagccctggaaaccgtgcaaaggttgttgccggtcctttgtcaagaccacggccttacaccggagcaagtcgtggccattgcatcccacgacggtggcaaacaggctcttgagacggttcagagacttctcccagttctctgtcaagcccacgggctgactcccgatcaagttgtagcgattgcgtcgaacattggagggaaacaagcattggagactgtccaacggctccttcccgtgttgtgtcaagcccacggtttgacgcctgcacaagtggtcgccatcgcctcgaatggcggcggtaagcaggcgctggaaacagtacagcgcctgctgcctgtactgtgccaggatcatggactgaccccagaccaggtagtcgcaatcgcgtcaaacggagggggaaagcaagccctggaaaccgtgcaaaggttgttgccggtcctttgtcaagaccacggccttacaccggagcaagtcgtggccattgcaagcaatgggggtggcaaacaggctcttgagacggttcagagacttctcccagttctctgtcaagcccacgggctgactcccgatcaagttgtagcgattgcgtcgcatgacggagggaaacaagcattggagactgtccaacggctccttcccgtgttgtgtcaagcccacggtttgacgcctgcacaagtggtcgccatcgcctcgaatggcggcggtaagcaggcgctggaaacagtacagcgcctgctgcctgtactgtgccaggatcatggactgaccccagaccaggtagtcgcaatcgcgaacaataatgggggaaagcaagccctggaaaccgtgcaaaggttgttgccggtcctttgtcaagaccacggccttacaccggagcaagtcgtggccattgcaagcaatgggggtggcaaacaggctcttgagacggttcagagacttctcccagttctctgtcaagcccacgggctgactcccgatcaagttgtagcgattgcgtcgcatgacggagggaaacaagcattggagactgtccaacggctccttcccgtgttgtgtcaagcccacggtttgacgcctgcacaagtggtcgccatcgcctccaatattggcggtaagcaggcgctggaaacagtacagcgcctgctgcctgtactgtgccaggatcatggactgaccccagaccaggtagtcgcaatcgcgtcaaacggagggggaaagcaagccctggaaaccgtgcaaaggttgttgccggtcctttgtcaagaccacggccttacaccggagcaagtcgtggccattgcatcccacgacggtggcaaacaggctcttgagacggttcagagacttctcccagttctctgtcaagcccacgggctgactcccgatcaagttgtagcgattgcgaataacaatggagggaaacaagcattggagactgtccaacggctccttcccgtgttgtgtcaagcccacggtttgacgcctgcacaagtggtcgccatcgcctcgaatggcggcggtaagcaggcgctggaaacagtacagcgcctgctgcctgtactgtgccaggatcatggactgacacccgaacaggtggtcgccattgcttctaacatcggaggacggccagccttggagtccatcgtagcccaattgtccaggcccgatcccgcgttggctgcgttaacgaatgaccatctggtggcgttggcatgtcttggtggacgacccgcgctcgatgcagtcaaaaagggtctgcctcatgctcccgcattgatcaaaagaaccaaccggcggattcccgagagaacttcccatcgagtcgcgggatcc

SEQ ID NO: 276 - protein, 808 aa, Artificial Sequence
  Description of Artificial Sequence: Synthetic polypeptide
ASTMDYKDHDGDYKDHDIDYKDDDDKMAPKKKRKVGIHRGVPMVDLRTLGYSQQQQEKIKPKVRSTVAQHHEALVGHGFTHAHIVALSQHPAALGTVAVKYQDMIAALPEATHEAIVGVGKQWSGARALEALLTVAGELRGPPLQLDTGQLLKIAKRGGVTAVEAVHAWRNALTGAPLNLTPDQVVAIASHDGGKQALETVQRLLPVLCQDHGLTPEQVVAIASHDGGKQALETVQRLLPVLCQAHGLTPDQVVAIASNIGGKQALETVQRLLPVLCQAHGLTPAQVVAIASNGGGKQALETVQRLLPVLCQDHGLTPDQVVAIASNGGGKQALETVQRLLPVLCQDHGLTPEQVVAIASNGGGKQALETVQRLLPVLCQAHGLTPDQVVAIASHDGGKQALETVQRLLPVLCQAHGLTPAQVVAIASNGGGKQALETVQRLLPVLCQDHGLTPDQVVAIANNNGGKQALETVQRLLPVLCQDHGLTPEQVVAIASNGGGKQALETVQRLLPVLCQAHGLTPDQVVAIASHDGGKQALETVQRLLPVLCQAHGLTPAQVVAIASNIGGKQALETVQRLLPVLCQDHGLTPDQVVAIASNGGGKQALETVQRLLPVLCQDHGLTPEQVVAIASHDGGKQALETVQRLLPVLCQAHGLTPDQVVAIANNNGGKQALETVQRLLPVLCQAHGLTPAQVVAIASNGGGKQALETVQRLLPVLCQDHGLTPEQVVAIASNIGGRPALESIVAQLSRPDPALAALTNDHLVALACLGGRPALDAVKKGLPHAPALIKRTNRRIPERTSHRVAGS

SEQ ID NO: 277 - DNA, 2424 bp, Artificial Sequence
  Description of Artificial Sequence: Synthetic polynucleotide
gctagcaccatggactacaaagaccatgacggtgattataaagatcatgacatcgattacaaggatgacgatgacaagatggcccccaagaagaagaggaaggtgggcattcaccgcggggtacctatggtggacttgaggacactcggttattcgcaacagcaacaggagaaaatcaagcctaaggtcaggagcaccgtcgcgcaacaccacgaggcgcttgtggggcatggcttcactcatgcgcatattgtcgcgctttcacagcaccctgcggcgcttgggacggtggctgtcaaataccaagatatgattgcggccctgcccgaagccacgcacgaggcaattgtaggggtcggtaaacagtggtcgggagcgcgagcacttgaggcgctgctgactgtggcgggtgagcttagggggcctccgctccagctcgacaccgggcagctgctgaagatcgcgaagagagggggagtaacagcggtagaggcagtgcacgcctggcgcaatgcgctcaccggggcccccttgaacctgaccccagaccaggtagtcgcaatcgcgaacaataatgggggaaagcaagccctggaaaccgtgcaaaggttgttgccggtcctttgtcaagaccacggccttacaccggagcaagtcgtggccattgcaagcaacatcggtggcaaacaggctcttgagacggttcagagacttctcccagttctctgtcaagcccacgggctgactcccgatcaagttgtagcgattgcgtcgaacattggagggaaacaagcattggagactgtccaacggctccttcccgtgttgtgtcaagcccacggtttgacgcctgcacaagtggtcgccatcgcctccaatattggcggtaagcaggcgctggaaacagtacagcgcctgctgcctgtactgtgccaggatcatggactgaccccagaccaggtagtcgcaatcgcgtcgaacattgggggaaagcaagccctggaaaccgtgcaaaggttgttgccggtcctttgtcaagaccacggccttacaccggagcaagtcgtggccattgcaagcaatgggggtggcaaacaggctcttgagacggttcagagacttctcccagttctctgtcaagcccacgggctgactcccgatcaagttgtagcgattgcgaataacaatggagggaaacaagcattggagactgtccaacggctccttcccgtgttgtgtcaagcccacggtttgacgcctgcacaagtggtcgccatcgcctccaatattggcggtaagcaggcgctggaaacagtacagcgcctgctgcctgtactgtgccaggatcatggactgaccccagaccaggtagtcgcaatcgcgtcacatgacgggggaaagcaagccctggaaaccgtgcaaaggttgttgccggtcctttgtcaagaccacggccttacaccggagcaagtcgtggccattgcaagcaatgggggtggcaaacaggctcttgagacggttcagagacttctcccagttctctgtcaagcccacgggctgactcccgatcaagttgtagcgattgcgaataacaatggagggaaacaagcattggagactgtccaacggctccttcccgtgttgtgtcaagcccacggtttgacgcctgcacaagtggtcgccatcgcctccaatattggcggtaagcaggcgctggaaacagtacagcgcctgctgcctgtactgtgccaggatcatggactgaccccagaccaggtagtcgcaatcgcgtcgaacattgggggaaagcaagccctggaaaccgtgcaaaggttgttgccggtcctttgtcaagaccacggccttacaccggagcaagtcgtggccattgcaagcaatgggggtggcaaacaggctcttgagacggttcagagacttctcccagttctctgtcaagcccacgggctgactcccgatcaagttgtagcgattgcgtcgaacattggagggaaacaagcattggagactgtccaacggctccttcccgtgttgtgtcaagcccacggtttgacgcctgcacaagtggtcgccatcgcctcgaatggcggcggtaagcaggcgctggaaacagtacagcgcctgctgcctgtactgtgccaggatcatggactgacacccgaacaggtggtcgccattgcttctaacatcggaggacggccagccttggagtccatcgtagcccaattgtccaggcccgatcccgcgttggctgcgttaacgaatgaccatctggtggcgttggcatgtcttggtggacgacccgcgctcgatgcagtcaaaaagggtctgcctcatgctcccgcattgatcaaaagaaccaaccggcggattcccgagagaacttcccatcgagtcgcgggatcc

SEQ ID NO: 278 - protein, 808 aa, Artificial Sequence
  Description of Artificial Sequence: Synthetic polypeptide
ASTMDYKDHDGDYKDHDIDYKDDDDKMAPKKKRKVGIHRGVPMVDLRTLGYSQQQQEKIKPKVRSTVAQHHEALVGHGFTHAHIVALSQHPAALGTVAVKYQDMIAALPEATHEAIVGVGKQWSGARALEALLTVAGELRGPPLQLDTGQLLKIAKRGGVTAVEAVHAWRNALTGAPLNLTPDQVVAIANNNGGKQALETVQRLLPVLCQDHGLTPEQVVAIASNIGGKQALETVQRLLPVLCQAHGLTPDQVVAIASNIGGKQALETVQRLLPVLCQAHGLTPAQVVAIASNIGGKQALETVQRLLPVLCQDHGLTPDQVVAIASNIGGKQALETVQRLLPVLCQDHGLTPEQVVAIASNGGGKQALETVQRLLPVLCQAHGLTPDQVVAIANNNGGKQALETVQRLLPVLCQAHGLTPAQVVAIASNIGGKQALETVQRLLPVLCQDHGLTPDQVVAIASHDGGKQALETVQRLLPVLCQDHGLTPEQVVAIASNGGGKQALETVQRLLPVLCQAHGLTPDQVVAIANNNGGKQALETVQRLLPVLCQAHGLTPAQVVAIASNIGGKQALETVQRLLPVLCQDHGLTPDQVVAIASNIGGKQALETVQRLLPVLCQDHGLTPEQVVAIASNGGGKQALETVQRLLPVLCQAHGLTPDQVVAIASNIGGKQALETVQRLLPVLCQAHGLTPAQVVAIASNGGGKQALETVQRLLPVLCQDHGLTPEQVVAIASNIGGRPALESIVAQLSRPDPALAALTNDHLVALACLGGRPALDAVKKGLPHAPALIKRTNRRIPERTSHRVAGS

SEQ ID NO: 279 - DNA, 2322 bp, Artificial Sequence
  Description of Artificial Sequence: Synthetic polynucleotide
gctagcaccatggactacaaagaccatgacggtgattataaagatcatgacatcgattacaaggatgacgatgacaagatggcccccaagaagaagaggaaggtgggcattcaccgcggggtacctatggtggacttgaggacactcggttattcgcaacagcaacaggagaaaatcaagcctaaggtcaggagcaccgtcgcgcaacaccacgaggcgcttgtggggcatggcttcactcatgcgcatattgtcgcgctttcacagcaccctgcggcgcttgggacggtggctgtcaaataccaagatatgattgcggccctgcccgaagccacgcacgaggcaattgtaggggtcggtaaacagtggtcgggagcgcgagcacttgaggcgctgctgactgtggcgggtgagcttagggggcctccgctccagctcgacaccgggcagctgctgaagatcgcgaagagagggggagtaacagcggtagaggcagtgcacgcctggcgcaatgcgctcaccggggcccccttgaacctgaccccagaccaggtagtcgcaatcgcgtcaaacggagggggaaagcaagccctggaaaccgtgcaaaggttgttgccggtcctttgtcaagaccacggccttacaccggagcaagtcgtggccattgcaaataataacggtggcaaacaggctcttgagacggttcagagacttctcccagttctctgtcaagcccacgggctgactcccgatcaagttgtagcgattgcgtcgcatgacggagggaaacaagcattggagactgtccaacggctccttcccgtgttgtgtcaagcccacggtttgacgcctgcacaagtggtcgccatcgccagccatgatggcggtaagcaggcgctggaaacagtacagcgcctgctgcctgtactgtgccaggatcatggactgaccccagaccaggtagtcgcaatcgcgtcaaacggagggggaaagcaagccctggaaaccgtgcaaaggttgttgccggtcctttgtcaagaccacggccttacaccggagcaagtcgtggccattgcaagcaacatcggtggcaaacaggctcttgagacggttcagagacttctcccagttctctgtcaagcccacgggctgactcccgatcaagttgtagcgattgcgtcgcatgacggagggaaacaagcattggagactgtccaacggctccttcccgtgttgtgtcaagcccacggtttgacgcctgcacaagtggtcgccatcgccaacaacaacggcggtaagcaggcgctggaaacagtacagcgcctgctgcctgtactgtgccaggatcatggactgaccccagaccaggtagtcgcaatcgcgtcacatgacgggggaaagcaagccctggaaaccgtgcaaaggttgttgccggtcctttgtcaagaccacggccttacaccggagcaagtcgtggccattgcatcccacgacggtggcaaacaggctcttgagacggttcagagacttctcccagttctctgtcaagcccacgggctgactcccgatcaagttgtagcgattgcgtcgaacattggagggaaacaagcattggagactgtccaacggctccttcccgtgttgtgtcaagcccacggtttgacgcctgcacaagtggtcgccatcgccagccatgatggcggtaagcaggcgctggaaacagtacagcgcctgctgcctgtactgtgccaggatcatggactgaccccagaccaggtagtcgcaatcgcgtcacatgacgggggaaagcaagccctggaaaccgtgcaaaggttgttgccggtcctttgtcaagaccacggccttacaccggagcaagtcgtggccattgcaagcaacatcggtggcaaacaggctcttgagacggttcagagacttctcccagttctctgtcaagcccacgggctgactcccgatcaagttgtagcgattgcgaataacaatggagggaaacaagcattggagactgtccaacggctccttcccgtgttgtgtcaagcccacggtctgacacccgaacaggtggtcgccattgcttcccacgacggaggacggccagccttggagtccatcgtagcccaattgtccaggcccgatcccgcgttggctgcgttaacgaatgaccatctggtggcgttggcatgtcttggtggacgacccgcgctcgatgcagtcaaaaagggtctgcctcatgctcccgcattgatcaaaagaaccaaccggcggattcccgagagaacttcccatcgagtcgcgggatcc

SEQ ID NO: 280 - protein, 774 aa, Artificial Sequence
  Description of Artificial Sequence: Synthetic polypeptide
ASTMDYKDHDGDYKDHDIDYKDDDDKMAPKKKRKVGIHRGVPMVDLRTLGYSQQQQEKIKPKVRSTVAQHHEALVGHGFTHAHIVALSQHPAALGTVAVKYQDMIAALPEATHEAIVGVGKQWSGARALEALLTVAGELRGPPLQLDTGQLLKIAKRGGVTAVEAVHAWRNALTGAPLNLTPDQVVAIASNGGGKQALETVQRLLPVLCQDHGLTPEQVVAIANNNGGKQALETVQRLLPVLCQAHGLTPDQVVAIASHDGGKQALETVQRLLPVLCQAHGLTPAQVVAIASHDGGKQALETVQRLLPVLCQDHGLTPDQVVAIASNGGGKQALETVQRLLPVLCQDHGLTPEQVVAIASNIGGKQALETVQRLLPVLCQAHGLTPDQVVAIASHDGGKQALETVQRLLPVLCQAHGLTPAQVVAIANNNGGKQALETVQRLLPVLCQDHGLTPDQVVAIASHDGGKQALETVQRLLPVLCQDHGLTPEQVVAIASHDGGKQALETVQRLLPVLCQAHGLTPDQVVAIASNIGGKQALETVQRLLPVLCQAHGLTPAQVVAIASHDGGKQALETVQRLLPVLCQDHGLTPDQVVAIASHDGGKQALETVQRLLPVLCQDHGLTPEQVVAIASNIGGKQALETVQRLLPVLCQAHGLTPDQVVAIANNNGGKQALETVQRLLPVLCQAHGLTPEQVVAIASHDGGRPALESIVAQLSRPDPALAALTNDHLVALACLGGRPALDAVKKGLPHAPALIKRTNRRIPERTSHRVAGS

SEQ ID NO: 281 - DNA, 2424 bp, Artificial Sequence
  Description of Artificial Sequence: Synthetic polynucleotide
gctagcaccatggactacaaagaccatgacggtgattataaagatcatgacatcgattacaaggatgacgatgacaagatggcccccaagaagaagaggaaggtgggcattcaccgcggggtacctatggtggacttgaggacactcggttattcgcaacagcaacaggagaaaatcaagcctaaggtcaggagcaccgtcgcgcaacaccacgaggcgcttgtggggcatggcttcactcatgcgcatattgtcgcgctttcacagcaccctgcggcgcttgggacggtggctgtcaaataccaagatatgattgcggccctgcccgaagccacgcacgaggcaattgtaggggtcggtaaacagtggtcgggagcgcgagcacttgaggcgctgctgactgtggcgggtgagcttagggggcctccgctccagctcgacaccgggcagctgctgaagatcgcgaagagagggggagtaacagcggtagaggcagtgcacgcctggcgcaatgcgctcaccggggcccccttgaacctgaccccagaccaggtagtcgcaatcgcgaacaataatgggggaaagcaagccctggaaaccgtgcaaaggttgttgccggtcctttgtcaagaccacggccttacaccggagcaagtcgtggccattgcatcccacgacggtggcaaacaggctcttgagacggttcagagacttctcccagttctctgtcaagcccacgggctgactcccgatcaagttgtagcgattgcgtccaacggtggagggaaacaagcattggagactgtccaacggctccttcccgtgttgtgtcaagcccacggtttgacgcctgcacaagtggtcgccatcgcctcgaatggcggcggtaagcaggcgctggaaacagtacagcgcctgctgcctgtactgtgccaggatcatggactgaccccagaccaggtagtcgcaatcgcgtcgaacattgggggaaagcaagccctggaaaccgtgcaaaggttgttgccggtcctttgtcaagaccacggccttacaccggagcaagtcgtggccattgcaaataataacggtggcaaacaggctcttgagacggttcagagacttctcccagttctctgtcaagcccacgggctgactcccgatcaagttgtagcgattgcgtcgaacattggagggaaacaagcattggagactgtccaacggctccttcccgtgttgtgtcaagcccacggtttgacgcctgcacaagtggtcgccatcgccagccatgatggcggtaagcaggcgctggaaacagtacagcgcctgctgcctgtactgtgccaggatcatggactgaccccagaccaggtagtcgcaatcgcgaacaataatgggggaaagcaagccctggaaaccgtgcaaaggttgttgccggtcctttgtcaagaccacggccttacaccggagcaagtcgtggccattgcatcccacgacggtggcaaacaggctcttgagacggttcagagacttctcccagttctctgtcaagcccacgggctgactcccgatcaagttgtagcgattgcgtccaacggtggagggaaacaagcattggagactgtccaacggctccttcccgtgttgtgtcaagcccacggtttgacgcctgcacaagtggtcgccatcgccaacaacaacggcggtaagcaggcgctggaaacagtacagcgcctgctgcctgtactgtgccaggatcatggactgaccccagaccaggtagtcgcaatcgcgaacaataatgggggaaagcaagccctggaaaccgtgcaaaggttgttgccggtcctttgtcaagaccacggccttacaccggagcaagtcgtggccattgcaagcaacatcggtggcaaacaggctcttgagacggttcagagacttctcccagttctctgtcaagcccacgggctgactcccgatcaagttgtagcgattgcgtccaacggtggagggaaacaagcattggagactgtccaacggctccttcccgtgttgtgtcaagcccacggtttgacgcctgcacaagtggtcgccatcgcctcgaatggcggcggtaagcaggcgctggaaacagtacagcgcctgctgcctgtactgtgccaggatcatggactgacacccgaacaggtggtcgccattgcttctaatgggggaggacggccagccttggagtccatcgtagcccaattgtccaggcccgatcccgcgttggctgcgttaacgaatgaccatctggtggcgttggcatgtcttggtggacgacccgcgctcgatgcagtcaaaaagggtctgcctcatgctcccgcattgatcaaaagaaccaaccggcggattcccgagagaacttcccatcgagtcgcgggatcc

SEQ ID NO: 282 - protein, 808 aa, Artificial Sequence
  Description of Artificial Sequence: Synthetic polypeptide
ASTMDYKDHDGDYKDHDIDYKDDDDKMAPKKKRKVGIHRGVPMVDLRTLGYSQQQQEKIKPKVRSTVAQHHEALVGHGFTHAHIVALSQHPAALGTVAVKYQDMIAALPEATHEAIVGVGKQWSGARALEALLTVAGELRGPPLQLDTGQLLKIAKRGGVTAVEAVHAWRNALTGAPLNLTPDQVVAIANNNGGKQALETVQRLLPVLCQDHGLTPEQVVAIASHDGGKQALETVQRLLPVLCQAHGLTPDQVVAIASNGGGKQALETVQRLLPVLCQAHGLTPAQVVAIASNGGGKQALETVQRLLPVLCQDHGLTPDQVVAIASNIGGKQALETVQRLLPVLCQDHGLTPEQVVAIANNNGGKQALETVQRLLPVLCQAHGLTPDQVVAIASNIGGKQALETVQRLLPVLCQAHGLTPAQVVAIASHDGGKQALETVQRLLPVLCQDHGLTPDQVVAIANNNGGKQALETVQRLLPVLCQDHGLTPEQVVAIASHDGGKQALETVQRLLPVLCQAHGLTPDQVVAIASNGGGKQALETVQRLLPVLCQAHGLTPAQVVAIANNNGGKQALETVQRLLPVLCQDHGLTPDQVVAIANNNGGKQALETVQRLLPVLCQDHGLTPEQVVAIASNIGGKQALETVQRLLPVLCQAHGLTPDQVVAIASNGGGKQALETVQRLLPVLCQAHGLTPAQVVAIASNGGGKQALETVQRLLPVLCQDHGLTPEQVVAIASNGGGRPALESIVAQLSRPDPALAALTNDHLVALACLGGRPALDAVKKGLPHAPALIKRTNRRIPERTSHRVAGS

SEQ ID NO: 283 - DNA, 2424 bp, Artificial Sequence
  Description of Artificial Sequence: Synthetic polynucleotide
gctagcaccatggactacaaagaccatgacggtgattataaagatcatgacatcgattacaaggatgacgatgacaagatggcccccaagaagaagaggaaggtgggcattcaccgcggggtacctatggtggacttgaggacactcggttattcgcaacagcaacaggagaaaatcaagcctaaggtcaggagcaccgtcgcgcaacaccacgaggcgcttgtggggcatggcttcactcatgcgcatattgtcgcgctttcacagcaccctgcggcgcttgggacggtggctgtcaaataccaagatatgattgcggccctgcccgaagccacgcacgaggcaattgtaggggtcggtaaacagtggtcgggagcgcgagcacttgaggcgctgctgactgtggcgggtgagcttagggggcctccgctccagctcgacaccgggcagctgctgaagatcgcgaagagagggggagtaacagcggtagaggcagtgcacgcctggcgcaatgcgctcaccggggcccccttgaacctgaccccagaccaggtagtcgcaatcgcgtcaaacggagggggaaagcaagccctggaaaccgtgcaaaggttgttgccggtcctttgtcaagaccacggccttacaccggagcaagtcgtggccattgcatcccacgacggtggcaaacaggctcttgagacggttcagagacttctcccagttctctgtcaagcccacgggctgactcccgatcaagttgtagcgattgcgaataacaatggagggaaacaagcattggagactgtccaacggctccttcccgtgttgtgtcaagcccacggtttgacgcctgcacaagtggtcgccatcgccaacaacaacggcggtaagcaggcgctggaaacagtacagcgcctgctgcctgtactgtgccaggatcatggactgaccccagaccaggtagtcgcaatcgcgtcaaacggagggggaaagcaagccctggaaaccgtgcaaaggttgttgccggtcctttgtcaagaccacggccttacaccggagcaagtcgtggccattgcaaataataacggtggcaaacaggctcttgagacggttcagagacttctcccagttctctgtcaagcccacgggctgactcccgatcaagttgtagcgattgcgtcgcatgacggagggaaacaagcattggagactgtccaacggctccttcccgtgttgtgtcaagcccacggtttgacgcctgcacaagtggtcgccatcgcctcgaatggcggcggtaagcaggcgctggaaacagtacagcgcctgctgcctgtactgtgccaggatcatggactgaccccagaccaggtagtcgcaatcgcgtcaaacggagggggaaagcaagccctggaaaccgtgcaaaggttgttgccggtcctttgtcaagaccacggccttacaccggagcaagtcgtggccattgcaagcaacatcggtggcaaacaggctcttgagacggttcagagacttctcccagttctctgtcaagcccacgggctgactcccgatcaagttgtagcgattgcgtcgcatgacggagggaaacaagcattggagactgtccaacggctccttcccgtgttgtgtcaagcccacggtttgacgcctgcacaagtggtcgccatcgccagccatgatggcggtaagcaggcgctggaaacagtacagcgcctgctgcctgtactgtgccaggatcatggactgaccccagaccaggtagtcgcaatcgcgtcaaacggagggggaaagcaagccctggaaaccgtgcaaaggttgttgccggtcctttgtcaagaccacggccttacaccggagcaagtcgtggccattgcaaataataacggtggcaaacaggctcttgagacggttcagagacttctcccagttctctgtcaagcccacgggctgactcccgatcaagttgtagcgattgcgaataacaatggagggaaacaagcattggagactgtccaacggctccttcccgtgttgtgtcaagcccacggtttgacgcctgcacaagtggtcgccatcgcctcgaatggcggcggtaagcaggcgctggaaacagtacagcgcctgctgcctgtactgtgccaggatcatggactgacacccgaacaggtggtcgccattgcttctaatgggggaggacggccagccttggagtccatcgtagcccaattgtccaggcccgatcccgcgttggctgcgttaacgaatgaccatctggtggcgttggcatgtcttggtggacgacccgcgctcgatgcagtcaaaaagggtctgcctcatgctcccgcattgatcaaaagaaccaaccggcggattcccgagagaacttcccatcgagtcgcgggatcc

SEQ ID NO: 284 - protein, 808 aa, Artificial Sequence
  Description of Artificial Sequence: Synthetic polypeptide
ASTMDYKDHDGDYKDHDIDYKDDDDKMAPKKKRKVGIHRGVPMVDLRTLGYSQQQQEKIKPKVRSTVAQHHEALVGHGFTHAHIVALSQHPAALGTVAVKYQDMIAALPEATHEAIVGVGKQWSGARALEALLTVAGELRGPPLQLDTGQLLKIAKRGGVTAVEAVHAWRNALTGAPLNLTPDQVVAIASNGGGKQALETVQRLLPVLCQDHGLTPEQVVAIASHDGGKQALETVQRLLPVLCQAHGLTPDQVVAIANNNGGKQALETVQRLLPVLCQAHGLTPAQVVAIANNNGGKQALETVQRLLPVLCQDHGLTPDQVVAIASNGGGKQALETVQRLLPVLCQDHGLTPEQVVAIANNNGGKQALETVQRLLPVLCQAHGLTPDQVVAIASHDGGKQALETVQRLLPVLCQAHGLTPAQVVAIASNGGGKQALETVQRLLPVLCQDHGLTPDQVVAIASNGGGKQALETVQRLLPVLCQDHGLTPEQVVAIASNIGGKQALETVQRLLPVLCQAHGLTPDQVVAIASHDGGKQALETVQRLLPVLCQAHGLTPAQVVAIASHDGGKQALETVQRLLPVLCQDHGLTPDQVVAIASNGGGKQALETVQRLLPVLCQDHGLTPEQVVAIANNNGGKQALETVQRLLPVLCQAHGLTPDQVVAIANNNGGKQALETVQRLLPVLCQAHGLTPAQVVAIASNGGGKQALETVQRLLPVLCQDHGLTPEQVVAIASNGGGRPALESIVAQLSRPDPALAALTNDHLVALACLGGRPALDAVKKGLPHAPALIKRTNRRIPERTSHRVAGS

SEQ ID NO: 285 - DNA, 2322 bp, Artificial Sequence
  Description of Artificial Sequence: Synthetic polynucleotide
gctagcaccatggactacaaagaccatgacggtgattataaagatcatgacatcgattacaaggatgacgatgacaagatggcccccaagaagaagaggaaggtgggcattcaccgcggggtacctatggtggacttgaggacactcggttattcgcaacagcaacaggagaaaatcaagcctaaggtcaggagcaccgtcgcgcaacaccacgaggcgcttgtggggcatggcttcactcatgcgcatattgtcgcgctttcacagcaccctgcggcgcttgggacggtggctgtcaaataccaagatatgattgcggccctgcccgaagccacgcacgaggcaattgtaggggtcggtaaacagtggtcgggagcgcgagcacttgaggcgctgctgactgtggcgggtgagcttagggggcctccgctccagctcgacaccgggcagctgctgaagatcgcgaagagagggggagtaacagcggtagaggcagtgcacgcctggcgcaatgcgctcaccggggcccccttgaacctgaccccagaccaggtagtcgcaatcgcgtcacatgacgggggaaagcaagccctggaaaccgtgcaaaggttgttgccggtcctttgtcaagaccacggccttacaccggagcaagtcgtggccattgcatcccacgacggtggcaaacaggctcttgagacggttcagagacttctcccagttctctgtcaagcccacgggctgactcccgatcaagttgtagcgattgcgtcgcatgacggagggaaacaagcattggagactgtccaacggctccttcccgtgttgtgtcaagcccacggtttgacgcctgcacaagtggtcgccatcgcctccaatattggcggtaagcaggcgctggaaacagtacagcgcctgctgcctgtactgtgccaggatcatggactgaccccagaccaggtagtcgcaatcgcgaacaataatgggggaaagcaagccctggaaaccgtgcaaaggttgttgccggtcctttgtcaagaccacggccttacaccggagcaagtcgtggccattgcaagcaacatcggtggcaaacaggctcttgagacggttcagagacttctcccagttctctgtcaagcccacgggctgactcccgatcaagttgtagcgattgcgtcgcatgacggagggaaacaagcattggagactgtccaacggctccttcccgtgttgtgtcaagcccacggtttgacgcctgcacaagtggtcgccatcgcctccaatattggcggtaagcaggcgctggaaacagtacagcgcctgctgcctgtactgtgccaggatcatggactgaccccagaccaggtagtcgcaatcgcgtcaaacggagggggaaagcaagccctggaaaccgtgcaaaggttgttgccggtcctttgtcaagaccacggccttacaccggagcaagtcgtggccattgcaaataataacggtggcaaacaggctcttgagacggttcagagacttctcccagttctctgtcaagcccacgggctgactcccgatcaagttgtagcgattgcgtcgaacattggagggaaacaagcattggagactgtccaacggctccttcccgtgttgtgtcaagcccacggtttgacgcctgcacaagtggtcgccatcgccagccatgatggcggtaagcaggcgctggaaacagtacagcgcctgctgcctgtactgtgccaggatcatggactgaccccagaccaggtagtcgcaatcgcgtcgaacattgggggaaagcaagccctggaaaccgtgcaaaggttgttgccggtcctttgtcaagaccacggccttacaccggagcaagtcgtggccattgcaaataataacggtggcaaacaggctcttgagacggttcagagacttctcccagttctctgtcaagcccacgggctgactcccgatcaagttgtagcgattgcgtcgcatgacggagggaaacaagcattggagactgtccaacggctccttcccgtgttgtgtcaagcccacggtctgacacccgaacaggtggtcgccattgcttcccacgacggaggacggccagccttggagtccatcgtagcccaattgtccaggcccgatcccgcgttggctgcgttaacgaatgaccatctggtggcgttggcatgtcttggtggacgacccgcgctcgatgcagtcaaaaagggtctgcctcatgctcccgcattgatcaaaagaaccaaccggcggattcccgagagaacttcccatcgagtcgcgggatcc

SEQ ID NO: 286 - protein, 774 aa, Artificial Sequence
  Description of Artificial Sequence: Synthetic polypeptide
ASTMDYKDHDGDYKDHDIDYKDDDDKMAPKKKRKVGIHRGVPMVDLRTLGYSQQQQEKIKPKVRSTVAQHHEALVGHGFTHAHIVALSQHPAALGTVAVKYQDMIAALPEATHEAIVGVGKQWSGARALEALLTVAGELRGPPLQLDTGQLLKIAKRGGVTAVEAVHAWRNALTGAPLNLTPDQVVAIASHDGGKQALETVQRLLPVLCQDHGLTPEQVVAIASHDGGKQALETVQRLLPVLCQAHGLTPDQVVAIASHDGGKQALETVQRLLPVLCQAHGLTPAQVVAIASNIGGKQALETVQRLLPVLCQDHGLTPDQVVAIANNNGGKQALETVQRLLPVLCQDHGLTPEQVVAIASNIGGKQALETVQRLLPVLCQAHGLTPDQVVAIASHDGGKQALETVQRLLPVLCQAHGLTPAQVVAIASNIGGKQALETVQRLLPVLCQDHGLTPDQVVAIASNGGGKQALETVQRLLPVLCQDHGLTPEQVVAIANNNGGKQALETVQRLLPVLCQAHGLTPDQVVAIASNIGGKQALETVQRLLPVLCQAHGLTPAQVVAIASHDGGKQALETVQRLLPVLCQDHGLTPDQVVAIASNIGGKQALETVQRLLPVLCQDHGLTPEQVVAIANNNGGKQALETVQRLLPVLCQAHGLTPDQVVAIASHDGGKQALETVQRLLPVLCQAHGLTPEQVVAIASHDGGRPALESIVAQLSRPDPALAALTNDHLVALACLGGRPALDAVKKGLPHAPALIKRTNRRIPERTSHRVAGS

SEQ ID NO: 287 - DNA, 2424 bp, Artificial Sequence
  Description of Artificial Sequence: Synthetic polynucleotide
gctagcaccatggactacaaagaccatgacggtgattataaagatcatgacatcgattacaaggatgacgatgacaagatggcccccaagaagaagaggaaggtgggcattcaccgcggggtacctatggtggacttgaggacactcggttattcgcaacagcaacaggagaaaatcaagcctaaggtcaggagcaccgtcgcgcaacaccacgaggcgcttgtggggcatggcttcactcatgcgcatattgtcgcgctttcacagcaccctgcggcgcttgggacggtggctgtcaaataccaagatatgattgcggccctgcccgaagccacgcacgaggcaattgtaggggtcggtaaacagtggtcgggagcgcgagcacttgaggcgctgctgactgtggcgggtgagcttagggggcctccgctccagctcgacaccgggcagctgctgaagatcgcgaagagagggggagtaacagcggtagaggcagtgcacgcctggcgcaatgcgctcaccggggcccccttgaacctgaccccagaccaggtagtcgcaatcgcgtcacatgacgggggaaagcaagccctggaaaccgtgcaaaggttgttgccggtcctttgtcaagaccacggccttacaccggagcaagtcgtggccattgcatcccacgacggtggcaaacaggctcttgagacggttcagagacttctcccagttctctgtcaagcccacgggctgactcccgatcaagttgtagcgattgcgtccaacggtggagggaaacaagcattggagactgtccaacggctccttcccgtgttgtgtcaagcccacggtttgacgcctgcacaagtggtcgccatcgcctcgaatggcggcggtaagcaggcgctggaaacagtacagcgcctgctgcctgtactgtgccaggatcatggactgaccccagaccaggtagtcgcaatcgcgtcaaacggagggggaaagcaagccctggaaaccgtgcaaaggttgttgccggtcctttgtcaagaccacggccttacaccggagcaagtcgtggccattgcaagcaatgggggtggcaaacaggctcttgagacggttcagagacttctcccagttctctgtcaagcccacgggctgactcccgatcaagttgtagcgattgcgaataacaatggagggaaacaagcattggagactgtccaacggctccttcccgtgttgtgtcaagcccacggtttgacgcctgcacaagtggtcgccatcgcctcgaatggcggcggtaagcaggcgctggaaacagtacagcgcctgctgcctgtactgtgccaggatcatggactgaccccagaccaggtagtcgcaatcgcgtcaaacggagggggaaagcaagccctggaaaccgtgcaaaggttgttgccggtcctttgtcaagaccacggccttacaccggagcaagtcgtggccattgcaagcaatgggggtggcaaacaggctcttgagacggttcagagacttctcccagttctctgtcaagcccacgggctgactcccgatcaagttgtagcgattgcgtcgcatgacggagggaaacaagcattggagactgtccaacggctccttcccgtgttgtgtcaagcccacggtttgacgcctgcacaagtggtcgccatcgcctcgaatggcggcggtaagcaggcgctggaaacagtacagcgcctgctgcctgtactgtgccaggatcatggactgaccccagaccaggtagtcgcaatcgcgaacaataatgggggaaagcaagccctggaaaccgtgcaaaggttgttgccggtcctttgtcaagaccacggccttacaccggagcaagtcgtggccattgcatcccacgacggtggcaaacaggctcttgagacggttcagagacttctcccagttctctgtcaagcccacgggctgactcccgatcaagttgtagcgattgcgtccaacggtggagggaaacaagcattggagactgtccaacggctccttcccgtgttgtgtcaagcccacggtttgacgcctgcacaagtggtcgccatcgcctccaatattggcggtaagcaggcgctggaaacagtacagcgcctgctgcctgtactgtgccaggatcatggactgacacccgaacaggtggtcgccattgcttctaacatcggaggacggccagccttggagtccatcgtagcccaattgtccaggcccgatcccgcgttggctgcgttaacgaatgaccatctggtggcgttggcatgtcttggtggacgacccgcgctcgatgcagtcaaaaagggtctgcctcatgctcccgcattgatcaaaagaaccaaccggcggattcccgagagaacttcccatcgagtcgcgggatcc

SEQ ID NO: 288 - protein, 808 aa, Artificial Sequence
  Description of Artificial Sequence: Synthetic polypeptide
ASTMDYKDHDGDYKDHDIDYKDDDDKMAPKKKRKVGIHRGVPMVDLRTLGYSQQQQEKIKPKVRSTVAQHHEALVGHGFTHAHIVALSQHPAALGTVAVKYQDMIAALPEATHEAIVGVGKQWSGARALEALLTVAGELRGPPLQLDTGQLLKIAKRGGVTAVEAVHAWRNALTGAPLNLTPDQVVAIASHDGGKQALETVQRLLPVLCQDHGLTPEQVVAIASHDGGKQALETVQRLLPVLCQAHGLTPDQVVAIASNGGGKQALETVQRLLPVLCQAHGLTPAQVVAIASNGGGKQALETVQRLLPVLCQDHGLTPDQVVAIASNGGGKQALETVQRLLPVLCQDHGLTPEQVVAIASNGGGKQALETVQRLLPVLCQAHGLTPDQVVAIANNNGGKQALETVQRLLPVLCQAHGLTPAQVVAIASNGGGKQALETVQRLLPVLCQDHGLTPDQVVAIASNGGGKQALETVQRLLPVLCQDHGLTPEQVVAIASNGGGKQALETVQRLLPVLCQAHGLTPDQVVAIASHDGGKQALETVQRLLPVLCQAHGLTPAQVVAIASNGGGKQALETVQRLLPVLCQDHGLTPDQVVAIANNNGGKQALETVQRLLPVLCQDHGLTPEQVVAIASHDGGKQALETVQRLLPVLCQAHGLTPDQVVAIASNGGGKQALETVQRLLPVLCQAHGLTPAQVVAIASNIGGKQALETVQRLLPVLCQDHGLTPEQVVAIASNIGGRPALESIVAQLSRPDPALAALTNDHLVALACLGGRPALDAVKKGLPHAPALIKRTNRRIPERTSHRVAGS

SEQ ID NO: 289 - DNA, 2424 bp, Artificial Sequence
  Description of Artificial Sequence: Synthetic polynucleotide
gctagcaccatggactacaaagaccatgacggtgattataaagatcatgacatcgattacaaggatgacgatgacaagatggcccccaagaagaagaggaaggtgggcattcaccgcggggtacctatggtggacttgaggacactcggttattcgcaacagcaacaggagaaaatcaagcctaaggtcaggagcaccgtcgcgcaacaccacgaggcgcttgtggggcatggcttcactcatgcgcatattgtcgcgctttcacagcaccctgcggcgcttgggacggtggctgtcaaataccaagatatgattgcggccctgcccgaagccacgcacgaggcaattgtaggggtcggtaaacagtggtcgggagcgcgagcacttgaggcgctgctgactgtggcgggtgagcttagggggcctccgctccagctcgacaccgggcagctgctgaagatcgcgaagagagggggagtaacagcggtagaggcagtgcacgcctggcgcaatgcgctcaccggggcccccttgaacctgaccccagaccaggtagtcgcaatcgcgtcaaacggagggggaaagcaagccctggaaaccgtgcaaaggttgttgccggtcctttgtcaagaccacggccttacaccggagcaagtcgtggccattgcaaataataacggtggcaaacaggctcttgagacggttcagagacttctcccagttctctgtcaagcccacgggctgactcccgatcaagttgtagcgattgcgtcgcatgacggagggaaacaagcattggagactgtccaacggctccttcccgtgttgtgtcaagcccacggtttgacgcctgcacaagtggtcgccatcgccagccatgatggcggtaagcaggcgctggaaacagtacagcgcctgctgcctgtactgtgccaggatcatggactgaccccagaccaggtagtcgcaatcgcgaacaataatgggggaaagcaagccctggaaaccgtgcaaaggttgttgccggtcctttgtcaagaccacggccttacaccggagcaagtcgtggccattgcaagcaatgggggtggcaaacaggctcttgagacggttcagagacttctcccagttctctgtcaagcccacgggctgactcccgatcaagttgtagcgattgcgtcgcatgacggagggaaacaagcattggagactgtccaacggctccttcccgtgttgtgtcaagcccacggtttgacgcctgcacaagtggtcgccatcgccagccatgatggcggtaagcaggcgctggaaacagtacagcgcctgctgcctgtactgtgccaggatcatggactgaccccagaccaggtagtcgcaatcgcgtcacatgacgggggaaagcaagccctggaaaccgtgcaaaggttgttgccggtcctttgtcaagaccacggccttacaccggagcaagtcgtggccattgcaagcaacatcggtggcaaacaggctcttgagacggttcagagacttctcccagttctctgtcaagcccacgggctgactcccgatcaagttgtagcgattgcgtcgaacattggagggaaacaagcattggagactgtccaacggctccttcccgtgttgtgtcaagcccacggtttgacgcctgcacaagtggtcgccatcgccaacaacaacggcggtaagcaggcgctggaaacagtacagcgcctgctgcctgtactgtgccaggatcatggactgaccccagaccaggtagtcgcaatcgcgtcacatgacgggggaaagcaagccctggaaaccgtgcaaaggttgttgccggtcctttgtcaagaccacggccttacaccggagcaagtcgtggccattgcaagcaacatcggtggcaaacaggctcttgagacggttcagagacttctcccagttctctgtcaagcccacgggctgactcccgatcaagttgtagcgattgcgtcgaacattggagggaaacaagcattggagactgtccaacggctccttcccgtgttgtgtcaagcccacggtttgacgcctgcacaagtggtcgccatcgcctcgaatggcggcggtaagcaggcgctggaaacagtacagcgcctgctgcctgtactgtgccaggatcatggactgacacccgaacaggtggtcgccattgctaataataacggaggacggccagccttggagtccatcgtagcccaattgtccaggcccgatcccgcgttggctgcgttaacgaatgaccatctggtggcgttggcatgtcttggtggacgacccgcgctcgatgcagtcaaaaagggtctgcctcatgctcccgcattgatcaaaagaaccaaccggcggattcccgagagaacttcccatcgagtcgcgggatcc

SEQ ID NO: 290 - protein, 808 aa, Artificial Sequence
  Description of Artificial Sequence: Synthetic polypeptide
ASTMDYKDHDGDYKDHDIDYKDDDDKMAPKKKRKVGIHRGVPMVDLRTLGYSQQQQEKIKPKVRSTVAQHHEALVGHGFTHAHIVALSQHPAALGTVAVKYQDMIAALPEATHEAIVGVGKQWSGARALEALLTVAGELRGPPLQLDTGQLLKIAKRGGVTAVEAVHAWRNALTGAPLNLTPDQVVAIASNGGGKQALETVQRLLPVLCQDHGLTPEQVVAIANNNGGKQALETVQRLLPVLCQAHGLTPDQVVAIASHDGGKQALETVQRLLPVLCQAHGLTPAQVVAIASHDGGKQALETVQRLLPVLCQDHGLTPDQVVAIANNNGGKQALETVQRLLPVLCQDHGLTPEQVVAIASNGGGKQALETVQRLLPVLCQAHGLTPDQVVAIASHDGGKQALETVQRLLPVLCQAHGLTPAQVVAIASHDGGKQALETVQRLLPVLCQDHGLTPDQVVAIASHDGGKQALETVQRLLPVLCQDHGLTPEQVVAIASNIGGKQALETVQRLLPVLCQAHGLTPDQVVAIASNIGGKQALETVQRLLPVLCQAHGLTPAQVVAIANNNGGKQALETVQRLLPVLCQDHGLTPDQVVAIASHDGGKQALETVQRLLPVLCQDHGLTPEQVVAIASNIGGKQALETVQRLLPVLCQAHGLTPDQVVAIASNIGGKQALETVQRLLPVLCQAHGLTPAQVVAIASNGGGKQALETVQRLLPVLCQDHGLTPEQVVAIANNNGGRPALESIVAQLSRPDPALAALTNDHLVALACLGGRPALDAVKKGLPHAPALIKRTNRRIPERTSHRVAGS

SEQ ID NO: 291 - DNA, 2424 bp, Artificial Sequence
  Description of Artificial Sequence: Synthetic polynucleotide
gctagcaccatggactacaaagaccatgacggtgattataaagatcatgacatcgattacaaggatgacgatgacaagatggcccccaagaagaagaggaaggtgggcattcaccgcggggtacctatggtggacttgaggacactcggttattcgcaacagcaacaggagaaaatcaagcctaaggtcaggagcaccgtcgcgcaacaccacgaggcgcttgtggggcatggcttcactcatgcgcatattgtcgcgctttcacagcaccctgcggcgcttgggacggtggctgtcaaataccaagatatgattgcggccctgcccgaagccacgcacgaggcaattgtaggggtcggtaaacagtggtcgggagcgcgagcacttgaggcgctgctgactgtggcgggtgagcttagggggcctccgctccagctcgacaccgggcagctgctgaagatcgcgaagagagggggagtaacagcggtagaggcagtgcacgcctggcgcaatgcgctcaccggggcccccttgaacctgaccccagaccaggtagtcgcaatcgcgaacaataatgggggaaagcaagccctggaaaccgtgcaaaggttgttgccggtcctttgtcaagaccacggccttacaccggagcaagtcgtggccattgcaagcaatgggggtggcaaacaggctcttgagacggttcagagacttctcccagttctctgtcaagcccacgggctgactcccgatcaagttgtagcgattgcgtccaacggtggagggaaacaagcattggagactgtccaacggctccttcccgtgttgtgtcaagcccacggtttgacgcctgcacaagtggtcgccatcgccagccatgatggcggtaagcaggcgctggaaacagtacagcgcctgctgcctgtactgtgccaggatcatggactgaccccagaccaggtagtcgcaatcgcgtcgaacattgggggaaagcaagccctggaaaccgtgcaaaggttgttgccggtcctttgtcaagaccacggccttacaccggagcaagtcgtggccattgcaagcaacatcggtggcaaacaggctcttgagacggttcagagacttctcccagttctctgtcaagcccacgggctgactcccgatcaagttgtagcgattgcgtccaacggtggagggaaacaagcattggagactgtccaacggctccttcccgtgttgtgtcaagcccacggtttgacgcctgcacaagtggtcgccatcgcctccaatattggcggtaagcaggcgctggaaacagtacagcgcctgctgcctgtactgtgccaggatcatggactgaccccagaccaggtagtcgcaatcgcgtcaaacggagggggaaagcaagccctggaaaccgtgcaaaggttgttgccggtcctttgtcaagaccacggccttacaccggagcaagtcgtggccattgcatcccacgacggtggcaaacaggctcttgagacggttcagagacttctcccagttctctgtcaagcccacgggctgactcccgatcaagttgtagcgattgcgaataacaatggagggaaacaagcattggagactgtccaacggctccttcccgtgttgtgtcaagcccacggtttgacgcctgcacaagtggtcgccatcgcctcgaatggcggcggtaagcaggcgctggaaacagtacagcgcctgctgcctgtactgtgccaggatcatggactgaccccagaccaggtagtcgcaatcgcgtcacatgacgggggaaagcaagccctggaaaccgtgcaaaggttgttgccggtcctttgtcaagaccacggccttacaccggagcaagtcgtggccattgcatcccacgacggtggcaaacaggctcttgagacggttcagagacttctcccagttctctgtcaagcccacgggctgactcccgatcaagttgtagcgattgcgaataacaatggagggaaacaagcattggagactgtccaacggctccttcccgtgttgtgtcaagcccacggtttgacgcctgcacaagtggtcgccatcgccaacaacaacggcggtaagcaggcgctggaaacagtacagcgcctgctgcctgtactgtgccaggatcatggactgacacccgaacaggtggtcgccattgctaataataacggaggacggccagccttggagtccatcgtagcccaattgtccaggcccgatcccgcgttggctgcgttaacgaatgaccatctggtggcgttggcatgtcttggtggacgacccgcgctcgatgcagtcaaaaagggtctgcctcatgctcccgcattgatcaaaagaaccaaccggcggattcccgagagaacttcccatcgagtcgcgggatcc

SEQ ID NO: 292 - protein, 808 aa, Artificial Sequence
  Description of Artificial Sequence: Synthetic polypeptide
ASTMDYKDHDGDYKDHDIDYKDDDDKMAPKKKRKVGIHRGVPMVDLRTLGYSQQQQEKIKPKVRSTVAQHHEALVGHGFTHAHIVALSQHPAALGTVAVKYQDMIAALPEATHEAIVGVGKQWSGARALEALLTVAGELRGPPLQLDTGQLLKIAKRGGVTAVEAVHAWRNALTGAPLNLTPDQVVAIANNNGGKQALETVQRLLPVLCQDHGLTPEQVVAIASNGGGKQALETVQRLLPVLCQAHGLTPDQVVAIASNGGGKQALETVQRLLPVLCQAHGLTPAQVVAIASHDGGKQALETVQRLLPVLCQDHGLTPDQVVAIASNIGGKQALETVQRLLPVLCQDHGLTPEQVVAIASNIGGKQALETVQRLLPVLCQAHGLTPDQVVAIASNGGGKQALETVQRLLPVLCQAHGLTPAQVVAIASNIGGKQALETVQRLLPVLCQDHGLTPDQVVAIASNGGGKQALETVQRLLPVLCQDHGLTPEQVVAIASHDGGKQALETVQRLLPVLCQAHGLTPDQVVAIANNNGGKQALETVQRLLPVLCQAHGLTPAQVVAIASNGGGKQALETVQRLLPVLCQDHGLTPDQVVAIASHDGGKQALETVQRLLPVLCQDHGLTPEQVVAIASHDGGKQALETVQRLLPVLCQAHGLTPDQVVAIANNNGGKQALETVQRLLPVLCQAHGLTPAQVVAIANNNGGKQALETVQRLLPVLCQDHGLTPEQVVAIANNNGGRPALESIVAQLSRPDPALAALTNDHLVALACLGGRPALDAVKKGLPHAPALIKRTNRRIPERTSHRVAGS

SEQ ID NO: 293 - DNA, 2424 bp, Artificial Sequence
  Description of Artificial Sequence: Synthetic polynucleotide
gctagcaccatggactacaaagaccatgacggtgattataaagatcatgacatcgattacaaggatgacgatgacaagatggcccccaagaagaagaggaaggtgggcattcaccgcggggtacctatggtggacttgaggacactcggttattcgcaacagcaacaggagaaaatcaagcctaaggtcaggagcaccgtcgcgcaacaccacgaggcgcttgtggggcatggcttcactcatgcgcatattgtcgcgctttcacagcaccctgcggcgcttgggacggtggctgtcaaataccaagatatgattgcggccctgcccgaagccacgcacgaggcaattgtaggggtcggtaaacagtggtcgggagcgcgagcacttgaggcgctgctgactgtggcgggtgagcttagggggcctccgctccagctcgacaccgggcagctgctgaagatcgcgaagagagggggagtaacagcggtagaggcagtgcacgcctggcgcaatgcgctcaccggggcccccttgaacctgaccccagaccaggtagtcgcaatcgcgaacaataatgggggaaagcaagccctggaaaccgtgcaaaggttgttgccggtcctttgtcaagaccacggccttacaccggagcaagtcgtggccattgcaaataataacggtggcaaacaggctcttgagacggttcagagacttctcccagttctctgtcaagcccacgggctgactcccgatcaagttgtagcgattgcgaataacaatggagggaaacaagcattggagactgtccaacggctccttcccgtgttgtgtcaagcccacggtttgacgcctgcacaagtggtcgccatcgccagccatgatggcggtaagcaggcgctggaaacagtacagcgcctgctgcctgtactgtgccaggatcatggactgaccccagaccaggtagtcgcaatcgcgtcacatgacgggggaaagcaagccctggaaaccgtgcaaaggttgttgccggtcctttgtcaagaccacggccttacaccggagcaagtcgtggccattgcaagcaacatcggtggcaaacaggctcttgagacggttcagagacttctcccagttctctgtcaagcccacgggctgactcccgatcaagttgtagcgattgcgaataacaatggagggaaacaagcattggagactgtccaacggctccttcccgtgttgtgtcaagcccacggtttgacgcctgcacaagtggtcgccatcgcctccaatattggcggtaagcaggcgctggaaacagtacagcgcctgctgcctgtactgtgccaggatcatggactgaccccagaccaggtagtcgcaatcgcgaacaataatgggggaaagcaagccctggaaaccgtgcaaaggttgttgccggtcctttgtcaagaccacggccttacaccggagcaagtcgtggccattgcaagcaacatcggtggcaaacaggctcttgagacggttcagagacttctcccagttctctgtcaagcccacgggctgactcccgatcaagttgtagcgattgcgtccaacggtggagggaaacaagcattggagactgtccaacggctccttcccgtgttgtgtcaagcccacggtttgacgcctgcacaagtggtcgccatcgccaacaacaacggcggtaagcaggcgctggaaacagtacagcgcctgctgcctgtactgtgccaggatcatggactgaccccagaccaggtagtcgcaatcgcgaacaataatgggggaaagcaagccctggaaaccgtgcaaaggttgttgccggtcctttgtcaagaccacggccttacaccggagcaagtcgtggccattgcatcccacgacggtggcaaacaggctcttgagacggttcagagacttctcccagttctctgtcaagcccacgggctgactcccgatcaagttgtagcgattgcgaataacaatggagggaaacaagcattggagactgtccaacggctccttcccgtgttgtgtcaagcccacggtttgacgcctgcacaagtggtcgccatcgccaacaacaacggcggtaagcaggcgctggaaacagtacagcgcctgctgcctgtactgtgccaggatcatggactgacacccgaacaggtggtcgccattgcttcccacgacggaggacggccagccttggagtccatcgtagcccaattgtccaggcccgatcccgcgttggctgcgttaacgaatgaccatctggtggcgttggcatgtcttggtggacgacccgcgctcgatgcagtcaaaaagggtctgcctcatgctcccgcattgatcaaaagaaccaaccggcggattcccgagagaacttcccatcgagtcgcgggatcc

SEQ ID NO: 294 - protein, 808 aa, Artificial Sequence
  Description of Artificial Sequence: Synthetic polypeptide
ASTMDYKDHDGDYKDHDIDYKDDDDKMAPKKKRKVGIHRGVPMVDLRTLGYSQQQQEKIKPKVRSTVAQHHEALVGHGFTHAHIVALSQHPAALGTVAVKYQDMIAALPEATHEAIVGVGKQWSGARALEALLTVAGELRGPPLQLDTGQLLKIAKRGGVTAVEAVHAWRNALTGAPLNLTPDQVVAIANNNGGKQALETVQRLLPVLCQDHGLTPEQVVAIANNNGGKQALETVQRLLPVLCQAHGLTPDQVVAIANNNGGKQALETVQRLLPVLCQAHGLTPAQVVAIASHDGGKQALETVQRLLPVLCQDHGLTPDQVVAIASHDGGKQALETVQRLLPVLCQDHGLTPEQVVAIASNIGGKQALETVQRLLPVLCQAHGLTPDQVVAIANNNGGKQALETVQRLLPVLCQAHGLTPAQVVAIASNIGGKQALETVQRLLPVLCQDHGLTPDQVVAIANNNGGKQALETVQRLLPVLCQDHGLTPEQVVAIASNIGGKQALETVQRLLPVLCQAHGLTPDQVVAIASNGGGKQALETVQRLLPVLCQAHGLTPAQVVAIANNNGGKQALETVQRLLPVLCQDHGLTPDQVVAIANNNGGKQALETVQRLLPVLCQDHGLTPEQVVAIASHDGGKQALETVQRLLPVLCQAHGLTPDQVVAIANNNGGKQALETVQRLLPVLCQAHGLTPAQVVAIANNNGGKQALETVQRLLPVLCQDHGLTPEQVVAIASHDGGRPALESIVAQLSRPDPALAALTNDHLVALACLGGRPALDAVKKGLPHAPALIKRTNRRIPERTSHRVAGS

SEQ ID NO: 295 - DNA, 2424 bp, Artificial Sequence
  Description of Artificial Sequence: Synthetic polynucleotide
gctagcaccatggactacaaagaccatgacggtgattataaagatcatgacatcgattacaaggatgacgatgacaagatggcccccaagaagaagaggaaggtgggcattcaccgcggggtacctatggtggacttgaggacactcggttattcgcaacagcaacaggagaaaatcaagcctaaggtcaggagcaccgtcgcgcaacaccacgaggcgcttgtggggcatggcttcactcatgcgcatattgtcgcgctttcacagcaccctgcggcgcttgggacggtggctgtcaaataccaagatatgattgcggccctgcccgaagccacgcacgaggcaattgtaggggtcggtaaacagtggtcgggagcgcgagcacttgaggcgctgctgactgtggcgggtgagcttagggggcctccgctccagctcgacaccgggcagctgctgaagatcgcgaagagagggggagtaacagcggtagaggcagtgcacgcctggcgcaatgcgctcaccggggcccccttgaacctgaccccagaccaggtagtcgcaatcgcgtcgaacattgggggaaagcaagccctggaaaccgtgcaaaggttgttgccggtcctttgtcaagaccacggccttacaccggagcaagtcgtggccattgcaagcaacatcggtggcaaacaggctcttgagacggttcagagacttctcccagttctctgtcaagcccacgggctgactcccgatcaagttgtagcgattgcgtcgaacattggagggaaacaagcattggagactgtccaacggctccttcccgtgttgtgtcaagcccacggtttgacgcctgcacaagtggtcgccatcgccaacaacaacggcggtaagcaggcgctggaaacagtacagcgcctgctgcctgtactgtgccaggatcatggactgaccccagaccaggtagtcgcaatcgcgtcacatgacgggggaaagcaagccctggaaaccgtgcaaaggttgttgccggtcctttgtcaagaccacggccttacaccggagcaagtcgtggccattgcatcccacgacggtggcaaacaggctcttgagacggttcagagacttctcccagttctctgtcaagcccacgggctgactcccgatcaagttgtagcgattgcgaataacaatggagggaaacaagcattggagactgtccaacggctccttcccgtgttgtgtcaagcccacggtttgacgcctgcacaagtggtcgccatcgccagccatgatggcggtaagcaggcgctggaaacagtacagcgcctgctgcctgtactgtgccaggatcatggactgaccccagaccaggtagtcgcaatcgcgtcacatgacgggggaaagcaagccctggaaaccgtgcaaaggttgttgccggtcctttgtcaagaccacggccttacaccggagcaagtcgtggccattgcaaataataacggtggcaaacaggctcttgagacggttcagagacttctcccagttctctgtcaagcccacgggctgactcccgatcaagttgtagcgattgcgtcgcatgacggagggaaacaagcattggagactgtccaacggctccttcccgtgttgtgtcaagcccacggtttgacgcctgcacaagtggtcgccatcgccagccatgatggcggtaagcaggcgctggaaacagtacagcgcctgctgcctgtactgtgccaggatcatggactgaccccagaccaggtagtcgcaatcgcgtcaaacggagggggaaagcaagccctggaaaccgtgcaaaggttgttgccggtcctttgtcaagaccacggccttacaccggagcaagtcgtggccattgcatcccacgacggtggcaaacaggctcttgagacggttcagagacttctcccagttctctgtcaagcccacgggctgactcccgatcaagttgtagcgattgcgtcgcatgacggagggaaacaagcattggagactgtccaacggctccttcccgtgttgtgtcaagcccacggtttgacgcctgcacaagtggtcgccatcgccaacaacaacggcggtaagcaggcgctggaaacagtacagcgcctgctgcctgtactgtgccaggatcatggactgacacccgaacaggtggtcgccattgctaataataacggaggacggccagccttggagtccatcgtagcccaattgtccaggcccgatcccgcgttggctgcgttaacgaatgaccatctggtggcgttggcatgtcttggtggacgacccgcgctcgatgcagtcaaaaagggtctgcctcatgctcccgcattgatcaaaagaaccaaccggcggattcccgagagaacttcccatcgagtcgcgggatcc

SEQ ID NO: 296 - protein, 808 aa, Artificial Sequence
  Description of Artificial Sequence: Synthetic polypeptide
ASTMDYKDHDGDYKDHDIDYKDDDDKMAPKKKRKVGIHRGVPMVDLRTLGYSQQQQEKIKPKVRSTVAQHHEALVGHGFTHAHIVALSQHPAALGTVAVKYQDMIAALPEATHEAIVGVGKQWSGARALEALLTVAGELRGPPLQLDTGQLLKIAKRGGVTAVEAVHAWRNALTGAPLNLTPDQVVAIASNIGGKQALETVQRLLPVLCQDHGLTPEQVVAIASNIGGKQALETVQRLLPVLCQAHGLTPDQVVAIASNIGGKQALETVQRLLPVLCQAHGLTPAQVVAIANNNGGKQALETVQRLLPVLCQDHGLTPDQVVAIASHDGGKQALETVQRLLPVLCQDHGLTPEQVVAIASHDGGKQALETVQRLLPVLCQAHGLTPDQVVAIANNNGGKQALETVQRLLPVLCQAHGLTPAQVVAIASHDGGKQALETVQRLLPVLCQDHGLTPDQVVAIASHDGGKQALETVQRLLPVLCQDHGLTPEQVVAIANNNGGKQALETVQRLLPVLCQAHGLTPDQVVAIASHDGGKQALETVQRLLPVLCQAHGLTPAQVVAIASHDGGKQALETVQRLLPVLCQDHGLTPDQVVAIASNGGGKQALETVQRLLPVLCQDHGLTPEQVVAIASHDGGKQALETVQRLLPVLCQAHGLTPDQVVAIASHDGGKQALETVQRLLPVLCQAHGLTPAQVVAIANNNGGKQALETVQRLLPVLCQDHGLTPEQVVAIANNNGGRPALESIVAQLSRPDPALAALTNDHLVALACLGGRPALDAVKKGLPHAPALIKRTNRRIPERTSHRVAGS

SEQ ID NO: 297 - DNA, 2424 bp, Artificial Sequence
  Description of Artificial Sequence: Synthetic polynucleotide
gctagcaccatggactacaaagaccatgacggtgattataaagatcatgacatcgattacaaggatgacgatgacaagatggcccccaagaagaagaggaaggtgggcattcaccgcggggtacctatggtggacttgaggacactcggttattcgcaacagcaacaggagaaaatcaagcctaaggtcaggagcaccgtcgcgcaacaccacgaggcgcttgtggggcatggcttcactcatgcgcatattgtcgcgctttcacagcaccctgcggcgcttgggacggtggctgtcaaataccaagatatgattgcggccctgcccgaagccacgcacgaggcaattgtaggggtcggtaaacagtggtcgggagcgcgagcacttgaggcgctgctgactgtggcgggtgagcttagggggcctccgctccagctcgacaccgggcagctgctgaagatcgcgaagagagggggagtaacagcggtagaggcagtgcacgcctggcgcaatgcgctcaccggggcccccttgaacctgaccccagaccaggtagtcgcaatcgcgaacaataatgggggaaagcaagccctggaaaccgtgcaaaggttgttgccggtcctttgtcaagaccacggccttacaccggagcaagtcgtggccattgcatcccacgacggtggcaaacaggctcttgagacggttcagagacttctcccagttctctgtcaagcccacgggctgactcccgatcaagttgtagcgattgcgtcgcatgacggagggaaacaagcattggagactgtccaacggctccttcccgtgttgtgtcaagcccacggtttgacgcctgcacaagtggtcgccatcgccagccatgatggcggtaagcaggcgctggaaacagtacagcgcctgctgcctgtactgtgccaggatcatggactgaccccagaccaggtagtcgcaatcgcgtcgaacattgggggaaagcaagccctggaaaccgtgcaaaggttgttgccggtcctttgtcaagaccacggccttacaccggagcaagtcgtggccattgcaaataataacggtggcaaacaggctcttgagacggttcagagacttctcccagttctctgtcaagcccacgggctgactcccgatcaagttgtagcgattgcgtcgaacattggagggaaacaagcattggagactgtccaacggctccttcccgtgttgtgtcaagcccacggtttgacgcctgcacaagtggtcgccatcgccagccatgatggcggtaagcaggcgctggaaacagtacagcgcctgctgcctgtactgtgccaggatcatggactgaccccagaccaggtagtcgcaatcgcgtcgaacattgggggaaagcaagccctggaaaccgtgcaaaggttgttgccggtcctttgtcaagaccacggccttacaccggagcaagtcgtggccattgcaagcaacatcggtggcaaacaggctcttgagacggttcagagacttctcccagttctctgtcaagcccacgggctgactcccgatcaagttgtagcgattgcgaataacaatggagggaaacaagcattggagactgtccaacggctccttcccgtgttgtgtcaagcccacggtttgacgcctgcacaagtggtcgccatcgccagccatgatggcggtaagcaggcgctggaaacagtacagcgcctgctgcctgtactgtgccaggatcatggactgaccccagaccaggtagtcgcaatcgcgtcgaacattgggggaaagcaagccctggaaaccgtgcaaaggttgttgccggtcctttgtcaagaccacggccttacaccggagcaagtcgtggccattgcaagcaacatcggtggcaaacaggctcttgagacggttcagagacttctcccagttctctgtcaagcccacgggctgactcccgatcaagttgtagcgattgcgtcgcatgacggagggaaacaagcattggagactgtccaacggctccttcccgtgttgtgtcaagcccacggtttgacgcctgcacaagtggtcgccatcgcctccaatattggcggtaagcaggcgctggaaacagtacagcgcctgctgcctgtactgtgccaggatcatggactgacacccgaacaggtggtcgccattgcttctaatgggggaggacggccagccttggagtccatcgtagcccaattgtccaggcccgatcccgcgttggctgcgttaacgaatgaccatctggtggcgttggcatgtcttggtggacgacccgcgctcgatgcagtcaaaaagggtctgcctcatgctcccgcattgatcaaaagaaccaaccggcggattcccgagagaacttcccatcgagtcgcgggatcc

SEQ ID NO: 298 - protein, 808 aa, Artificial Sequence
  Description of Artificial Sequence: Synthetic polypeptide
ASTMDYKDHDGDYKDHDIDYKDDDDKMAPKKKRKVGIHRGVPMVDLRTLGYSQQQQEKIKPKVRSTVAQHHEALVGHGFTHAHIVALSQHPAALGTVAVKYQDMIAALPEATHEAIVGVGKQWSGARALEALLTVAGELRGPPLQLDTGQLLKIAKRGGVTAVEAVHAWRNALTGAPLNLTPDQVVAIANNNGGKQALETVQRLLPVLCQDHGLTPEQVVAIASHDGGKQALETVQRLLPVLCQAHGLTPDQVVAIASHDGGKQALETVQRLLPVLCQAHGLTPAQVVAIASHDGGKQALETVQRLLPVLCQDHGLTPDQVVAIASNIGGKQALETVQRLLPVLCQDHGLTPEQVVAIANNNGGKQALETVQRLLPVLCQAHGLTPDQVVAIASNIGGKQALETVQRLLPVLCQAHGLTPAQVVAIASHDGGKQALETVQRLLPVLCQDHGLTPDQVVAIASNIGGKQALETVQRLLPVLCQDHGLTPEQVVAIASNIGGKQALETVQRLLPVLCQAHGLTPDQVVAIANNNGGKQALETVQRLLPVLCQAHGLTPAQVVAIASHDGGKQALETVQRLLPVLCQDHGLTPDQVVAIASNIGGKQALETVQRLLPVLCQDHGLTPEQVVAIASNIGGKQALETVQRLLPVLCQAHGLTPDQVVAIASHDGGKQALETVQRLLPVLCQAHGLTPAQVVAIASNIGGKQALETVQRLLPVLCQDHGLTPEQVVAIASNGGGRPALESIVAQLSRPDPALAALTNDHLVALACLGGRPALDAVKKGLPHAPALIKRTNRRIPERTSHRVAGS

SEQ ID NO: 299 - DNA, 2424 bp, Artificial Sequence
  Description of Artificial Sequence: Synthetic polynucleotide
gctagcaccatggactacaaagaccatgacggtgattataaagatcatgacatcgattacaaggatgacgatgacaagatggcccccaagaagaagaggaaggtgggcattcaccgcggggtacctatggtggacttgaggacactcggttattcgcaacagcaacaggagaaaatcaagcctaaggtcaggagcaccgtcgcgcaacaccacgaggcgcttgtggggcatggcttcactcatgcgcatattgtcgcgctttcacagcaccctgcggcgcttgggacggtggctgtcaaataccaagatatgattgcggccctgcccgaagccacgcacgaggcaattgtaggggtcggtaaacagtggtcgggagcgcgagcacttgaggcgctgctgactgtggcgggtgagcttagggggcctccgctccagctcgacaccgggcagctgctgaagatcgcgaagagagggggagtaacagcggtagaggcagtgcacgcctggcgcaatgcgctcaccggggcccccttgaacctgaccccagaccaggtagtcgcaatcgcgtcacatgacgggggaaagcaagccctggaaaccgtgcaaaggttgttgccggtcctttgtcaagaccacggccttacaccggagcaagtcgtggccattgcatcccacgacggtggcaaacaggctcttgagacggttcagagacttctcccagttctctgtcaagcccacgggctgactcccgatcaagttgtagcgattgcgtcgcatgacggagggaaacaagcattggagactgtccaacggctccttcccgtgttgtgtcaagcccacggtttgacgcctgcacaagtggtcgccatcgccagccatgatggcggtaagcaggcgctggaaacagtacagcgcctgctgcctgtactgtgccaggatcatggactgaccccagaccaggtagtcgcaatcgcgaacaataatgggggaaagcaagccctggaaaccgtgcaaaggttgttgccggtcctttgtcaagaccacggccttacaccggagcaagtcgtggccattgcatcccacgacggtggcaaacaggctcttgagacggttcagagacttctcccagttctctgtcaagcccacgggctgactcccgatcaagttgtagcgattgcgaataacaatggagggaaacaagcattggagactgtccaacggctccttcccgtgttgtgtcaagcccacggtttgacgcctgcacaagtggtcgccatcgccaacaacaacggcggtaagcaggcgctggaaacagtacagcgcctgctgcctgtactgtgccaggatcatggactgaccccagaccaggtagtcgcaatcgcgtcacatgacgggggaaagcaagccctggaaaccgtgcaaaggttgttgccggtcctttgtcaagaccacggccttacaccggagcaagtcgtggccattgcaagcaatgggggtggcaaacaggctcttgagacggttcagagacttctcccagttctctgtcaagcccacgggctgactcccgatcaagttgtagcgattgcgtcgcatgacggagggaaacaagcattggagactgtccaacggctccttcccgtgttgtgtcaagcccacggtttgacgcctgcacaagtggtcgccatcgccagccatgatggcggtaagcaggcgctggaaacagtacagcgcctgctgcctgtactgtgccaggatcatggactgaccccagaccaggtagtcgcaatcgcgtcacatgacgggggaaagcaagccctggaaaccgtgcaaaggttgttgccggtcctttgtcaagaccacggccttacaccggagcaagtcgtggccattgcatcccacgacggtggcaaacaggctcttgagacggttcagagacttctcccagttctctgtcaagcccacgggctgactcccgatcaagttgtagcgattgcgaataacaatggagggaaacaagcattggagactgtccaacggctccttcccgtgttgtgtcaagcccacggtttgacgcctgcacaagtggtcgccatcgccagccatgatggcggtaagcaggcgctggaaacagtacagcgcctgctgcctgtactgtgccaggatcatggactgacacccgaacaggtggtcgccattgcttcccacgacggaggacggccagccttggagtccatcgtagcccaattgtccaggcccgatcccgcgttggctgcgttaacgaatgaccatctggtggcgttggcatgtcttggtggacgacccgcgctcgatgcagtcaaaaagggtctgcctcatgctcccgcattgatcaaaagaaccaaccggcggattcccgagagaacttcccatcgagtcgcgggatcc

SEQ ID NO: 300 - protein, 808 aa, Artificial Sequence
  Description of Artificial Sequence: Synthetic polypeptide
ASTMDYKDHDGDYKDHDIDYKDDDDKMAPKKKRKVGIHRGVPMVDLRTLGYSQQQQEKIKPKVRSTVAQHHEALVGHGFTHAHIVALSQHPAALGTVAVKYQDMIAALPEATHEAIVGVGKQWSGARALEALLTVAGELRGPPLQLDTGQLLKIAKRGGVTAVEAVHAWRNALTGAPLNLTPDQVVAIASHDGGKQALETVQRLLPVLCQDHGLTPEQVVAIASHDGGKQALETVQRLLPVLCQAHGLTPDQVVAIASHDGGKQALETVQRLLPVLCQAHGLTPAQVVAIASHDGGKQALETVQRLLPVLCQDHGLTPDQVVAIANNNGGKQALETVQRLLPVLCQDHGLTPEQVVAIASHDGGKQALETVQRLLPVLCQAHGLTPDQVVAIANNNGGKQALETVQRLLPVLCQAHGLTPAQVVAIANNNGGKQALETVQRLLPVLCQDHGLTPDQVVAIASHDGGKQALETVQRLLPVLCQDHGLTPEQVVAIASNGGGKQALETVQRLLPVLCQAHGLTPDQVVAIASHDGGKQALETVQRLLPVLCQAHGLTPAQVVAIASHDGGKQALETVQRLLPVLCQDHGLTPDQVVAIASHDGGKQALETVQRLLPVLCQDHGLTPEQVVAIASHDGGKQALETVQRLLPVLCQAHGLTPDQVVAIANNNGGKQALETVQRLLPVLCQAHGLTPAQVVAIASHDGGKQALETVQRLLPVLCQDHGLTPEQVVAIASHDGGRPALESIVAQLSRPDPALAALTNDHLVALACLGGRPALDAVKKGLPHAPALIKRTNRRIPERTSHRVAGS

SEQ ID NO: 301 - DNA, 88 bp, Homo sapiens
ttcccagactcagtgggaagagctccctcaccatgagtagcgctatgttggtgacttgcctcccggaccccagcagcagcttccgtga

SEQ ID NO: 302 - DNA, 80 bp, Homo sapiens
ttcccagactcagtgggaagagctccctcaccatgagtagcgctatgttgcctcccggaccccagcagcagcttccgtga

SEQ ID NO: 303 - DNA, 57 bp, Homo sapiens
ttcccagactcagtgggaagagctccctcacccggaccccagcagcagcttccgtga

SEQ ID NO: 304 - DNA, 88 bp, Homo sapiens
ggcgtgggagagtggatttccgaagctgacagatgggtattctttgacggggggtaggggcggaacctgagaggcgtaaggcgttgtg

SEQ ID NO: 305 - DNA, 71 bp, Homo sapiens
ggcgtgggagagtggatttccgaagctgacagatgggtaggggcggaacctgagaggcgtaaggcgttgtg

SEQ ID NO: 306 - DNA, 65 bp, Homo sapiens
ggcgtgggagagtggatttccgaagctgacagaggggcggaacctgagaggcgtaaggcgttgtg

SEQ ID NO: 307 - DNA, 61 bp, Homo sapiens
ggcgtgggagagtggatttccgaagctgacagatggaacctgagaggcgtaaggcgttgtg

SEQ ID NO: 308 - DNA, 50 bp, Homo sapiens
ggcgtgggagagtggatttccgaagctgacagatggggtaaggcgttgtg

SEQ ID NO: 309 - DNA, 49 bp, Homo sapiens
ggcgtgggagagtggatttccgaagctgacagatgggtaaggcgttgtg

SEQ ID NO: 310 - DNA, 60 bp, Homo sapiens
agtggatttccgaagctgacagatgtggaagaagaggctggtcatgaggtcaggagttcc

SEQ ID NO: 311 - DNA, 60 bp, Homo sapiens
cgctcaggaggccttcaccctctgctctgggtaaaggaactggaatatgccttgaggggg

SEQ ID NO: 312 - DNA, 88 bp, Homo sapiens
cctgagctgtggtttggaggagccgtgtgttggaagaagatggcagatccaggaatgatgagtctttttggcgaggatgggaatattt

SEQ ID NO: 313 - DNA, 79 bp, Homo sapiens
cctgagctgtggtttggaggagccgtgtgttggaagaagatcagaatgatgagtctttttggcgaggatgggaatattt

SEQ ID NO: 314 - DNA, 78 bp, Homo sapiens
cctgagctgtggtttggaggagccgtgtgttggaagaagatggaatgatgagtctttttggcgaggatgggaatattt

SEQ ID NO: 315 - DNA, 60 bp, Homo sapiens
cctgagctgtggtttggaggagccgtgtgttggaagaagatggcgaggatgggaatattt

SEQ ID NO: 316 - DNA, 41 bp, Homo sapiens
taaagaaatatggaatgacataaaatccagtaaatcctatg

SEQ ID NO: 317 - DNA, 88 bp, Homo sapiens
gaggggggggaagatggcggacgtgcttagcgtcctgcgacagtacaacatccagaagaaggagattgtggtgaagggagacgaagtg

SEQ ID NO: 318 - DNA, 81 bp, Homo sapiens
gaggggggggaagatggcggacgtgcttagcgtcctgcgacagtacagaagaaggagattgtggtgaagggagacgaagtg

SEQ ID NO: 319 - DNA, 80 bp, Homo sapiens
gaggggggggaagatggcggacgtgcttagcgtcctgcgacagtacaacgaaggagattgtggtgaagggagacgaagtg

SEQ ID NO: 320 - DNA, 80 bp, Homo sapiens
gaggggggggaagatggcggacgtgcttagcgtcctgcgacatccagaagaaggagattgtggtgaagggagacgaagtg

SEQ ID NO: 321 - DNA, 76 bp, Homo sapiens
gaggggggggaagatggcggacgtgcttagcgtcctgcgacagaagaaggagattgtggtgaagggagacgaagtg

SEQ ID NO: 322 - DNA, 68 bp, Homo sapiens
gaggggggggaagatggcggacgtgcttagcgtcctgcgacagtattgtggtgaagggagacgaagtg

SEQ ID NO: 323 - DNA, 66 bp, Homo sapiens
gaggggggggaagatggcggacgtgcttagcgtcctgcgacagttgtggtgaagggagacgaagtg

SEQ ID NO: 324 - DNA, 88 bp, Homo sapiens
gaggggggggaagatggcggacgtgcttagcgtcctgcgacagtacaacaacatccagaagaaggagattgtggtgaagggagacgaa

SEQ ID NO: 325 - DNA, 56 bp, Homo sapiens
agggcgaggcgacaagagaagaaggaggcaggattgtggtgaagggagacgaagtg

SEQ ID NO: 326 - DNA, 88 bp, Homo sapiens
ttagtattttgaagttaatatcacaatgagttcaggcttatggagccaagaaaaagtcacttcaccctactgggaagagcggattttt

SEQ ID NO: 327 - DNA, 79 bp, Homo sapiens
ttagtattttgaagttaatatcacaatgagttcaggcttatggaaagtcacttcaccctactgggaagagcggattttt

SEQ ID NO: 328 - DNA, 59 bp, Homo sapiens
ttagtattttgaagttaatatcacaagtcacttcaccctactgggaagagcggattttt

SEQ ID NO: 329 - DNA, 47 bp, Homo sapiens
ttagtattttgaagttaatatcaccctactgggaagagcggattttt

SEQ ID NO: 330 - DNA, 40 bp, Homo sapiens
ttagtattttgaagttccctactgggaagagcggattttt

SEQ ID NO: 331 - DNA, 36 bp, Homo sapiens
taagtcacttcaccctactgggaagagcggattttt

SEQ ID NO: 332 - DNA, 33 bp, Homo sapiens
ttagtatttccctactgggaagagcggattttt

SEQ ID NO: 333 - DNA, 31 bp, Homo sapiens
ttagtattttgaagttgaagagcggattttt

SEQ ID NO: 334 - DNA, 22 bp, Homo sapiens
ttagtattttgaacggattttt

SEQ ID NO: 335 - DNA, 4 bp, Homo sapiens
ttag

SEQ ID NO: 336 - DNA, 116 bp, Homo sapiens
taatatcacaatgagttctcaggggcacaccaggccccaggggaacaccaggccctgggtaagcatgcagtcccaggtggacatcaggtgccaggaggaaaagtcacttcacccta

SEQ ID NO: 337 - DNA, 88 bp, Homo sapiens
tccacacagcctgtggcacagacgtggagggccactgagccccgctacccgccccacagcctttcctacccagtgcagatcgcccgga

SEQ ID NO: 338 - DNA, 87 bp, Homo sapiens
tccacacagcctgtggcacagacgtggagggccactgagccccgctaccgccccacagcctttcctacccagtgcagatcgcccgga

SEQ ID NO: 339 - DNA, 81 bp, Homo sapiens
tccacacagcctgtggcacagacgtggagggccactgagccccgccccacagcctttcctacccagtgcagatcgcccgga

SEQ ID NO: 340 - DNA, 76 bp, Homo sapiens
tccacacagcctgtggcacagacgtggagggccactgagccccacagcctttcctacccagtgcagatcgcccgga

SEQ ID NO: 341 - DNA, 19 bp, Homo sapiens
tccacacagatcgcccgga

SEQ ID NO: 342 - DNA, 38 bp, Homo sapiens
cccccaccacctttcctacccagtgcagatcgcccgga

SEQ ID NO: 343 - DNA, 33 bp, Homo sapiens
gcttattgcggcctttctcctgggagccaggct

SEQ ID NO: 344 - DNA, 88 bp, Homo sapiens
tccacacagcctgtggcacagacgtggagggccactgagccccgctaccacccgccccacagcctttcctacccagtgcagatcgccc

SEQ ID NO: 345 - DNA, 88 bp, Homo sapiens
tttctcttacaggcaaatgttctgaaaaagactctgcatgggaatggcctgccttacgatgacagaaatggagggaacatccacctct

SEQ ID NO: 346 - DNA, 84 bp, Homo sapiens
tttctcttacaggcaaatgttctgaaaaagactctgcatggggcctgccttacgatgacagaaatggagggaacatccacctct

SEQ ID NO: 347 - DNA, 83 bp, Homo sapiens
tttctcttacaggcaaatgttctgaaaaagactctgcatgggcctgccttacgatgacagaaatggagggaacatccacctct

SEQ ID NO: 348 - DNA, 82 bp, Homo sapiens
tttctcttacaggcaaatgttctgaaaaagactctgcatgggaatggttacgatgacagaaatggagggaacatccacctct

SEQ ID NO: 349 - DNA, 80 bp, Homo sapiens
tttctcttacaggcaaatgttctgaaaaagactctgcagcctgccttacgatgacagaaatggagggaacatccacctct

SEQ ID NO: 350 - DNA, 73 bp, Homo sapiens
tttctcttacaggcaaatgttctgaaaaagactctgccttacgatgacagaaatggagggaacatccacctct

SEQ ID NO: 351 - DNA, 64 bp, Homo sapiens
tttctcttacaggcaaatgttctgaaaaagactctgcatgggaatggagggaacatccacctct

SEQ ID NO: 352 - DNA, 63 bp, Homo sapiens
tttctcttacaggcaaatgttctgaaaaagacgatgacagaaatggagggaacatccacctct

SEQ ID NO: 353 - DNA, 62 bp, Homo sapiens
tttctcttacaggcaaatgttctgaaaaagactctgcagaaatggagggaacatccacctct

SEQ ID NO: 354 - DNA, 35 bp, Homo sapiens
tttctcttacaggcatggagggaacatccacctct

SEQ ID NO: 355 - DNA, 34 bp, Homo sapiens
tacgatgacagaaatggagggaacatccacctct

SEQ ID NO: 356 - DNA, 84 bp, Homo sapiens
tttctcttacaggcaaatgttctgaaaaagactctgcatggagtaagtcttacgatgacagaaatggagggaacatccacctct

SEQ ID NO: 357 - DNA, 60 bp, Homo sapiens
cggaggtttgctgcaaacagagaaatttcgatgacagaaatggagggaacatccacctct

SEQ ID NO: 358 - DNA, 88 bp, Homo sapiens
cgggaggcgagccgatgccgagctgctccacgtccaccatgccgggcatgatctgcaagaacccagacctcgagtttgactcgctaca

SEQ ID NO: 359 - DNA, 82 bp, Homo sapiens
cgggaggcgagccgatgccgagctgctccacgtcctcccccatgatctgcaggaacccagacctcgagtttgactcgctaca

SEQ ID NO: 360 - DNA, 80 bp, Homo sapiens
cgggaggcgagccgatgccgagctgctccacgtccgggcatgatctgcaagaacccagacctcgagtttgactcgctaca

SEQ ID NO: 361 - DNA, 78 bp, Homo sapiens
cgggaggcgagccgatgccgagctgctccacgtccaccatatctgcaagaacccagacctcgagtttgactcgctaca

SEQ ID NO: 362 - DNA, 77 bp, Homo sapiens
cgggaggcgagccgatgccgagctgctccacgtccaccatgctgcaagaacccagacctcgagtttgactcgctaca

SEQ ID NO: 363 - DNA, 76 bp, Homo sapiens
cgggaggcgagccgatgccgagctgctccacgtccatgatctgcaagaacccagacctcgagtttgactcgctaca

SEQ ID NO: 364 - DNA, 70 bp, Homo sapiens
cgggaggcgagccgatgccgagctgctccacgtccaccaagaacccagacctcgagtttgactcgctaca

SEQ ID NO: 365 - DNA, 69 bp, Homo sapiens
cgggaggcgagccgatgccgagctgctcatgatctgcaagaacccagacctcgagtttgactcgctaca

SEQ ID NO: 366 - DNA, 46 bp, Homo sapiens
aaggaagcacccccggtcttaaagacctcgagtttgactcgctaca

SEQ ID NO: 367 - DNA, 60 bp, Homo sapiens
agtgttggaggtcggcgccggcccccgggcatgatctgcaagaacccagacctcgagttt

SEQ ID NO: 368 - DNA, 34 bp, Homo sapiens
aaggaagcacccccggtattaaacgaagatgact

SEQ ID NO: 369 - DNA, 222 bp, Homo sapiens
gaggcgagccgatgcccgtgatctgggtcacggctgctccagcttggaggagaggcggctctcccggcgaccctcctcgcgcgggcgcccctgccattcccgggaacaggggctcagccccctttgttagtgctcgtatgtcttggcctggggagcattttggaggcagtgctaggggcagagaggtcctgtttcccccaagtcttgatctgcaagaaccca

SEQ ID NO: 370 - DNA, 88 bp, Homo sapiens
tgcacgtcggccccagccctgaggagccggaccgatgtggaaactgctgcccgccgcgggcccggcaggaggtaagggcagaagggaa

SEQ ID NO: 371 - DNA, 83 bp, Homo sapiens
tgcacgtcggccccagccctgaggagccggaccgatgtgggctgcccgccgcgggcccggcaggaggtaagggcagaagggaa

SEQ ID NO: 372 - DNA, 81 bp, Homo sapiens
tgcacgtcggccccagccctgaggagccggaccgatgtgctgcccgccgcgggcccggcaggaggtaagggcagaagggaa

SEQ ID NO: 373 - DNA, 75 bp, Homo sapiens
tgcacgtcggccccagccctgaggagccggaccgatgtggaaactggcccggcaggaggtaagggcagaagggaa

SEQ ID NO: 374 - DNA, 71 bp, Homo sapiens
tgcacgtcggccccagccctgaggagccggaccgatgtggactcccggcaggaggtaagggcagaagggaa

SEQ ID NO: 375 - DNA, 69 bp, Homo sapiens
tgcacgtcggccccagccctgaggagccggaccgatgtggacccggcaggaggtaagggcagaagggaa

SEQ ID NO: 376 - DNA, 60 bp, Homo sapiens
tgcacgtcggccccagccctgaggagccggaccgatgcaggaggtaagggcagaagggaa

SEQ ID NO: 377 - DNA, 60 bp, Homo sapiens
tgcacgtcggccccagccctgaggagccggaccgatgtggaaagtaagggcagaagggaa

SEQ ID NO: 378 - DNA, 58 bp, Homo sapiens
tgcacgtcggccccagccctgaggagccggaccggcaggaggtaagggcagaagggaa

SEQ ID NO: 379 - DNA, 53 bp, Homo sapiens
tgcacgtcggccccagccctgaggagccggaaggaggtaagggcagaagggaa

SEQ ID NO: 380 - DNA, 49 bp, Homo sapiens
tgcacgtcggccccgcgcgggcccggcaggaggtaagggcagaagggaa

SEQ ID NO: 381 - DNA, 43 bp, Homo sapiens
tgcacgtcggccccagccggcaggaggtaagggcagaagggaa

SEQ ID NO: 382 - DNA, 52 bp, Homo sapiens
gctcccgggagcgcgcacgtcccggagcccatgcctgcgggtgattcctgcg

SEQ ID NO: 383 - DNA, 88 bp, Homo sapiens
tcgcgaagtggaatttgcccagacaagcaacatggctcggaaacgcgcggccggcggggagccgcggggacgcgaactgcgcagccag

SEQ ID NO: 384 - DNA, 86 bp, Homo sapiens
tcgcgaagtggaatttgcccagacaagcaacatggctcggaggaacggccggcggggagccgcggggacgcgaactgcgcagccag

SEQ ID NO: 385 - DNA, 76 bp, Homo sapiens
tcgcgaagtggaatttgcccagacaagcaacatggctcggaaaggggagccgcggggacgcgaactgcgcagccag

SEQ ID NO: 386 - DNA, 73 bp, Homo sapiens
tcgcgaagtggaatttgcccagacaagcaacatggccggcggggagccgcggggacgcgaactgcgcagccag

SEQ ID NO: 387 - DNA, 71 bp, Homo sapiens
tcgcgaagtggaatttgcccagacaagcaacatggctcggggagccgcggggacgcgaactgcgcagccag

SEQ ID NO: 388 - DNA, 69 bp, Homo sapiens
tcgcgaagtggaatttgcccagacaagcaacatggcggggagccgcggggacgcgaactgcgcagccag

SEQ ID NO: 389 - DNA, 53 bp, Homo sapiens
tcgcgaagtggaatttgcccagacaagcaacatgttgcgaactgcgcagccag

SEQ ID NO: 390 - DNA, 49 bp, Homo sapiens
tcgcgaagtggaatttgcccagacaagcaacatggctcggcgcagccag

SEQ ID NO: 391 - DNA, 12 bp, Homo sapiens
tcgcgcagccag

SEQ ID NO: 392 - DNA, 31 bp, Homo sapiens
tcgcgaagtggaatccaaggccaagagcaag

SEQ ID NO: 393 - DNA, 88 bp, Homo sapiens
gtcgaccccgctgcacagtccggccggcgccatgaagtgagaagggggctgggggtcgcgctcgctagcgggcgcggggggtcttgaa

SEQ ID NO: 394 - DNA, 81 bp, Homo sapiens
gtcgaccccgctgcacagtccggccggcgccatgaagtgggctgggggtcgcgctcgctagcgggcgcggggggtcttgaa

SEQ ID NO: 395 - DNA, 77 bp, Homo sapiens
gtcgaccccgctgcacagtccggccggcgccatgaagctgggggtcgcgctcgctagcgggcgcggggggtcttgaa

SEQ ID NO: 396 - DNA, 57 bp, Homo sapiens
gtcgaccccgctgcacagtccggccggcgctcgctagcgggcgcggggggtcttgaa

SEQ ID NO: 397 - DNA, 49 bp, Homo sapiens
gtcgaccccgctgcacagtccggccggcgccatgaagtggggtcttgaa

SEQ ID NO: 398 - DNA, 43 bp, Homo sapiens
ggcctctcgctgaatattcatgatggggtcatcggtgggcgcg

SEQ ID NO: 399 - DNA, 53 bp, Homo sapiens
gtcgaccccgctgcacagtccggccggcgccatgaagggtgaaggggtgggac

SEQ ID NO: 400 - DNA, 65 bp, Homo sapiens
gtcgaccccgctgcacagtccggccggcgccatgaagtgcgtccggggtgggacgggggcagccg

SEQ ID NO: 401 - DNA, 60 bp, Homo sapiens
gtcgaccccgctgcacagtccggccggcgccatgaagtggcagccgcagggagcagcagt

SEQ ID NO: 402 - DNA, 51 bp, Homo sapiens
atggtctcgtaatataggtggagcgagccctcgaggggggtcttgaagatg

SEQ ID NO: 403 - DNA, 33 bp, Homo sapiens
gtcgaccccgctgctgaggacctgagggttacc

SEQ ID NO: 404 - DNA, 42 bp, Homo sapiens
ggcctctcgctgaatattcagctcctgaggacctgagggtta

SEQ ID NO: 405 - DNA, 44 bp, Homo sapiens
gtcgaccccgctgcacagtccggcccgtcacccttctctgggct

SEQ ID NO: 406 - DNA, 40 bp, Homo sapiens
gtcgaccccgctgcacagtccggccgctcgacgaccgggc

SEQ ID NO: 407 - DNA, 46 bp, Homo sapiens
gtcgaccccgctgcacagtccggccggcgaccgggcactgtggagg

SEQ ID NO: 408 - DNA, 39 bp, Homo sapiens
gtcgaccccgctgcacagtccggccgggcactgtggagg

SEQ ID NO: 409 - DNA, 19 bp, Homo sapiens
gtcgacccagcagcccctg

SEQ ID NO: 410 - DNA, 19 bp, Homo sapiens
gtcgacccccctgccgcca

SEQ ID NO: 411 - DNA, 43 bp, Homo sapiens
ggcctctcgctgaatattcatgagccgccaggctcaacgtgga

SEQ ID NO: 412 - DNA, 18 bp, Homo sapiens
tatgtacgcctccctggg

SEQ ID NO: 413 - DNA, 18 bp, Homo sapiens
tacagaagcgggcaaagg

SEQ ID NO: 414 - DNA, 18 bp, Homo sapiens
tccgaagctgacagatgg

SEQ ID NO: 415 - DNA, 18 bp, Homo sapiens
tcaggttccgcccctacc

SEQ ID NO: 416 - DNA, 18 bp, Homo sapiens
ttagacttaggtaagtaa

SEQ ID NO: 417 - DNA, 18 bp, Homo sapiens
tagtttgtagttctcccc

SEQ ID NO: 418 - DNA, 17 bp, Homo sapiens
tccggccggcgccatga

SEQ ID NO: 419 - DNA, 16 bp, Homo sapiens
tagcgagcgcgacccc

SEQ ID NO: 420 - DNA, 18 bp, Homo sapiens
taggcgccaaggccatgt

SEQ ID NO: 421 - DNA, 18 bp, Homo sapiens
tggcccgaggcggagttc

SEQ ID NO: 422 - DNA, 18 bp, Homo sapiens
tgaagggacatcaccttt

SEQ ID NO: 423 - DNA, 17 bp, Homo sapiens
tctactgaatcttgagc

SEQ ID NO: 424 - DNA, 16 bp, Homo sapiens
tcggccaccatgtccc

SEQ ID NO: 425 - DNA, 18 bp, Homo sapiens
tccaggcagctggagccc

SEQ ID NO: 426 - DNA, 18 bp, Homo sapiens
tctgaaaaagactctgca

SEQ ID NO: 427 - DNA, 18 bp, Homo sapiens
tccatttctgtcatcgta

SEQ ID NO: 428 - DNA, 18 bp, Homo sapiens
tgaaaatgactgaatata

SEQ ID NO: 429 - DNA, 17 bp, Homo sapiens
ttgcctacgccaccagc

SEQ ID NO: 430 - DNA, 18 bp, Homo sapiens
tgcttagacgctggattt

SEQ ID NO: 431 - DNA, 18 bp, Homo sapiens
ttcggtgcttacctggtt

SEQ ID NO: 432 - DNA, 17 bp, Homo sapiens
tcccagacatgacagcc

SEQ ID NO: 433 - DNA, 18 bp, Homo sapiens
tccttttgtttctgctaa

SEQ ID NO: 434 - DNA, 18 bp, Homo sapiens
ttgccgtcccaagcaatg

SEQ ID NO: 435 - DNA, 18 bp, Homo sapiens
tgttcaatatcgtccggg

SEQ ID NO: 436 - DNA, 18 bp, Homo sapiens
tgggccagagatggcggc

SEQ ID NO: 437 - DNA, 18 bp, Homo sapiens
taaagccgccgcctccgg

SEQ ID NO: 438 - DNA, 18 bp, Homo sapiens
tgcccagacaagcaacat

SEQ ID NO: 439 - DNA, 18 bp, Homo sapiens
tccccgcggctccccgcc